European Patent Specification EP 3 414 334 B1, published October 11, 2023. Title: Process. Applicant: Bergen Teknologioverføring AS University of New South Wales Innovations. The sequence listing filed with the application follows.

SEQUENCE LISTING (101 sequences)

SEQ ID NO: 1 - protein, 252 aa, Cylindrospermopsis raciborskii T3
MIDTISVLLREWTVISLTGLAFWLWEIRSPFHQIEYKAKFFKELGWAGISFVFRNVYAYVSVAIIKLLSSLFMGESANFAGVMYVPLWLRIITAYILQDLTDYLLHRTMHSNQFLWLTHKWHHSTKQSWWLSGNKDSFTGGLLYTVTALWFPLLDIPSEVMSVVAVHQVIHNNWIHLNVKWNSWLGIIEWIYVTPRIHTLHHLDTGGRNLSSMFTFIDRLFGTYVFPENFDIEKSKNRLDDQSVTVKTILGF

SEQ ID NO: 2 - DNA, 759 bp, Cylindrospermopsis raciborskii T3
atgatagatacaatatcagtactattaagagagtggactgtaatttttcttacaggtttagccttctggctttgggaaattcgctctcccttgcatcaaattgaatacaaagctaaattcttcaaggaattgggatgggcgggaatatcattcgtctttagaattgtttatgcatatgtttctgtggcaattataaaactattgagttctctatttatgggagagtcagcaaattttgcaggagtaatgtatgtgcccctctggctgaggatcatcactgcatatatattacaggacttaactgactatctattacacaggacaatgcatagtaatcagtttctttggttgacgcacaaatggcatcattcaacaaagcaatcatggtggctgagtggaaacaaagatagctttaccggcggacttttatatactgttacagctttgtggtttccactgctggacattccctcagaggttatgtctgtagtggcagtacatcaagtgattcataacaattggatacacctcaatgtaaagtggaactcctggttaggaataattgaatggatttatgttacgccccgtattcacactttgcatcatcttgatacagggggaagaaatttgagttctatgtttactttcatcgaccgattatttggaacctatgtgtttccagaaaactttgatatagaaaaatctaaaaatagattggatgatcaatcagtaacggtgaagacaattttgggtttttaa

SEQ ID NO: 3 - DNA, 759 bp, Cylindrospermopsis raciborskii T3
atgattgataccattagcgttctgctgcgtgaatggaccgttatttttctgaccggtctggcattttggctgtgggaaattcgtagtccgctgcatcagattgaatacaaagccaaatttttcaaagaactgggttgggcaggtatcagctttgtttttcgtattgtttatgcctatgttagcgtggccattatcaaactgctgagcagcctgtttatgggtgaaagcgcaaattttgccggtgttatgtatgttccgctgtggctgcgtattattaccgcatatattctgcaggatctgaccgattatctgctgcatcgtaccatgcatagcaatcagtttctgtggctgacccataaatggcatcatagcaccaaacagagttggtggctgagcggtaataaagatagctttaccggtggtctgctgtataccgttaccgcactgtggtttccgctgctggatattccgagcgaagttatgagcgttgttgcagttcatcaggtgattcataacaactggattcacctgaatgtgaaatggaatagctggctgggtattatcgaatggatttatgttacaccgcgtatccataccctgcatcatctggataccggtggtcgtaatctgagcagtatgtttacctttattgatcgtctgtttggcacctatgtgtttccggaaaactttgatatcgaaaaaagcaaaaaccgcctggatgatcagagcgttaccgttaaaaccattctgggtttctga

SEQ ID NO: 4 - protein, 117 aa, Cylindrospermopsis raciborskii T3
MFQTKSYYSVVGLETELIKGKFFMSNELTNEQVFKLVCMEVIEKMGFAHFPPIILVYEMTNSGFVDWCEQMVFVDDKGKLDEGEKFLLDWMRRNVGNFDLIRELMPVAERLEMKMRS

SEQ ID NO: 5 - DNA, 354 bp, Cylindrospermopsis raciborskii T3
atgttccagaccaagagttattactctgtggtaggattagaaacagaattgattaaaggaaaattctttatgtctaatgaattgacaaacgaacaagtatttaagctggtttgtatggaagtcattgaaaaaatgggattcgcacactttcctcccatcattttagtctatgagatgactaattccggatttgtagattggtgcgagcagatggtttttgttgatgataaaggtaagctagatgaaggagaaaaattcttattagactggatgagacggaacgtaggaaactttgatctgatacgtgagttaatgcccgttgctgaacgtctagaaatgaaaatgaggtcataa

SEQ ID NO: 6 - DNA, 354 bp, Cylindrospermopsis raciborskii T3
atgtttcagaccaaaagctattatagcgtcgttggcctggaaaccgaactgattaaaggtaaattcttcatgagcaacgaactgaccaatgaacaggtgtttaaactggtgtgcatggaagtgattgaaaaaatgggttttgcacactttccgcctattatcctggtttatgaaatgaccaattccggctttgttgattggtgcgagcagatggtttttgtggatgataaaggcaaactggatgagggcgaaaaatttctgctggattggatgcgtcgtaatgtgggtaattttgatctgattcgcgaactgatgccggtggcagaacgcctggaaatgaaaatgcgtagctaa

SEQ ID NO: 7 - protein, 318 aa, Cylindrospermopsis raciborskii T3
MTHVALEQAIAKVPRSIQSELRTILAQHAVIDSSVVASWIDRLGTNISTLMIQLLPVAATYARVPISQFYVGAIALGKPQSKNQLGSGTLYFGADMEFVGQALSFSVHAEQSATINAWLHGETGLQALAIHEAPCGYCRQFLYEMATVNQNFVLLVKSNESQPEQTYTSNKLPHFLPEPFGPADLGLTGGLMQTVFHDLETYSTDDVVLAALSAANQSYAPYTKNFAGVALKDSHGNIFTGRYAENAAFNSSMSPMESALTFMNMNRYSQSLFDICDAVLVEVETGISQRPVTEAFLSSIAPKVKLRYAPATPSSNKL

SEQ ID NO: 8 - DNA, 957 bp, Cylindrospermopsis raciborskii T3
atgacccatgtagcattagaacaggcgattgccaaggttccacgttccattcaatcagagttaaggacaattcttgcccaacatgctgtaattgactcaagtgttgtcgcatcttggattgatcgacttggtactaatattagtacgttaatgattcaattactacccgtagccgcaacttatgctagggtaccaatatcgcagttttatgtaggggcgatcgctcttggtaaaccacaatctaagaatcaactgggttctggaactctttattttggtgccgacatggaatttgtaggacaggcacttagtttctcagttcacgcagaacaatccgccaccataaatgcgtggttgcacggagaaaccggtttacaagcattagcaatccacgaagcaccatgtggatactgccgacaatttttatacgagatggcaactgtaaatcaaaattttgttcttcttgtgaagtctaatgaatcacagcctgagcaaacttatacctcaaataaactcccacattttctacccgagccatttggaccagcggatctaggactcacaggtggattaatgcaaacagtatttcatgatctggagacctattctaccgatgatgttgtgcttgctgctctatccgctgccaatcaaagttatgctccctacacgaaaaattttgcaggggtagcgttaaaagattcccacgggaatatatttacaggtcgatacgctgaaaacgctgcctttaattcatccatgtctccgatggaatctgctctgactttcatgaatatgaatagatattctcaatcactattcgacatttgtgatgctgttttagttgaagtggaaactgggattagtcaaagacccgtcactgaagccttcctttcttctatcgctcccaaggtcaagttaaggtatgcccctgcaactccgtcaagtaataagttatga

SEQ ID NO: 9 - DNA, 957 bp, Cylindrospermopsis raciborskii T3
atgacccatgttgccctggaacaggcaattgcaaaagttccgcgtagcattcagagcgaactgcgtaccattctggcacagcatgcagttattgatagcagcgttgtggcaagctggattgatcgtctgggcaccaatattagtaccctgatgatccagctgctgccggttgcagcaacctatgcacgtgttccgattagccagttttatgttggtgccattgcactgggcaaaccgcagagtaaaaatcagctgggtagcggcaccctgtattttggtgcagatatggaatttgttggtcaggcactgagctttagcgttcatgcagaacagagcgccaccattaatgcctggctgcatggcgaaaccggactgcaggcactggcaatccatgaagcaccgtgtggttattgtcgccagtttctgtatgaaatggcaaccgtgaatcagaattttgtgctgctggtgaaaagcaatgaaagccagccggaacagacctataccagcaacaaactgccgcattttctgcctgaaccgtttggtccagccgatctgggtctgaccggtggcctgatgcagaccgtgtttcacgatctggaaacctatagcaccgatgatgttgttctggcagcactgagtgcagcaaatcagagttatgcaccgtataccaaaaactttgccggtgttgcactgaaagatagtcatggtaacatttttacaggtcgctatgccgaaaacgcagcatttaatagcagcatgagcccgatggaaagcgcactgacctttatgaatatgaatcgttattcacagagcctgttcgatatttgtgatgcagttctggtagaagtggaaaccggtattagtcagcgtccggttaccgaagcctttctgagtagcattgcaccgaaagtgaaactgcgctatgcaccggcaaccccgagcagtaacaaactgtga

SEQ ID NO: 10 - protein, 1245 aa, Cylindrospermopsis raciborskii T3
MLQKINRYTHGFVAVPVILACREKGVFELLADESPLSLNQMVEHLGANSGHFQVALRMLESLHWLSRNKELKYSLTAEAAIHNKISEDILQLYNLPIQSYLEGKQGNLLGRWIERSCQLWNLDNPLMADFLDGLLVIPLLLALHKHNLLADSEDKPLLSSLSSTVQEELGKLFLHLGWADLTAGRLTITELGRFMGERALNTAIVASYTPMLSRIHDVLFGNCLSVFQRDASGHERHIDRTLNVIGSGFQHQKYFADLEESILSVFNQLPLEEQPKYITDMGCGDGTLLKRVWETIQFKSARGKALEQYPLRLIGVDYNEASLKATTRTLASLPHLVLQGDIGNPEQMVRSLEAHGIHDPENILHIRSFLDHDRLFIPPQKRNELKERAHLPYQSVCVDDQGELIPPHVMVQSLVEHLERWSQVVNKHGLMILEVHCLEPRVVYQFLDKSENLHFDAFQGFSQQYLVEAEVFLMSAAQVGLFPKLELSKRYPKTFPFTRITLNYFEKRPYKISHAYLSDLPALVDLEVKCWPENLRASTHEIRRRLELNPQGNLVLIIEDQIIGAIYSQTITSTEALENVKYAQVPTLHTPQGSVIQLLALNILPEFQARGLGNELRDFMLYYCTLKGGIESVVGVTRCRNYVNYSQMPMMEYLKLHNEQRQLLDPIVGFHVSGGAEIRGIIANYRPEDTDNLGMGILIEYNLRDSALHSPGDRKGPYINSAIGSLVPKATSATKENKTVADLVKECILKVMGSQRQAAYAPQQKLLDMGLDSLDLLELQTLLEERLGINLSGTFFLQKNTPTAIITYFQNQVVQEKQSDLAPPVDSANEINTLENVVNQQKIPQVTRVVTEQQGRKVLIDGHWVIDFASCNYLGLDLHPKVKEAIPPALDKWGTHPSWTRLVASPAIYEELEEELSKLLGVPDVLVFPAVTLLQIGILPLLTGNNGVIFGDIAAHRCIYEACCLAQHKGAQFIQYRHNDLNDLAEKLAKYPPEQVKIIVIDGVYSMSADFPDLPAYVHLAKEYNALIYMDDAHGFGILGENPSSDMPYGYKGNGMVNYFDLRFAEDNIIYVAGLSKAYSSYAAFLTCGDRRIKTNFRNAWTAIFSGPSPVASLASALAGLQVNRQEGEQLRKQIYHLTHKLVTQARAIGFEVDNYGYVPIVGVLVGDAQHMIDVCQLLWEYGILITPAIFPIVPLNKSALRFSITAANTEEEIDQAIKSLKAVWDLLQKRKALPCKQEENILKH

SEQ ID NO: 11 - DNA, 3738 bp, Cylindrospermopsis raciborskii T3
atgttacaaaagattaatcgttatactcacggctttgtggcggttcccgttattcttgcgtgtcgagaaaaaggtgtttttgaattactcgccgatgaaagtcctctctctttaaaccaaatggtggaacatctgggagctaacagcggacattttcaagttgctttgaggatgctcgagtctttacattggctttcccgaaataaggagcttaaatactctctaaccgcagaagcagcgattcacaacaaaatttcggaagacattcttcaattgtacaacctaccaattcagtcttatttagaagggaaacaaggaaatttgctgggaagatggattgagcgttcttgccaattgtggaacctggacaatcccctaatggcagattttttagatggattactggtcatcccactcctgctggcactgcacaaacacaacttgcttgcagattcggaggacaaacctttgctctcctcattaagctcaacagtgcaagaagagttgggtaagttatttctccaccttggctgggctgaccttacagcaggtcgtttgaccataaccgaacttggtcgatttatgggagagcgagccttgaatacagccatagtggcgtcctacactcctatgttgtcccgcattcatgatgtattgtttggcaattgtctctccgtattccaaagagatgcttccggtcacgaaaggcacattgatcgcacccttaacgtgatcgggagtggatttcaacaccagaaatattttgccgatttagaagaaagtatcctctcagtattcaatcagttgccattagaagaacaacccaaatacattactgacatggggtgtggcgatggaactctcctgaaacgagtctgggaaaccattcaatttaagtctgctaggggaaaagcactcgaacagtatcccctgcgtcttataggtgtagattataacgaagcttctttaaaagctaccacacgcacccttgctagccttccccacttagttttacagggagatattgggaacccagaacaaatggtgcgttctttagaagctcatggcattcatgatcccgaaaatatcctgcacatccgttcgttcctcgaccatgatcgtctctttattcctcctcagaaaagaaacgaattgaaagaacgtgctcacttaccttaccaatcagtctgtgtcgatgatcaaggagagcttattcctcctcatgttatggtgcaaagtttggtggaacacttagaaagatggtctcaagtggtcaataaacacggtttaatgattttggaggtccattgtttggaaccaagggtagtctatcagtttttagacaaaagcgaaaacttacatttcgatgcgtttcagggattttctcagcagtatcttgtggaagctgaggtttttctcatgtctgctgcacaagtaggtctatttccaaaactagagctttctaaaagatacccaaaaacatttccttttactcgcattacgcttaattacttcgagaaaagaccttacaaaattagtcatgcctatttgtcagatttacctgccttagttgacttggaggtcaagtgttggccagaaaatttacgggcatctactcatgaaattcggcgaagacttgagctaaacccgcaaggtaatttagtgctgattatagaagatcaaattattggtgcgatttattcccaaacaattaccagcactgaggcattagagaatgtaaaatatgcgcaagtgccgacgttacatactccccaagggtcagttattcaactgctcgcactaaatattctacctgagtttcaggcgcgggggttaggaaatgaattgcgggactttatgctttactactgtaccctgaaaggcggcattgagagcgtggtgggtgtaactcgctgtcgaaattatgtcaattattcccaaatgccgatgatggagtatttaaagctacacaatgagcaacgacagcttctggatccaattgtgggtttccatgtgtcgggaggagccgaaattaggggaattattgctaattatcgtccggaagatacagataatctcggcatgggtattttgattgaatataacctgcgcgacagtgctttgcactcgcctggtgatcgcaaaggaccgtatattaactcagcaattggttcattggtaccaaaagcaacatctgcaactaaggaaaacaaaactgtagcggatctcgttaaagaatgcatcttaaaagtaatgggttcccaacgtcaggcagcctacgctccacaacaaaaactgctggatatgggattagattctttagatttattagaactgcaaacgctcctagaggaacgtttagggatcaatctgtctggaacgttctttttacaaaagaacactccaactgccatcatcacttatttccaaaaccaagtggtacaagagaaacaatctgatctagctccacctgttgactcagccaacgaaatcaacactctggaaaacgtagttaaccaacaaaaaattcctcaagtcacaagagtcgtcacagaacaacaaggtcgcaaggtgctaattgacggacattgggtgatagactttgcttcttgcaactatttaggtcttgacttgcatccaaaagttaaggaagcaattccaccagctttggataaatggggcacacatccaagctggactcggcttgttgcttccccagcaatttatgaggaattggaggaagaattgtccaaacttttaggcgtacctgatgttttagtatttccagctgtaacactgcttcagataggaattttaccactattaactgggaataatggtgtcatctttggtgacatagctgcacatcgttgtatttatgaagcgtgctgtctggctcagcacaaaggagcccagttcatccaatatcgacataatgatttgaacgatttagccgaaaaactagcaaaatatccgcctgaacaagtaaagattattgtcattgatggcgtgtattccatgtcggcagattttcccgatctgccagcttacgtgcatctggcaaaagagtacaatgccttaatttacatggatgatgctcatggttttggcattttgggcgaaaatcccagcagcgatatgccttacggttacaaaggaaacgggatggtgaattattttgacctgcggtttgcagaggataatatcatctatgtagctggtttgtccaaagcctattcttcttacgcagcattcttaacttgtggcgatcgccggatcaaaaccaacttccgcaacgcttggactgccatattttctggtccttctcctgttgcgagtttggcaagtgccttagccggattacaggtgaatcgtcaggagggggagcagttaagaaaacaaatttatcacctaactcacaaattggttacacaagcaagagccattggattcgaagtggataactatggttacgttcccatcgtaggcgtgttagtgggagatgctcaacacatgattgatgtgtgtcaactcctttgggaatatggtattttaattactcctgctatttttccaatcgtacctttaaataaaagtgctttaaggttttcgattacagccgccaataccgaagaggagatagaccaagcaattaaatctctcaaagcagtttgggatttgctacaaaaaaggaaagctttgccttgtaagcaggaggaaaacatactcaagcattaa

SEQ ID NO: 12 - DNA, 3738 bp, Cylindrospermopsis raciborskii T3
atgctgcagaaaatcaatcgttatacccatggttttgttgccgttccggttattctggcatgtcgtgaaaaaggtgtttttgaactgctggcagatgaaagtccgctgagcctgaatcagatggttgaacatctgggtgccaatagcggtcattttcaggttgcactgcgtatgctggaaagtctgcattggctgagccgtaataaagaactgaaatatagcctgaccgcagaagcagcaattcataacaaaattagcgaagatatcctgcagctgtataatctgccgattcagagctatctggaaggtaaacagggcaatctgctgggtcgttggattgaacgtagctgtcagctgtggaatctggataatccgctgatggcagattttctggatggtctgctggttattccgctgctgctggcactgcataaacataacctgctggccgattctgaagataaaccgctgctgagcagcctgagcagtaccgttcaagaagaactgggtaaactgtttctgcatctgggttgggcagatctgacagcaggtcgtctgaccattaccgaactgggtcgctttatgggtgaacgtgcactgaataccgcaattgttgcaagctataccccgatgctgagtcgtattcatgatgttctgtttggtaattgcctgagcgtttttcagcgtgatgcaagcggtcatgaacgtcatattgatcgtaccctgaatgttattggtagcggttttcagcaccagaaatactttgcagatctggaagaaagcattctgagcgtgtttaatcagctgccgctggaagaacagccgaaatacattaccgatatgggttgtggtgatggcaccctgctgaaacgtgtttgggaaaccattcagtttaaaagcgcacgtggtaaagcactggaacagtatccgctgcgtctgattggtgttgattataatgaagcaagcctgaaagcaaccacccgtaccctggcaagcctgccgcatctggttctgcagggtgatattggtaatccggaacaaatggttcgtagcctggaagcacatggcattcatgatccggaaaatattctgcatattcgcagctttctggatcacgatcgtctgtttattccgcctcagaaacgtaatgaactgaaagaacgtgcccatctgccgtatcagagtgtttgtgttgatgatcagggtgaactgattcctccgcatgttatggttcagagcctggtggaacacctggaacgttggagccaggttgttaataaacatggtctgatgattctggaagtgcattgtctggaaccgcgtgttgtttatcagtttctggataaaagcgaaaacctgcactttgatgcatttcagggttttagccagcagtatctggttgaagccgaagtttttctgatgagcgcagcacaggttggtctgtttccgaaactggaactgagcaaacgttatccgaaaacctttccgtttacccgtattaccctgaactatttcgaaaaacgtccgtacaaaatcagccatgcatatctgagcgatctgcctgcactggttgacctggaagttaaatgttggcctgagaatctgcgtgcaagcacccatgaaattcgtcgtcgtctggaactgaatccgcagggtaacctggttctgattattgaagatcagattatcggtgccatttacagccagaccattacaagcaccgaagccctggaaaatgttaaatatgcacaggttccgaccctgcatacaccgcagggttcagtgattcagctgctggccctgaacattctgccggaatttcaggcacgtggtctgggcaatgaactgcgtgattttatgctgtattattgcaccctgaaaggtggtattgaaagcgttgttggtgttacccgttgtcgcaattatgtgaattatagccagatgccgatgatggaatatctgaaactgcataatgaacagcgtcaactgctggatccgattgttggttttcatgttagcggtggtgcagaaattcgtggcattattgcaaattatcgtccggaagatacagataatctgggtatgggtattctgatcgaatataacctgcgtgatagcgcactgcattcaccgggtgatcgtaaaggtccgtatatcaatagcgcaattggtagcctggttccgaaagcgaccagcgcaaccaaagaaaacaaaaccgttgcggatctggtgaaagaatgtattctgaaagtgatgggtagccagcgtcaggcagcatatgcaccgcagcagaaactgctggacatgggtctggatagcctggatctgctggaactgcagaccctgctggaagaacgtctgggtattaatctgagcggcaccttttttctgcaaaaaaacaccccgaccgccatcattacctattttcagaatcaggtcgtgcaagagaaacagagtgatctggcaccgcctgttgatagcgccaatgaaatcaatacactggaaaacgttgtgaatcagcagaaaattccgcaggttacacgtgttgttaccgaacagcagggacgtaaagttctgattgatggtcattgggttattgattttgccagctgtaattatctgggcctggacctgcatccgaaagttaaagaagcaattcctccggcactggataaatggggcacccatccgagctggacccgtctggttgcaagtccggcaatttatgaggaactggaagaggaactgtcaaaactgctgggtgtgccggatgttctggtttttccggcagttacactgctgcagattggtattctgcctctgctgaccggtaataatggtgtgatttttggcgatattgcagcccatcgttgtatttatgaagcatgttgtctggcccagcataaaggtgcacagtttattcagtatcgtcataacgacctgaatgatctggccgaaaaactggccaaatatccgcctgaacaggttaaaatcattgtgatcgatggtgtgtatagcatgagtgccgatttcccggacctgcctgcatatgttcatctggcaaaagaatataacgccctgatctatatggatgatgcacatggctttggcattctgggtgaaaatccgagcagcgatatgccgtatggttataaaggtaatggcatggtgaactactttgatctgcgttttgccgaagataacatcatttatgttgcaggtctgagcaaagcctatagcagctatgcagcatttctgacctgtggtgatcgtcgtattaaaaccaattttcgtaatgcatggaccgcgatttttagcggtccgagtccggttgcaagcctggccagcgcactggcaggtctgcaggttaatcgtcaagaaggtgaacagctgcgcaaacaaatctatcatctgacacataaactggttacccaggctcgtgccattggttttgaagttgataattatggttatgtgccgattgtgggtgttctggtgggtgatgcacagcatatgattgatgtgtgccaactgctgtgggaatatggtatcctgattacccctgcaatttttccgattgtgccgctgaataaatcagcactgcgttttagcattaccgcagcaaataccgaagaagaaattgatcaggccatcaaaagtctgaaagcagtttgggacctgctgcaaaaacgtaaagccctgccgtgtaaacaagaagaaaatatcctgaaacattga

SEQ ID NO: 13 - protein, 128 aa, Cylindrospermopsis raciborskii T3
MLKDFNQFLIRTLAFVFAFGIFLTTGVGIAKADYLVKGGKITNVQNTSSNGDNYAVSISGGFGPCADRVIILPTSGVINRDIHMRGYEAALTALSNGFLVDIYDYTGSSCSNGGQLTITNQLGKLISN

SEQ ID NO: 14 - DNA, 387 bp, Cylindrospermopsis raciborskii T3
atgttgaaagatttcaaccagtttttaatcagaacactagcattcgtattcgcatttggtattttcttaaccactggagttggcattgctaaagctgactacctagttaaaggtggaaagattaccaatgttcaaaatacttcttctaacggtgataattatgccgttagtatcagcggtgggtttggtccttgcgcagatagagtgattatcctaccaacttcaggagtgataaatcgagacattcatatgcgtggctatgaagccgcattaactgcactatccaatggctttttagtagatatttacgactatactggctcttcttgcagcaatggtggccaactaactattaccaaccaattaggtaagctaatcagcaattag

SEQ ID NO: 15 - DNA, 387 bp, Cylindrospermopsis raciborskii T3
atgctgaaagattttaaccagttcctgattcgtaccctggcatttgtttttgcctttggcatttttctgacaaccggtgttggtattgcaaaagcagattatctggtgaaaggtggcaaaattaccaatgttcagaataccagcagcaacggtgataattatgcagttagcattagcggtggttttggtccgtgtgcagatcgtgttattattctgccgaccagcggtgttattaatcgtgatattcacatgcgtggttatgaagcagcactgaccgcactgagcaatggttttctggttgatatctatgattataccggtagcagctgtagcaatggtggccagctgaccattaccaatcagctgggtaaactgattagcaattga

SEQ ID NO: 16 - protein, 471 aa, Cylindrospermopsis raciborskii T3
METTSKKFKSDLILEARASLKLGIPLVISQMCETGIYTANAVMMGLLGTQVLAAGALGALAFLTLLFACHGILSVGGSLAAEAFGANKIDEVSRIASGQIWLAVTLSLPAMLLLWHGDTILLLFGQEESNVLLTKTYLHSILWGFPAALSILTLRGIASALNVPRLITITMLTQLILNTAADYVLIFGKFGLPQLGLAGIGWATALGFWVSFTLGLILLIFSLKVRDYKLFRYLHQFDKQIFVKIFQTGWPMGFQWGAETALFNVTAWVAGYLGTVTLAAHDIGFQTAELAMVIPLGVGNVAMTRVGQSIGEKNPLGARRVASIGITIVGIYASIVALVFWLFPYQIAGIYLNINNPENIEAIKKATTFIPLAGLFQMFYSIQIIIVGALVGLRDTFVPVSMNLIVWGLGLAGSYFMAIILGWGGIGIWLAMVLSPLLSAVILTVRFYRVIDNLLANSDDMLQNASVTTLG

SEQ ID NO: 17 - DNA, 1416 bp, Cylindrospermopsis raciborskii T3
atggaaacaacctcaaaaaaatttaagtcagatctgatattagaagcacgagcaagcctaaagttgggaatccccttagtcatttcacaaatgtgcgaaacgggtatttatacagcgaatgcagtcatgatgggtttacttggtacgcaagttttggccgccggtgctttgggcgcgctcgcttttttgaccttattatttgcctgccatggtattctctcagtaggaggatcactagcagccgaagcttttggggcaaataaaatagatgaagttagtcgtattgcttccgggcaaatatggctagcagttaccttgtctttacctgcaatgcttctgctttggcatggcgatactatcttgctgctattcggtcaagaggaaagcaatgtgttattgacaaaaacgtatttacactcaattttatggggctttcccgctgcgcttagtattttgacattaagaggcattgcctctgctctcaacgttccccgattgataactattactatgctcactcagctgatattgaataccgccgccgattatgtgttaatattcggtaaatttggtcttcctcaacttggtttggctggaataggctgggcaactgctctgggtttttgggttagttttacattggggcttatcttgctgattttctccctgaaagttagagattataaacttttccgctacttgcatcagtttgataaacagatctttgtcaaaatttttcaaactggatggcccatggggtttcaatggggggcggaaacggcactatttaacgtcaccgcttgggtagcagggtatttaggaacggtaacattagcagcccatgatattggcttccaaacggcagaactggcgatggttataccactcggagtcggcaatgtcgctatgacaagagtaggtcagagtataggagaaaaaaaccctttgggtgcaagaagggtagcatcgattggaattacaatagttggcatttatgccagtattgtagcacttgttttctggttgtttccatatcaaattgccggaatttatttaaatataaacaatcccgagaatatcgaagcaattaagaaagcaactacttttatccccttggcgggactattccaaatgttttacagtattcaaataattattgttggggctttggtcggtctgcgggatacatttgttccagtatcaatgaacttaattgtctggggtcttggattggcaggaagctatttcatggcaatcattttaggatggggggggatcgggatttggttggctatggttttgagtccactcctctcggcagttattttaactgttcgtttttatcgagtgattgacaatcttcttgccaacagtgatgatatgttacagaatgcgtctgttactactctaggctga

SEQ ID NO: 18 - DNA, 1416 bp, Cylindrospermopsis raciborskii T3
atggaaaccacgagcaaaaaattcaaaagcgatctgattctggaagcacgtgcaagcctgaaactgggtattccgctggttattagccagatgtgtgaaaccggtatttataccgcaaatgcagttatgatgggtctgctgggcacccaggttctggcagccggtgctctgggtgcactggcatttctgaccctgctgtttgcatgtcatggtattctgagcgttggtggtagcctggcagcggaagcatttggtgcaaacaaaattgatgaagttagccgtattgcaagcggtcagatttggctggcagttaccctgagcctgcctgcaatgctgctgctgtggcatggtgataccattctgctgttatttggtcaagaagaaagcaacgttctgctgaccaaaacctatctgcatagcattctgtggggttttccggcagcactgagtattctgacactgcgtggtattgccagcgcactgaatgttccgcgtctgattaccattaccatgctgacccagctgattctgaataccgcagcagattatgttctgatctttggtaaatttggtctgccgcagctgggtctggcaggtattggttgggcaaccgcactgggtttttgggttagctttaccctgggtctgatcctgctgatttttagcctgaaagtgcgtgattataaactgtttcgttatctgcaccagttcgacaagcagatctttgtgaaaatctttcagaccggttggccgatgggttttcagtggggtgcagaaacagcactgtttaatgttaccgcatgggttgcaggttatctgggcaccgttaccctggcagcacatgatattggttttcagacagcagaactggcaatggttatcccgctgggtgttggtaatgttgcaatgacccgtgttggtcagagcattggtgaaaaaaatccactgggtgcccgtcgtgttgcaagcattggtattaccattgttggtatttatgccagcattgttgccctggttttttggctgtttccgtatcagattgcaggcatttatctgaacattaataacccggaaaacattgaagccatcaaaaaagccaccacctttattccactggcaggtctgtttcagatgttttatagcattcagatcattatcgttggtgcgctggttggtctgcgtgatacctttgttccggttagcatgaatctgattgtttggggtctgggtttagcaggtagctattttatggcaattattctgggttggggtggtattggtatctggctggccatggttctgagtccgctgctgagcgcagttattctgaccgttcgtttttatcgcgtgattgataatctgctggccaacagtgatgatatgctgcagaatgcaagcgttaccaccctgggatga

SEQ ID NO: 19 - protein, 377 aa, Cylindrospermopsis raciborskii T3
MTNQNNQELENDLPIAKQPCPVNSYNEWDTLEEVIVGSVEGAMLPALEPINKWTFPFEELESAQKILSERGGVPYPPEMITLAHKELNEFIHILEAEGVKVRRVKPVDFSVPFSTPAWQVGSGFCAANPRDVFLVIGNEIIEAPMADRNRYFETWAYREMLKEYFQAGAKWTAAPKPQLFDAQYDFNFQFPQLGEPPRFVVTEFEPTFDAADFVRCGRDIFGQKSHVTNGLGIEWLQRHLEDEYRIHIIESHCPEALHIDTTLMPLAPGKILVNPEFVDVNKLPKILKSWDILVAPYPNHIPQNQLRLVSEWAGLNVLMLDEERVIVEKNQEQMIKALKDWGFKPIVCHFESYYPFLGSFHCATLDVRRRGTLQSYF

SEQ ID NO: 20 - DNA, 1134 bp, Cylindrospermopsis raciborskii T3
atgaccaatcaaaataaccaagaattagagaacgatttaccaatcgccaagcagccttgtccggtcaattcttataatgagtgggacacacttgaggaggtcattgttggtagtgttgaaggtgcaatgttaccggccctagaaccaatcaacaaatggacattcccttttgaagaattggaatctgcccaaaagatactctctgagaggggaggagttccttatccaccagagatgattacattagcacacaaagaactaaatgaatttattcacattcttgaagcagaaggggtcaaagttcgtcgagttaaacctgtagatttctctgtccccttctccacaccagcttggcaagtaggaagtggtttttgtgccgccaatcctcgcgatgtttttttggtgattgggaatgagattattgaagcaccaatggcagatcgcaaccgctattttgaaacttgggcgtatcgagagatgctcaaggaatattttcaggcaggagctaagtggactgcagcgccgaagccacaattattcgacgcacagtatgacttcaatttccagtttcctcaactgggggagccgccgcgtttcgtcgttacagagtttgaaccgacttttgatgcggcagattttgtgcgctgtggacgagatatttttggtcaaaaaagtcatgtgactaatggtttgggcatagaatggttacaacgtcacttggaagacgaataccgtattcatattattgaatcgcattgtccggaagcactgcacatcgataccaccttaatgcctcttgcacctggcaaaatactagtaaatccagaatttgtagatgttaataaattgccaaaaatcctgaaaagctgggacattttggttgcaccttaccccaaccatatacctcaaaaccagctgagactggtcagtgaatgggcaggtttgaatgtactgatgttagatgaagagcgagtcattgtagaaaaaaaccaggagcagatgattaaagcactgaaagattggggatttaagcctattgtttgccattttgaaagctactatccatttttaggatcatttcactgtgcaacattagacgttcgccgacgcggaactcttcagtcctatttttaa

SEQ ID NO: 21 - DNA, 1134 bp, Cylindrospermopsis raciborskii T3
atgaccaatcagaacaaccaagagctggaaaatgatctgccgattgcaaaacagccgtgtccggttaatagctataatgaatgggataccctggaagaagttattgttggtagcgttgaaggtgcaatgctgcctgcactggaaccgattaacaaatggacctttccgtttgaagaactggaaagcgcacagaaaattctgagcgaacgtggtggtgttccgtatccgcctgaaatgattaccctggcacataaagaactgaacgagtttattcatatcctggaagccgaaggtgttaaagttcgtcgtgttaaaccggttgattttagcgttccgtttagcacaccggcatggcaggttggtagcggtttttgtgcagcaaatccgcgtgatgtttttctggttattggcaacgaaattatcgaagcaccgatggcagatcgtaatcgttattttgaaacctgggcatatcgcgaaatgctgaaagaatattttcaggcaggcgcaaaatggaccgcagcaccgaaaccgcagctgtttgatgcacagtatgatttcaattttcagtttccgcagctgggtgaaccgcctcgttttgttgttaccgaatttgaaccgacctttgatgcagccgattttgttcgttgtggtcgtgatatttttggccagaaaagccatgttaccaatggtctgggtattgaatggctgcagcgtcatctggaagatgaatatcgcattcatatcatcgaaagccattgtccggaagcactgcatattgataccaccctgatgccgctggcaccgggtaaaattctggttaatccggaatttgtggacgtgaataaactgccgaaaattctgaaaagctgggatattctggttgcaccgtatccgaatcatattccgcagaatcagctgcgtctggttagcgaatgggcaggtctgaatgttctgatgctggatgaagaacgtgtgatcgtggaaaaaaatcaagagcagatgatcaaagccctgaaagattggggttttaaaccgattgtttgccacttcgaaagctattatccgtttctgggtagctttcattgtgcaaccctggatgttcgtcgtcgtggcaccctgcagagctatttttga

SEQ ID NO: 22 - protein, 334 aa, Cylindrospermopsis raciborskii T3
MTTADLILINNWYVVAKVEDCKPGSITTALLLGVKLVLWRSREQNSPIQIWQDYCPHRGVALSMGEIVNNTLVCPYHGWRYNQAGKCVHIPAHPDMTPPASAQAKIYHCQERYGLVWVCLGDPVNDIPSLPEWDDPNYHNTCTKSYFIQASAFRVMDNFIDVSHFPFVHDGGLGDRNHAQIEEFEVKVDKDGISIGNLKLQMPRFNSSNEDDSWTLYQRISHPLCQYYITESSEIRTADLMLVTPIDEDNSLVRMLVTWNRSEILESTVLEEFDETIEQDIPIIHSQQPARLPLLPSKQINMQWLSQEIHVPSDRCTVAYRRWLKELGVTYGVC

SEQ ID NO: 23 - DNA, 1005 bp, Cylindrospermopsis raciborskii T3
atgacaactgctgacctaatcttaattaacaactggtacgtagtcgcaaaggtggaagattgtaaaccaggaagtatcaccacggctcttttattgggagttaagttggtactatggcgcagtcgtgaacagaattcccccatacagatatggcaagactactgccctcaccgaggtgtggctctgtctatgggagaaattgttaataatactttggtttgtccgtatcacggatggagatataatcaagcaggtaaatgcgtacatatcccggctcaccctgacatgacacccccagcaagtgcccaagccaagatctatcattgccaggagcgatacggattagtatgggtgtgcttaggtgatcctgtcaatgatataccttcattacccgaatgggacgatccgaattatcataatacttgtactaaatcttattttattcaagctagtgcgtttcgtgtaatggataatttcatagatgtatctcattttccttttgtccacgacggtgggttaggtgatcgcaaccacgcacaaattgaagaatttgaggtaaaagtagacaaagatggcattagcataggtaaccttaaactccagatgccaaggtttaacagcagtaacgaagatgactcatggactctttaccaaaggattagtcatcccttgtgtcaatactatattactgaatcctctgaaattcggactgcggatttgatgctggtaacaccgattgatgaagacaacagcttagtgcgaatgttagtaacgtggaaccgctccgaaatattagagtcaacggtactagaggaatttgacgaaacaatagaacaagatattccgattatacactctcaacagccagcgcgtttaccactgttaccttcaaagcagataaacatgcaatggttgtcacaggaaatacatgtaccgtcagatcgatgcacagttgcctatcgtcgatggctaaaggaactgggcgttacctatggtgtttgttaa

SEQ ID NO: 24 - DNA, 1005 bp, Cylindrospermopsis raciborskii T3
atgacgaccgcagatctgattctgatcaataattggtatgttgtggccaaggtggaagattgtaaaccgggtagcattaccaccgcactgctgctgggtgttaaactggttctgtggcgtagccgtgaacagaatagcccgattcagatttggcaggattattgtccgcatcgtggtgttgcactgagcatgggtgaaattgtgaataataccctggtttgtccgtatcatggttggcgttataatcaggcaggtaaatgtgttcatattccggcacatccggatatgacccctccggcaagcgcacaggcaaaaatctatcattgtcaagaacgttatggtctggtttgggtttgtctgggtgatccggttaatgatattccgagtctgccggaatgggatgatccgaattatcataatacctgcaccaagagctactttatccaggcaagcgcatttcgtgtgatggataactttattgatgtgagccattttccgtttgtgcatgatggtggtctgggcgatcgtaatcatgcacagattgaagaatttgaggtgaaagtggataaagacggtattagcattggcaatctgaaactgcagatgcctcgttttaatagcagcaatgaagatgatagctggaccctgtatcagcgtattagccatccgctgtgtcagtattatatcaccgaaagcagcgaaattcgtacagcagatctgatgctggttaccccgattgatgaagataattcactggttcgtatgctggtgacctggaatcgtagcgaaattctggaaagcaccgttctggaagaatttgatgaaaccattgaacaggatatcccgattattcatagccagcagcctgcacgtctgccgctgctgccgagcaagcagattaatatgcagtggctgagccaagaaattcatgttccgagcgatcgttgtaccgttgcatatcgtcgttggctgaaagaactgggcgttacctatggtgtttgttga

SEQ ID NO: 25 - protein, 612 aa, Cylindrospermopsis raciborskii T3
MQILGISAYYHDSAAAMVIDGEIVAAAQEERFSRRKHDAGFPTGAITYCLKQVGTKLQYIDQIVFYDKPLVKFERLLETYLAYAPKGFGSFITAMPVWLKEKLYLKTLLKKELALLGECKASQLPPLLFTSHHQAHAAAAFFPSPFQRAAVLCLDGVGEWATTSVWLGEGNKLTPQWEIDFPHSLGLLYSAFTYYTGFKVNSGEYKLMGLAPYGEPKYVDQILKHLLDLKEDGTFRLNMDYFNYTVGLTMTNHKFHSMFGGPPRQAEGKISQRDMDLASSIQKVTEEVILRLARTIKKELGVEYLCLAGGVGLNCVANGRILRESDFKDIWIQPAAGDAGSAVGAALAIWHEYHKKPRTSTAGDRMKGSYLGPSFSEAEILQFLNSVNIPYHRCVDNELMARLAEILDQGNVVGWFSGRMEFGPRALGGRSIIGDSRSPKMQSVMNLKIKYRESFRPFAPSVLAERVSDYFDLDRPSPYMLLVAQVKENLHIPMTQEQHELFGIEKLNVPRSQIPAVTHVDYSARIQTVHKETNPRYYELIRHFEARTGCAVLVNTSFNVRGEPIVCTPEDAYRCFMRTEMDYLVMENFLLVKSEQPRGNSDESWQKEFELD

SEQ ID NO: 26 - DNA, 1839 bp, Cylindrospermopsis raciborskii T3
atgcagatcttaggaatttcagcttactaccacgatagtgctgccgcgatggttatcgatggcgaaattgttgctgcagctcaggaagaacgtttctcaagacgaaagcacgatgctgggtttccgactggagcgattacttactgtctaaaacaagtaggaaccaagttacaatatatcgatcaaattgttttttacgacaagccattagtcaaatttgagcggttgctagaaacatatttagcatatgccccaaagggatttggctcgtttattactgctatgcccgtttggctcaaagaaaagctttacctaaaaacacttttaaaaaaagaattggcgcttttgggggagtgcaaagcttctcaattgcctcctctactgtttacctcacatcaccaagcccatgcggccgctgctttttttcccagtccttttcagcgtgctgccgttctgtgcttagatggtgtaggagagtgggcaactacttctgtctggttgggagaaggaaataaactcacaccacaatgggaaattgattttccccattccctcggtttgctttactcagcgtttacctactacactgggttcaaagttaactcaggtgagtacaaactcatgggtttagcaccctacggggaacccaaatatgtggaccaaattctcaagcatttgttggatctcaaagaagatggtacttttaggttgaatatggactacttcaactacacggtggggctaaccatgaccaatcataagttccatagtatgtttggaggaccaccacgccaggcggaaggaaaaatctcccaaagagacatggatctggcaagttcgatccaaaaggtgactgaagaagtcatactgcgtctggctagaactatcaaaaaagaactgggtgtagagtatctatgtttagcaggtggtgtcggtctcaattgcgtggctaacggacgaattctccgagaaagtgatttcaaagatatttggattcaacccgcagcaggagatgccggtagtgcagtgggagcagctttagcgatttggcatgaataccataagaaacctcgcacttcaacagcaggcgatcgcatgaaaggttcttatctgggacctagctttagcgaggcggagattctccagtttcttaattctgttaacataccctaccatcgatgcgttgataacgaacttatggctcgtcttgcagaaattttagaccagggaaatgttgtaggctggttttctggacgaatggagtttggtccgcgtgctttgggtggccgttcgattattggcgattcacgcagtccaaaaatgcaatcggtcatgaacctgaaaattaaatatcgtgagtccttccgtccatttgctccttcagtcttggctgaacgagtctccgactacttcgatcttgatcgtcctagtccttatatgcttttggtagcacaagtcaaagagaatctgcacattcctatgacacaagagcaacacgagctatttgggatcgagaagctgaatgttcctcgttcccaaattcccgcagtcactcacgttgattactcagctcgtattcagacagttcacaaagaaacgaatcctcgttactacgagttaattcgtcattttgaggcacgaactggttgtgctgtcttggtcaatacttcgtttaatgtccgcggcgaaccaattgtttgtactcccgaagacgcttatcgatgctttatgagaactgaaatggactatttggttatggagaatttcttgttggtcaaatctgaacagccacggggaaatagtgatgagtcatggcaaaaagaattcgagttagattaa

SEQ ID NO: 27 - DNA, 1839 bp, Cylindrospermopsis raciborskii T3
atgcagattctgggtatcagcgcctattatcatgatagcgcagcagcaatggttattgatggtgaaattgttgcagcagcacaagaagaacgttttagccgtcgtaaacatgatgcaggttttccgaccggtgcaattacctattgtctgaaacaggttggcaccaaactgcagtatattgatcagatcgtgttctatgataaaccgctggtgaaatttgaacgtctgctggaaacctatctggcctatgcaccgaaaggttttggtagttttattaccgcaatgccggtgtggctgaaagagaaactgtatctgaaaaccctgctgaaaaaagaactggcactgctgggtgaatgtaaagcaagccagctgcctccgctgctgtttaccagccatcatcaggcacatgcagcagcagcattttttccgagcccgtttcagcgtgcagcagttctgtgtctggatggtgttggtgaatgggcaaccaccagtgtttggctgggtgaaggtaataaactgacaccgcagtgggaaattgattttccgcatagcctgggcctgctgtatagcgcatttacctattataccggctttaaagtgaacagcggtgagtataaactgatgggtctggcaccgtatggtgaaccgaaatatgttgatcagattctgaaacatctgctggatctgaaagaagatggcacctttcgtctgaacatggattatttcaattataccgttggtctgaccatgaccaaccataaatttcatagcatgtttggtggtccgcctcgtcaggcagaaggtaaaattagccagcgtgatatggatctggcaagcagcattcagaaagttaccgaagaagtgattctgcgtctggcacgtaccattaagaaagaattaggtgttgaatacctgtgtctggcaggcggtgttggtctgaattgtgttgcaaatggtcgtattctgcgtgagagcgattttaaagatatttggattcagcctgcagccggtgatgcaggtagcgcagttggtgcagcactggcaatttggcatgaatatcataaaaaaccgcgtaccagcaccgcaggcgatcgtatgaaaggtagctatctgggtccgagctttagcgaagcagaaattctgcagtttctgaacagcgtgaatattccgtatcatcgttgtgtggataatgaactgatggcacgtctggcggaaattctggatcagggtaatgttgttggttggtttagcggtcgtatggaatttggtccgcgtgcactgggtggtcgtagcattattggtgatagccgtagcccgaaaatgcagagcgttatgaatctgaaaatcaaatatcgcgaaagcttccgtccgtttgcaccgagcgttctggcagaacgtgttagcgattattttgatctggatcgtccgagcccgtatatgctgctggttgcacaggttaaagaaaatctgcatattccgatgacccaagaacagcatgaactgtttggtatcgaaaaactgaatgttccgcgtagccagattccggcagttacccatgttgattatagcgcacgtattcagaccgttcataaagaaaccaatccgcgttattatgaactgatccgtcattttgaagcacgtaccggttgtgcagttctggttaataccagctttaatgttcgtggtgaaccgattgtgtgtacaccggaagatgcatatcgttgttttatgcgtaccgagatggattacctggtgatggaaaattttctgctggtgaaaagcgaacagcctcgtggtaatagtgatgaaagctggcagaaagaatttgagctggattga

SEQ ID NO: 28 - protein, 147 aa, Cylindrospermopsis raciborskii T3
MSEFFPQKSGKLKMEQIKELDKKGLREFGLIGGSIVAVLFGFLLPVIRHHSLSVIPWVVAGFLWIWAIIAPTTLSFIYQIWMRIGLVLGWIQTRIILGVLFYIMITPIGFIRRLLNQDPMTRIFEPELPTYRQLSKSRTTQSMEKPF

SEQ ID NO: 29 - DNA, 405 bp, Cylindrospermopsis raciborskii T3
atggaacagataaaagaacttgacaaaaaaggattgcgtgagtttggactgattggcggttctatagtggcggttttattcggctttttactgccagttatacgccatcattccttatcagttatcccttgggttgttgctggatttctctggatttgggcaataatcgcacctacgactttaagttttatttaccaaatatggatgaggattggacttgttttaggatggatacaaacacgaattattttgggagttttattttatataatgatcacaccaataggattcataagacggctgttgaatcaagatccaatgacgcgaatcttcgagccagagttgccaacttatcgccaattgagtaagtcaagaactacacaaagtatggagaaaccattctaa

SEQ ID NO: 30 - DNA, 405 bp, Cylindrospermopsis raciborskii T3
atggaacaaattaaagaactggataagaaaggcctgcgtgaatttggtctgattggtggtagcattgttgccgttctgtttggttttctgctgccggttattcgtcatcatagcctgagcgttattccgtgggttgttgcaggttttctgtggatttgggcaattattgcaccgaccaccctgagctttatctatcagatttggatgcgtattggtctggtgctgggttggattcagacccgtattattctgggtgttctgttctatattatgattaccccgatcggttttattcgtcgtctgctgaatcaggatccgatgacccgtatttttgaaccggaactgccgacctatcgtcagctgagcaaaagccgtaccacccagagcatggaaaaaccgttctga

SEQ ID NO: 31 - protein, 54 aa, Cylindrospermopsis raciborskii T3
MLKDTWDFIKDIAGFIKEQKNYLLIPLIITLVSLGALIVFAQSSAIAPFIYTLF

SEQ ID NO: 32 - DNA, 165 bp, Cylindrospermopsis raciborskii T3
atgctaaaagacacttgggattttattaaagacattgccggatttattaaagaacaaaaaaactatttgttgattcccctaattatcaccctggtatccttgggggcgctgattgtctttgctcaatcttctgcgatcgcacctttcatttacactcttttttaa

SEQ ID NO: 33 - DNA, 165 bp, Cylindrospermopsis raciborskii T3
atgttaaaagacacctgggattttatcaaggatatcgcaggctttatcaaagaacagaaaaactatctgctgattccgctgattattaccctggttagcctgggtgcactgattgtttttgcacagagcagcgcaattgcaccgtttatctataccctgttttga

SEQ ID NO: 34 - protein, 432 aa, Cylindrospermopsis raciborskii T3
MSNFKGSVKIALMGILIFCGLIFGVAFVEIGLRIAGIEHIAFHSIDEHRGWVGRPHVSGWYRTEGEAHIQMNSDGFRDREHIKVKPENTFRIALLGDSFVESMQVPLEQNLAAVIEGEISSCIALAGRKAEVINFGVTGYGTDQELITLREKVWDYSPDIVVLDFYTGNDIVDNSRALSQKFYPNELGSLKPFFILRDGNLVVDASFINTDNYRSKLTWWGKTYMKIKDHSRILQVLNMVRDALNNSSRGFSSQAIEEPLFSDGKQDTKLSGFFDIYKPPTDPEWQQAWQVTEKLISSMQHEVTAKKADFLVVTFGGPFQREPLVRQKEMQELGLTDWFYPEKRITRLGEDEGFSVLNLSPNLQVYSEQNNACLYGFDDTQGCVGHWNALGHQVAGKMIASKICQQQMRESILPHKHDPSSQSSPITQSVIQ

SEQ ID NO: 35 - DNA, 1299 bp, Cylindrospermopsis raciborskii T3
atgagtaacttcaagggttcggtaaagatagcattgatgggaatattgattttttgtgggctaatctttggcgtagcatttgttgaaattgggttacgtattgccgggatcgaacacatagcattccatagcattgatgaacacagggggtgggtagggcgacctcatgtttccgggtggtatagaaccgaaggtgaagctcacatccaaatgaatagtgatggctttcgagatcgagaacacatcaaggtcaaaccagaaaataccttcaggatagcgctgttgggagattcctttgtagagtccatgcaagtaccgttggagcaaaatttggcagcagttatagaaggagaaatcagtagttgtatagctttagctggacgaaaggcggaagtgattaattttggagtgactggttatggaacagaccaagaactaattactctacgggagaaagtttgggactattcacctgatatagtagtgctagatttttatactggcaacgacattgttgataactcccgtgcgctgagtcagaaattctatcctaatgaactaggttcactaaagccgttttttatacttagagatggtaatctggtggttgatgcttcgtttatcaatacggataattatcgctcaaagctgacatggtggggcaaaacttatatgaaaataaaagaccactcacggattttacaggttttaaacatggtacgggatgctcttaacaactctagtagagggttttcttctcaagctatagaggaaccgttatttagtgatggaaaacaggatacaaaattgagcgggttttttgatatctacaaaccacctactgaccctgaatggcaacaggcatggcaagtcacagagaaactgattagctcaatgcaacacgaggtgactgcgaagaaagcagattttttagttgttacttttggcggtccctttcaacgagaacctttagtgcgtcaaaaagaaatgcaagaattgggtctgactgattggttttacccagagaagcgaattacacgtttgggtgaggatgaggggttcagtgtactcaatctcagcccaaatttgcaggtttattctgagcagaacaatgcttgcctatatgggtttgatgatactcaaggctgtgtagggcattggaatgctttaggacatcaggtagcaggaaaaatgattgcatcgaagatttgtcaacagcagatgagagaaagtatattgcctcataagcacgacccttcaagccaaagctcacctattacccaatcagtgatccaataa

SEQ ID NO: 36 - DNA, 1299 bp, Cylindrospermopsis raciborskii T3
atgagcaacttcaaaggcagcgttaaaattgcactgatgggcattctgattttttgcggtctgatttttggtgtggcctttgttgaaattggtctgcgtattgcaggcattgaacatattgcctttcatagcattgatgaacatcgtggttgggttggtcgtccgcatgttagcggttggtatcgtaccgaaggtgaagcacatattcagatgaatagtgatggttttcgtgatcgcgaacacattaaagtgaaaccggaaaatacctttcgtattgccctgctgggtgatagctttgttgaaagcatgcaggttccgctggaacagaatctggcagcagttattgaaggcgaaattagcagctgtattgcactggcaggtcgtaaagccgaagttattaactttggtgttaccggttatggcaccgatcaagaactgattaccctgcgtgaaaaagtgtgggattatagtccggatattgttgtgctggatttctataccggtaacgatattgttgataatagccgtgcactgtcccagaaattctatccgaatgaactgggtagcctgaaaccgttttttatcctgcgtgatggtaatctggttgttgatgcaagctttatcaacaccgataactatcgtagcaaactgacctggtggggtaaaacctatatgaaaatcaaagatcatagccgcattctgcaggtcctgaatatggttcgtgatgcactgaataatagcagccgtggttttagcagccaggcaattgaagaaccgctgtttagtgatggtaaacaggataccaaactgagcggcttcttcgatatctataaaccgcctaccgatccggaatggcagcaggcctggcaggttaccgaaaaactgattagtagcatgcagcatgaagtgaccgccaaaaaagccgattttctggttgttacctttggcggtccgtttcagcgcgaaccgctggttcgtcagaaagaaatgcaagaactgggtctgaccgattggttttatccggaaaaacgtattacccgtctgggtgaagatgaaggttttagcgtgctgaatctgagcccgaatctgcaggtttatagcgaacagaataatgcctgtctgtatggttttgatgatacccagggttgtgttggtcattggaatgcactgggtcatcaggttgcaggtaaaatgattgcaagcaaaatttgtcagcagcagatgcgtgaaagcattctgccgcataaacatgatccgagcagccagagcagcccgattacccagagcgttattcagtaa

SEQ ID NO: 37 - protein, 482 aa, Cylindrospermopsis raciborskii T3
MTNTERGLAEITSTGYKSELRSEARVSLQLAIPLVLVEICGTSINVVDVVMMGLLGTQVLAAGALGAIAFLSVSNTCYNMLLSGVAKASEAFGANKIDQVSRIASGQIWLALTLSLPAMLLLWYMDTILVLFGQVESNTLIAKTYLHSIVWGFPAAVGILILRGIASAVNVPQLVTVTMLVGLVLNAPANYVLMFGKFGLPELGLAGIGWASTLVFWISFLVGVVLLIFSPKVRDYKLFRYLHQFDRQTVVEIFQTGWPMGFLLGVESVVLSLTAWLTGYLGTVTLAAHEIAIQTAELAIVIPLGIGNVAVTRVGQTIGEKNPLGARRAALIGIMIGGIYASLVAVIFWLFPYQIAGLYLKINDPESMEAVKTATNFLFLAGLFQFFHSVQIIVVGVLIGLQDTFIPLLMNLVGWGLGLAVSYYMGIILCWGGMGIWLGLVLSPLLSGLILMVRFYQEIANRIANSDDGQESISIDNVEELS

SEQ ID NO: 38 - DNA, 1449 bp, Cylindrospermopsis raciborskii T3
atgacaaataccgaaagaggattagcagaaataacatcaacaggatataagtcagagcttagatcggaggcacgagttagcctccaactggcaattcccttagtccttgtcgaaatatgcggaacgagtattaatgtggtggatgtagtcatgatgggcttacttggtactcaagttttggctgctggtgccttgggtgcgatcgcttttttatctgtatcgaatacttgttataatatgcttttgtcgggggtagcaaaggcatctgaggcttttggggcaaacaaaatagatcaggttagtcgtattgcttctgggcaaatatggctggcactcaccttgtctttgcctgcaatgcttttgctttggtatatggatactatattggtgctatttggtcaagttgaaagcaacacattaattgcaaaaacgtatttacactcaattgtgtggggatttccggcggcagttggtattttgatattaagaggcattgcctctgctgtgaacgtcccccaattggtaactgtgacgatgctagtagggctggtcttgaatgccccggccaattatgtattaatgttcggtaaatttggtcttcctgaacttggtttagctggaataggctgggcaagtactttggttttttggattagttttctagtgggggttgtcttgctgattttctccccaaaagttagagattataaacttttccgctacttgcatcagtttgatcgacagacggttgtggaaatttttcaaactggatggcctatgggttttctactgggagtggaatcagtagtattgagcctcaccgcttggttaacaggctatttgggaacagtaacattagcagctcatgagatcgcgatccaaacagcagaactggcgatagtgataccactcggaatcgggaatgttgccgtcacgagagtaggtcagactataggagaaaaaaaccctttgggtgctagaagggcagcattgattgggattatgattggtggcatttatgccagtcttgtggcagtcattttctggttgtttccatatcagattgcgggactttatttaaaaataaacgatccagagagtatggaagcagttaagacagcaactaattttctcttcttggcgggattattccaattttttcatagcgttcaaataattgttgttggggttttaatagggttgcaggatacgtttatcccattgttaatgaatttggtaggctggggtcttggcttggcagtaagctattacatgggaatcattttatgttggggaggtatgggtatctggttaggtctggttttgagtccactcctgtccggacttattttaatggttcgtttttatcaagagattgccaataggattgccaatagtgatgatgggcaagagagtatatctattgacaacgttgaagaactctcctga

SEQ ID NO: 39 - DNA, 1449 bp, Cylindrospermopsis raciborskii T3
atgaccaataccgaacgtggtctggccgaaattaccagcaccggttataaaagcgaactgcgtagcgaagcccgtgttagcctgcagctggcaattcctctggttctggttgaaatttgtggcaccagcattaatgttgttgatgttgtgatgatgggtttactgggtacacaagtgttagcagcgggtgccctgggagcaattgccttcctgagcgttagcaatacctgctataatatgctgctgagtggtgttgcaaaagcaagcgaagcctttggagccaataaaatcgatcaggtttcacgtattgcctcaggccagatttggttagccctgaccctgtcattaccagccatgctgttactgtggtatatggataccatcctggttctgtttggtcaggttgaaagcaataccctgattgcgaaaacatacctgcattcaattgtgtggggctttcctgccgcagttggtatcctgattctgcgtggcatagcaagtgcagttaacgttcctcagctggttaccgtgaccatgctggttggcctggtgctgaatgcaccggctaattatgtgctgatgttcggcaaattcggtttaccggaattaggcctggctggcattggctgggccagcacactggtgttttggattagttttctggttggtgttgtgctgctgatattttcaccgaaagttcgcgactacaaactgttccgctatttacatcagtttgatcgtcagaccgtggttgagatttttcagacgggctggcctatgggcttcctgctgggtgtggaaagcgttgttctgagcctgaccgcatggctgaccggctatctgggtacagtgaccttagcagcccatgaaattgcaatccagactgccgaactggcgattgtgattccgttaggtattggcaatgttgccgttacccgtgtgggccagacaatcggcgaaaaaaacccgctgggagcacgccgtgcagccctgattggcattatgattggtggcatttatgcgagcctggttgcagtgattttttggttattcccttatcaaatcgcaggcctgtacctgaaaattaacgatccggaatcaatggaagcagttaaaaccgcaacaaactttctgtttttagctggcctgttccagttttttcatagcgtgcagattattgttgtgggtgttctgattggcctgcaggatacctttatccctctgctgatgaatctggtgggctggggactgggcctggcggtttcctattatatgggtattatcctgtgctggggtggcatgggcatctggttaggtctggtactgtcaccgctgctgtcaggcctgatcctgatggtgcgcttttatcaagaaattgccaatcgcattgcgaatagcgacgatggccaagaaagcattagcattgataatgttgaagaactgagctaa

SEQ ID NO: 40 - protein, 276 aa, Cylindrospermopsis raciborskii T3
MKTNKHIAMWACPRSRSTVITRAFENLDGCVVYDEPLEAPNVLMTTYTMSNSRTLAEEDLKQLILQNNVETDLKKVIEQLTGDLPDGKLFSFQKMITGDYRSEFGIDWAKKLTNFFLIRHPQDIIFSFDIAERKTGITEPFTQQNLGMKTLYEVFQQIEVITGQTPLVIHSDDIIKNPPSALKWLCKNLGLAFDEKMLTWKANLEDSNLKYTKLYANSASGSSEPWFETLRSTKTFLAYEKKEKKLPARLIPLLDESIPYYEKLLQHCHIFEWSEH

SEQ ID NO: 41 - DNA, 831 bp, Cylindrospermopsis raciborskii T3
atgaaaacaaacaaacatatagctatgtgggcttgtcctagaagtcgttctactgtaattacccgtgcttttgagaacttagatgggtgtgttgtttatgatgagcctctagaggctccgaatgtcttgatgacaacttacacgatgagtaacagtcgtacgttagcagaagaagacttaaagcaattaatactgcaaaataatgtagaaacagacctcaagaaagttatagaacaattgactggagatttaccggacggaaaattattctcatttcaaaaaatgataacaggtgactatagatctgaatttggaatagattgggcaaaaaagctaactaacttctttttaataaggcatccccaagatattattttttctttcgatatagcggagagaaagacaggtatcacagaaccattcacacaacaaaatcttggcatgaaaacactttatgaagttttccaacaaattgaagttattacagggcaaacacctttagttattcactcagatgatataattaaaaaccctccttctgctttgaaatggctgtgtaaaaacttagggcttgcatttgatgaaaagatgctgacatggaaagcaaatctagaagactccaatttaaagtatacaaaattatatgctaattctgcgtctggcagttcagaaccttggtttgaaactttaagatcgaccaaaacatttctcgcctatgaaaagaaggagaaaaaattaccagctcggttaatacctctactagatgaatctattccttactatgaaaaactcttacagcattgtcatatttttgaatggtcagaacactga

SEQ ID NO: 42 - protein, 257 aa, Cylindrospermopsis raciborskii T3
MSFQKFVQEAAYKVAPFKPNRFAKISEREDKCAIPVPAWRALLANRDLFTWKGIPFLKGCTEIALYSMLLYELRPKTIIEIGALSGGSAIWLADHLELFQIEGCVYCIDIDLSLLDEKAKTDSRVHFLEGDCNNMGAIMSSELLSGLAHPWLIVEDAHANAVGVVEYFHENGLKSGDYLIVEDTNKTMWELDREELDRDDLDEQELIEKGEQKLAELKSWLMLHENEYLIDTYYQDMYGYNGSRNWNSILKRVEKNF

SEQ ID NO: 43 - DNA, 774 bp, Cylindrospermopsis raciborskii T3
atgagcttccaaaaatttgttcaagaagccgcctataaagttgcacctttcaaacctaatcggtttgccaaaatttctgaaagagaagataaatgtgctattccagtgccagcttggagagcgctcttggcaaaccgcgatttgttcacttggaaagggatacccttcctgaaagggtgcaccgaaatagctctttattcaatgctcctgtatgagcttcgcccgaaaacaataatcgaaataggagcattaagcggtggcagcgcgatttggctagccgatcacttagaactgttccaaatagaaggttgtgtctactgtatcgatatcgatctttccctactcgacgagaaagcaaaaactgactctcgcgttcattttttagagggggattgtaacaatatgggtgcaataatgtcgtcggaactgctttctgggcttgctcatccctggttgatcgtagaagatgcccatgctaatgcggtgggagtagttgaatattttcacgaaaacggtctaaaaagtggagactacttgattgtcgaagataccaacaaaactatgtgggagttggacagggaggagttggacagggatgatttggatgagcaagaattaatagaaaaaggagagcagaaattagcggagttaaaaagctggttaatgctccacgaaaatgagtacctcatcgatacgtactatcaagatatgtacggttacaacggctctagaaactggaattctatcctgaaaagagtagaaaaaaatttttag

SEQ ID NO: 44 - DNA, 774 bp, Cylindrospermopsis raciborskii T3
atgtcatttcagaaatttgtgcaagaagcagcctataaagtcgcaccgtttaaaccgaatcgttttgccaaaattagcgagcgtgaagataaatgtgcaattccggttccggcatggcgtgcactgctggccaatcgtgacctgtttacctggaaaggtattccgtttctgaaaggttgtaccgaaattgcactgtatagcatgctgctgtatgaactgcgtccgaaaacgattattgaaattggtgcgctgagcggtggtagcgcaatttggctggcagatcatctggaactgtttcagattgaaggttgcgtgtattgcattgatattgatctgtctctgctggacgaaaaagcaaaaaccgatagccgtgttcattttctggaaggtgattgcaataatatgggtgcaattatgtcaagcgagctgctgagtggtctggcacatccttggctgattgttgaagatgcacatgcaaatgccgttggtgtggttgaatattttcacgaaaacggtctgaaaagtggcgattacctgatcgtggaagataccaataaaacaatgtgggaactggatcgcgaagaactggaccgtgatgacctggatgaacaagaactgatcgaaaaaggtgagcagaaattagcagaactgaaaagctggctgatgctgcatgagaatgaatatctgatagatacctactatcaggatatgtatggctataatggtagccgtaattggaacagcattctgaaacgtgtggaaaagaacttttaa

SEQ ID NO: 45 - protein, 108 aa, Cylindrospermopsis raciborskii T3
MIELVSHKLCINCNVCVQVCPTNVFDAVPNQPPAIARQEDCQTCFICEAYCPADALYVAPQSHTNVAVNEDDLIDSGIMGEYRRILGWGYGRKNNSELDTDHKLRLFE

SEQ ID NO: 46 - DNA, 327 bp, Cylindrospermopsis raciborskii T3
atgatcgagcttgtcagccataaactctgtattaattgtaatgtttgcgtccaagtatgccctaccaatgtctttgatgcagttcccaaccaaccgcctgcgatcgcccgacaggaagactgtcaaacttgtttcatctgtgaagcatattgtcctgcggatgcgctctatgttgcgccgcaatctcataccaatgttgcagtcaacgaggatgatttaattgacagtggcattatgggtgaatatcgtcgcatcttaggttggggatatggcagaaaaaacaatagcgaattggataccgatcataaactacggctatttgaataa

SEQ ID NO: 47 - DNA, 327 bp, Cylindrospermopsis raciborskii T3
atgattgaactggtgagccataagctgtgcattaattgtaatgtttgtgttcaggtgtgcccgaccaatgtttttgatgcagtgccgaatcagcctccggcaattgcacgccaagaagattgtcagacctgttttatttgtgaagcatattgtcctgcagatgcgctgtatgttgcaccgcagagccataccaatgttgcagttaacgaagatgatttaatcgacagcggcattatgggtgaatatcgtcgcattctgggttggggctatggtcgtaaaaacaatagcgaactggataccgaccataaactgcgtctgtttgaatga

SEQ ID NO: 48 - protein, 550 aa, Cylindrospermopsis raciborskii T3
MNLTLNKEEKQLLTAYSGTELQLTADVLVIGGGPAAAWAAWAAGAQGVKVIIVDKGFLGTSGAAAASGNSVMAPSPENWEKDVSECYSKGNNLANLRWIERVIEKAWLSLPLVEDWGYRFPKENGESVRQSYYGPEYMRVLRKNLLRVGVQIFDQSPALELLLAQDGSVAGARGVQRQNHRTYTVRAGAVVLANGGCAFLSKALGCNTNTGDGLLMAVEAGGELSSMEASSHYTISTAFNATVTRAAPFYWASYTDEAGNDLGGYINGRRDPSFLPNALLKGPVYARLDRATPEIQALVEKSHFIAFLPYKKAGIDPYTERVPVTLVLEGTVRGTGGIRIVNDSCGTKVPGLYAAGDAASREFLAGIASGGDGPNAAWAISTGQWAGEGAAAFAKSLGAHVHERVVRPAGQAGLRSQYPGSETFDSEAVVRGVQAEMFPLEKNYLRCEQGLLDSLAKLEMLWQQVQGNPKQDTVRDLEFSRRAAALVSVARWAYFSALHRKETRSEHIRIDYPETDPNQLYYQATGGLERLWVRRDWVKDASATPPVLTT

SEQ ID NO: 49 - DNA, 1653 bp, Cylindrospermopsis raciborskii T3
atgaacttgactttaaacaaggaggaaaagcaattgcttacagcctatagcggcactgaactacaattaactgctgacgtgctggtaattggtggtggtcctgccgccgcatgggcagcatgggcggctggagcccaaggtgtcaaagtcatcattgttgataaaggttttctaggtacgagcggtgcagctgctgccagtggcaatagcgtcatggcaccttctccagagaattgggagaaagatgtatccgaatgttacagcaaaggaaataacctcgctaacttacgttggattgaacgtgtaattgaaaaagcttggctgagtttgcccttagtggaagattggggctatcgtttccccaaagaaaatggggaatccgtgcgccagagttattatggtccggaatatatgcgggtacttcgcaagaacctgttgcgtgtgggtgtgcaaattttcgaccaaagtccggctctagaactgttattagcccaggacggctccgtggctggagctagaggtgtacagaggcaaaatcatcgcacctataccgttcgcgctggtgcagtagttctagcgaatggcggttgtgcattcctaagtaaagctttaggttgcaataccaatacaggcgatggactgctgatggcggtggaagctggcggcgaactctccagtatggaagcttccagtcactataccatctcgaccgctttcaatgccacagtgacaagggctgctcccttttactgggctagttacaccgatgaggcaggtaacgatcttggtggctatatcaatggtcgtcgcgatccatcgttcctgcccaatgccctcctgaaaggtcccgtttatgctcgtttggatcgagccacacctgaaatccaagcattggttgaaaagtctcacttcatcgcctttctaccctataaaaaagctggcattgacccttatacagaacgagtacctgtaacactggttttagaaggtacagtccgtggtacaggtggaattcggattgtgaatgatagttgtggtacaaaagttcctggactgtatgccgccggagatgcagcatcgcgggagtttttagctgggatagcttctgggggtgatggtcctaatgctgcttgggcaatctctacaggacaatgggcaggggaaggtgcagccgcctttgccaagagtttgggcgctcatgtccatgaacgggttgtgcgtccagcaggtcaagccggattacgttcccagtaccctggttccgaaacattcgatagcgaggcagttgtccgcggtgtacaagccgagatgttcccattagagaagaattacttgcgctgtgagcagggacttttggattccctcgccaaattagaaatgctgtggcagcaagtacaagggaacccgaaacaagatacagtgcgcgatctggaattttctcgtcgagcggctgctcttgtgtctgtagcacgatgggcatattttagcgctttacatcgcaaggaaacgcgtagcgaacatattcgcatagactatcctgaaaccgatccaaatcagctttattaccaagccacgggcggcttagaaaggctttgggtgagacgggattgggtgaaggatgcgagcgctacaccaccagtattaaccacttaa

SEQ ID NO: 50 - DNA, 1653 bp, Cylindrospermopsis raciborskii T3
atgaacctgaccctgaacaaagaagaaaaacagctgctgacggcatatagcggcaccgaactgcagctgacagcagatgttctggttattggtggtggtccggcagccgcatgggcagcttgggcagcaggcgcacagggtgtgaaagttattattgtggataaaggttttctgggcaccagcggtgccgcagccgcaagcggtaatagcgttatggcaccgtcaccggaaaattgggaaaaagatgtgagcgaatgttacagcaaaggtaataatctggcaaatctgcgttggattgaacgtgttattgaaaaagcctggctgtcactgccgctggttgaagattggggttatcgttttcctaaagaaaatggtgaaagcgtgcgtcagagctattatggtcctgaatatatgcgtgttctgcggaaaaatctgctgcgcgttggtgttcagatctttgatcagtcaccggcactggaattactgctggcacaggatggtagcgttgccggtgcacgtggtgtgcagcgtcagaatcatcgtacatataccgttcgtgccggtgccgttgttctggccaatggtggttgcgcatttctgagtaaagcactgggttgtaataccaataccggtgatggtctgttaatggcagttgaagccggtggtgaactgagcagtatggaagccagcagccattataccattagcaccgcctttaatgcaaccgttacccgtgcagctccgttttattgggcaagctataccgatgaagctggcaatgatctgggtggctatattaacggtcgtcgtgatccgagctttctgccgaacgcactgctgaaaggtccggtttatgcacgtctggatcgtgcaacaccggaaattcaggcgctggtagaaaaaagccattttattgcatttctgccgtacaagaaagccggtattgatccgtataccgaacgtgttccggttaccctggtgctggaaggcaccgtgcgtggcaccggtggtattcgcattgttaatgattcatgtggcaccaaagttccgggactgtatgcagcgggtgatgcagcaagccgtgaatttctggcaggcattgccagcggtggtgatggaccgaatgcagcatgggcaatttcaaccggtcagtgggcaggcgaaggtgcagcagcctttgcaaaaagtctgggtgcacatgttcatgaacgcgttgttcgtccggcaggccaggcaggtctgcgtagtcagtatccgggtagcgaaacctttgatagtgaagcagttgttcgtggcgttcaggcagaaatgtttccgctggaaaaaaactatctgcgctgtgaacagggactgctggatagcctggcaaaactggaaatgctgtggcagcaggttcagggtaatccgaaacaggatacagttcgtgatctggaattttcacgtcgtgcggcagcactggttagcgtggcacgttgggcatattttagcgcactgcatcgtaaagaaacccgtagcgaacatatccgtattgattacccggaaacggatccgaatcaactgtattatcaggcaaccggtggcctggaacgtctgtgggtgcgtcgtgattgggttaaagatgcaagcgccacccctccggtgctgaccacctga

SEQ ID NO: 51 - protein, 249 aa, Cylindrospermopsis raciborskii T3
MAGKLDGKVAIITGASSGIGEATAFALAAEGAKVAIAARRAELLHALAKRIEASGGQALPIVTDITDESQVNHLVQKTKVELGHVDILVNNAGIGVFGAIDTGNPADWRRAFDVNVLGVLYAIHAVLPLLKAQKSGHIVNISSVDGRIAQSGAVVYSAAKSGVNALSEALRQEVSLDNIRVTIIEPGLVDTPFNDLISDPITKQLSKEQLSTITPLQSEDIARAIIYAVTQPDHVNVNEILIRPTAEDN

SEQ ID NO: 52 - DNA, 750 bp, Cylindrospermopsis raciborskii T3
atggcaggtaaattggatggaaaagtggcgattattactggagcttcctctgggattggagaggctacagcatttgctttagctgcggagggggcaaaagttgcgatcgccgcaagacgtgctgagcttttgcatgcactagcaaaacggattgaagccagtggtggtcaagcattgcctattgttacagatattacagacgaatctcaagtaaatcatctagtccaaaagaccaaggttgagctaggacatgtagatattttggtgaataatgcaggaattggtgtgtttggtgcaattgatactggaaatcccgcagactggaggcgagcattcgatgtgaatgttctgggagttttatatgctatccacgcagttttgcctcttctgaaggcccaaaaatccggtcatatagtcaatatatcttctgtcgatggcaggatagcgcagtccggtgcggtcgtttatagtgctgccaaatcaggcgtcaatgctctttcagaagcattacgccaggaggtatctttagacaacattcgcgttaccatcattgagccaggtttagtcgatacgccatttaatgacttaatttctgacccgatcacgaaacagcttagtaaagaacaacttagtacaataacacctttacaaagtgaggatattgcaagagctataatttatgcagtgacacaacccgatcatgtaaatgtaaatgaaattttgattcgaccgactgcagaagataattaa

SEQ ID NO: 53 - DNA, 750 bp, Cylindrospermopsis raciborskii T3
atggcaggtaaactggatggtaaggttgcaattattaccggtgcaagcagcggtattggtgaagccaccgcatttgcactggcagcagaaggtgcaaaagttgcaattgcagcccgtcgtgcagaactgttacatgcactggccaaacgtattgaagcaagcggtggtcaggcactgccgattgttaccgatatcaccgatgaaagccaggttaatcatctggttcagaaaaccaaagttgaactgggtcatgttgatatcctggtgaataatgcaggtattggcgtttttggtgcaatcgataccggtaatccggcagattggcgtcgtgcatttgatgttaatgtgctgggtgttctgtatgcaattcatgcagttctgcctttactgaaagcacagaaaagcggtcatattgtgaatattagcagcgtggatggtcgtattgcacagagcggtgcagttgtttatagcgcagcaaaaagcggtgttaatgccctgagcgaagcactgcgtcaagaagtgagcctggataatattcgtgtgaccattattgaaccgggtctggtagataccccgtttaatgatctgattagtgatccgattaccaaacagctgagcaaagaacagctgtcaaccattactccgctgcagagcgaagatattgcacgtgccattatctatgcagttacccagccggatcatgttaacgttaatgaaattctgattcgtccgaccgcagaggataattga

SEQ ID NO: 54 - protein, 334 aa, Cylindrospermopsis raciborskii T3
MTTTDPILINNWHVVANVEDCKPGSITRSRLLGVKLVLWRSYEQNSPIQVWLDYCPHRGVPLSMGEITNNTLVCPYHGWRYNEAGKCIQIPAHPGMVPPASAEARTYHSQERYGLVWVCLGDPVNDIPSFPEWDDPNYHKTYTKSYLIKASAFRVMDNSLDVSHFPFIHDGWLGDRNYTKVEEFEVKLDKDGLTMGKYQFQTSRIVSHIEDDSWVNWFRLSHPLCQYCVSESPEMRIVDLMTITPIDEENSVLRMLIMWNGYETLESKMLTEYDETIEQDIRILHAQQPVRLPLLTPKQINTQLFSHEIHVPSDRCTLAYRRWLKQLGVTYGVC

SEQ ID NO: 55 - DNA, 1005 bp, Cylindrospermopsis raciborskii T3
atgacaactaccgacccaatcttaatcaataactggcacgtagtcgccaatgtagaagactgtaaacctggaagtatcaccagatctcgtttgttgggagtgaagttggtattatggcgcagttatgaacaaaattcacccatacaggtatggcttgactactgcccccaccgaggtgttcctctgtctatgggagaaattacgaataatactttagtttgtccgtatcacggatggagatacaatgaggctggtaaatgcatacagatcccagctcaccctggcatggtaccaccggcaagtgctgaagccaggacatatcactcccaggagcgctatggcttagtgtgggtgtgcttgggcgatcctgttaatgatataccttcatttcctgaatgggatgatccgaattatcacaagacttataccaagtcttacttgattaaagctagtgcgtttcgtgtgatggataattccttagacgtgtctcattttccttttatccatgacggttggttaggtgatcgcaattatacaaaagtggaagaatttgaggtgaaattagataaagatggccttactatgggtaagtatcaattccagacatcaaggattgtcagccatatcgaagatgactcttgggttaattggttcaggcttagtcatcctttatgtcaatactgcgtttcagaatcccctgaaatgaggattgtggatttaatgacgatcacaccgattgatgaggaaaatagtgtattgcgtatgttgataatgtggaacgggtatgaaacgttagagtcaaagatgctaactgaatatgacgaaacaatagaacaagatattcggatcttacatgcacaacagccggtacgtttaccactgttaactccaaagcagataaatacacaattgttttcacacgaaatccacgtaccatcagatagatgcacacttgcctatcgtcgatggctaaagcaactaggtgttacttatggggtttgttaa

SEQ ID NO: 56 - DNA, 1005 bp, Cylindrospermopsis raciborskii T3
atgacaaccaccgatccgatcctgattaataactggcatgttgtggcaaatgtcgaggattgtaaaccgggtagcattacccgtagccgtttactgggtgttaaactggttctgtggcgtagctatgaacagaatagcccgattcaggtttggctggattattgtccgcatcgtggtgttccgctgagcatgggtgaaattaccaataataccctggtttgtccgtatcatggctggcgttataatgaagcaggtaaatgtattcagattccggcacatccgggtatggttccgcctgcaagcgcagaagcacgtacctatcatagccaagaacgttatggtctggtttgggtttgtctgggtgatccggttaatgatattccgtcatttccggaatgggatgatccgaattatcacaaaacctacaccaaaagctatctgattaaagcaagcgcctttcgcgttatggataattcactggatgttagccattttccgtttattcatgatggctggctgggcgatcgtaactataccaaagtggaagaatttgaagtgaaactggataaagatggtctgacgatgggcaaatatcagtttcagaccagccgtattgtgagccatattgaagatgatagctgggtgaattggtttcgtctgagccatccgctgtgtcagtattgtgttagcgaaagtccggaaatgcgtattgttgatctgatgaccattacgccgattgatgaagaaaatagcgttctgcgcatgctgatcatgtggaatggttatgaaaccctggaaagcaaaatgctgacagagtatgatgaaacgatcgaacaggatattcgtattctgcatgcccagcagccggtgcgtctgccgctgctgacaccgaagcagattaatacccagctgtttagccatgaaattcatgttccgagcgatcgttgtaccctggcatatcgtcgttggctgaaacaactgggtgtgacctatggtgtttgttga

SEQ ID NO: 57 - protein, 241 aa, Cylindrospermopsis raciborskii T3
MLTAEQKQAYTNDGYFTVEEAVPKALIEEIRHEVELITEQKRGGVLAGDYEWWSEHTIPDPVRYQKIIQRLLELPTVMGPVQALIGSDIFLLITDLAIIRAGTGYIAWHQDHGYVVEVLNALASMSKNELNDDALRLLVPVANQAMVFITIYLQDTDNTMGTMRVIPSSHQWEHSLDSSSANSLNAEICLSLPGGAAMFYTPTVWHTAAANTSITDYRMLTLIFTKNNIKPLLVDALKRII

SEQ ID NO: 58 - DNA, 726 bp, Cylindrospermopsis raciborskii T3
atgctcacagcggaacaaaaacaagcttacacaaatgatggttatttcacagttgaagaagctgtaccaaaagcgttaattgaagaaatacggcatgaagtagaacttattaccgaacaaaaacgtgggggagtattggcgggtgactatgagtggtggtctgagcatactatcccagatccagttaggtatcaaaagataattcagaggcttttagagcttccaactgtgatgggaccagtacaggctctaattgggtctgatatcttcctattgatcaccgatctagccataattcgtgcaggtacaggatacattgcttggcatcaagaccatggatatgtagttgaagtattgaacgcacttgcatccatgtcaaaaaacgagttaaatgacgacgcgcttcggttgttggttccagtagccaatcaagccatggtattcataactatatacttacaggatacagataatactatgggtacaatgcgagttataccaagtagccaccaatgggaacactcattagattcatcttctgccaattcactaaatgcagaaatatgtctttcacttccaggaggggcagcaatgttttatacaccaactgtatggcataccgcagctgccaacacttcaattaccgattacaggatgctaactctgatttttacaaaaaacaacatcaaaccactgttggtggatgccttgaaaaggataatttag

SEQ ID NO: 59 - DNA, 726 bp, Cylindrospermopsis raciborskii T3
atgctgaccgcagaacagaaacaggcatataccaatgatggctattttaccgtggaagaagcagttccgaaagcactgattgaagaaattcgccatgaagtggaactgatcaccgagcagaaacgtggtggtgtgctggcaggcgattatgaatggtggtcagaacacaccattccggatccggttcgttatcagaaaattatccagcgtctgctggaactgccgaccgttatgggtccggttcaggccctgattggtagcgatatttttctgttaattaccgacctggcaattattcgtgcaggcaccggttatattgcatggcatcaggatcatggctatgttgttgaagttctgaacgccctggcaagcatgagcaaaaatgagctgaatgatgatgcactgcgcctgctggtgccggttgcaaatcaggcaatggtgtttattaccatctatctgcaggataccgataacaccatgggcaccatgcgtgtgattccgagcagccatcagtgggaacatagtctggatagcagcagcgccaattcactgaatgcagaaatttgtctgagcctgcctggtggtgcagcaatgttttataccccgaccgtttggcataccgcagcagcaaataccagcattaccgattatcgtatgctgacgctgatcttcaccaaaaacaacattaaaccgctgctggttgatgccctgaaacgtattatttga

SEQ ID NO: 60 - protein, 191 aa, Cylindrospermopsis raciborskii T3
MINIEQFRQEIEDWIINVVSIPNPLTGNFPPCPYAKAAWLNNRVSVRWFHGPELPELLMEQIRTWNNDFEMVIFGCDPQNLDAQRLERYITKANYVLPEYDLVALGSHPDKQYVGDDAENVNNVIITHPKYVLASVQSFSQLQEASDELLRLGYFQYWSAEKLAEMKSERASHNLSSIQRKNSYRIIPTNH

SEQ ID NO: 61 - DNA, 576 bp, Cylindrospermopsis raciborskii T3
atgataaatatcgaacaatttcgccaagaaatagaggattggattatcaatgttgtcagcattcccaatcctctaacaggaaattttccaccctgtccttacgcgaaggcagcttggttaaataaccgtgttagtgttcgttggtttcatggacctgaactgccagagcttctaatggaacagataagaacatggaataatgactttgaaatggtgatttttggctgcgaccctcaaaacctagatgcacagaggttggaaaggtacattaccaaggcgaattatgtattaccagaatacgatttggtagctttaggatcgcatccagacaaacaatatgttggtgatgacgcggagaatgtgaataacgtaatcataactcaccctaagtatgttttagcatcagtacagtcattcagccagttacaagaggctagtgatgaattattaagattgggatattttcagtattggtctgcagaaaaattggctgaaatgaagtcggagcgagcttctcacaacctttcttctatccagagaaagaacagctataggataattcctactaaccattga

SEQ ID NO: 62 - DNA, 576 bp, Cylindrospermopsis raciborskii T3
atgatcaacatcgaacagtttcgccaagaaatcgaagattggattattaacgttgtcagcattccgaacccgctgaccggtaattttcctccgtgtccgtatgcaaaagcagcatggctgaataatcgtgttagcgtgcgttggtttcatggtccggaactgcctgaactgctgatggaacaaattcgtacatggaacaacgatttcgagatggtgatttttggttgcgatcctcagaatctggatgcacagcgtctggaacgttatatcaccaaagcaaattatgtgctgcccgaatatgacctggttgcactgggtagccatccggataaacagtatgttggtgatgatgccgaaaatgtgaacaacgtgattattacccatccgaaatatgttctggcaagcgttcagagctttagccagctgcaagaggcaagtgatgagctgctgcgtctgggttatttccagtattggtcagcagaaaaactggccgaaatgaaaagcgaacgtgcaagccataatctgagcagcattcagcgtaaaaatagctatcgtattatcccgaccaaccattga

SEQ ID NO: 63 - protein, 258 aa, Cylindrospermopsis raciborskii T3
MTIQIVQHNLEYSFVTPKETSDFVERTMSVFDQAYPKFLIHDVWADPASLALFEIYPEFQFGLVEATTQLMIAQGNCIPLTYESRFDELPDEGCDWALAKWLEDREQNRLPNALCVVSISILPEYQGKNLSQYLIGYMKELAQYHGLNSLIMAARPSLKYLYPLIPIERYITWRDKNGLIFDPWLRVNVKHGAKIAGICFKSTTINDTIDGWEDRVGMRFPETGDYIIPKGLVPVKIDYPNNMGIYIEPNIWLYYDLD

SEQ ID NO: 64 - DNA, 777 bp, Cylindrospermopsis raciborskii T3
atgaccattcaaattgtacagcataatttagagtatagctttgtaaccccaaaagaaacttctgattttgtggaaaggacgatgagtgtctttgatcaagcatacccaaaatttttgatacatgatgtctgggcagatccagcttccttagctctatttgaaatttatccagaattccagtttgggttagtagaagctaccacacagcttatgatagcgcaaggaaactgtatccctttaacttatgaaagccgttttgatgagttaccggacgaaggttgtgactgggctttagccaagtggcttgaagaccgagaacagaaccgcctgcctaatgcgttatgtgtagtatcgatttcaatcctaccagagtatcaaggcaaaaacttgagtcagtatctgattggatacatgaaagaacttgctcaataccacggtcttaattctttgatcatggctgcacgtccaagcctaaaatatctttacccacttatacccatagagcggtatattacctggcgagataaaaatggtcttatatttgacccttggttacgagttaatgtcaaacatggggctaaaattgcagggatctgttttaaatccacaacaattaatgatactattgacggttgggaagatagagttgggatgcgttttccagaaactggtgactatattattcccaaaggcttagtacctgtcaaaattgactatcccaacaatatgggaatatacatcgagcctaatatatggttatactatgacctagattaa

SEQ ID NO: 65 - DNA, 777 bp, Cylindrospermopsis raciborskii T3
atgaccatccagattgtgcagcataacctggaatatagctttgtgaccccgaaagaaaccagcgattttgttgaacgtaccatgagcgtttttgatcaggcatatccgaaatttctgatccatgatgtttgggcagatccggcaagcctggccctgtttgaaatttatccggaatttcagtttggtctggtggaagcaaccacccagctgatgattgcacagggtaattgtattccgctgacctatgaaagccgttttgatgaactgccggatgaaggttgtgattgggcactggcaaaatggctggaagatcgcgaacagaatcgtctgccgaatgccctgtgtgttgtgagcattagcatcctgccggaatatcagggtaaaaatctgagccagtatctgatcggctatatgaaagaactggcacagtatcatggtctgaatagcctgattatggcagcacgtccgagcctgaaatatctgtatccgctgattccgattgaacgctatattacctggcgtgataaaaacggcctgatttttgatccgtggctgcgtgttaatgttaaacatggcgcaaaaattgccggtatctgctttaaaagcaccaccattaatgataccattgatggttgggaggatcgtgttggtatgcgttttccggaaaccggtgattatatcattccgaaaggtctggttccggtgaaaattgattatccgaataacatgggcatctacatcgaaccgaatatctggctgtattatgatctggactga

SEQ ID NO: 66 - protein, 258 aa, Cylindrospermopsis raciborskii T3
MVIKNLCPDGVTPIWNKSQMESSLLEECLPAWVRTSYSTFVETISDSAFPCFWGTIGEQKGMIRYLIVSSLTDPILVEHTLEGIYKYIDEVNENELLQHENADLLTLVIFFPPEPTVLTVEEYAGQAFDFLNALHSLDAVSCPCHWSADPQSANWSYSLGGCALFVSVSTPANQKRRSRHLGSGMTFVITPVEVLLNKHGGENSSIFRRVRQYDGIPPHPNLLIMPGNGKVGNELTVQVLPDNNDSEISFDFQYKFKD

SEQ ID NO: 67 - DNA, 777 bp, Cylindrospermopsis raciborskii T3
atggtaatcaagaatttatgtcctgacggagttacaccaatctggaacaaaagccagatggaatcctctcttctagaggagtgccttcctgcttgggtacgcactagctactcaacatttgttgaaacaatcagcgattctgccttcccttgcttctggggaactatcggggaacagaagggaatgattagatacctgatagtctcatctttaactgacccgatcttggttgagcatacgcttgagggtatctacaaatacattgatgaagttaatgaaaacgaattgcttcagcacgaaaatgcggatcttctgacacttgtcatctttttcccacctgaaccaacagttcttacagtagaggaatatgcaggtcaagcatttgattttttgaatgcgttacatagccttgatgcggtgtcttgtccctgccattggtctgccgatccgcagtctgctaactggtcttattctctaggagggtgtgccttatttgttagtgtttccactccagcaaatcaaaagcggcgatcgcgccaccttgggtcaggaatgacttttgtcatcacaccagttgaagtcctcttgaataaacatggtggcgagaattcgagcatttttcgccgcgtccgagagtacgacggcattccacctcaccctaacttattaattatgcctgggaatgggaaagtcggtaatgaattgacagtgcaagtacttccagataataacgatagtgagatctcatttgacttccagtataaatttaaggattag

SEQ ID NO: 68 - DNA, 777 bp, Cylindrospermopsis raciborskii T3
atggtgattaaaaacctgtgtccggatggtgttaccccgatttggaataaaagccagatggaaagcagcctgctggaagaatgtctgcctgcatgggttcgtaccagctatagcacctttgttgaaaccattagcgatagcgcatttccgtgtttttggggcaccattggtgaacagaaaggtatgattcgttatctgattgttagcagcctgaccgatccgattctggttgaacataccctggaaggtatctacaaatatatcgatgaagtgaacgaaaacgaactgctgcagcatgaaaatgcagatctgctgaccctggttatcttttttccgcctgaaccgaccgttctgaccgttgaagaatatgcaggtcaggcatttgattttctgaatgcactgcatagcctggatgcagttagctgtccgtgtcattggagcgcagatccgcagagcgcaaattggagctatagcctgggtggttgtgcactgtttgttagcgttagcacaccggcaaatcagaaacgtcgtagccgtcatctgggtagcggtatgacctttgttattacaccggttgaagtgctgctgaataaacatggtggtgaaaacagcagcatttttcgtcgtgttcgtgaatatgatggtattccgcctcatccgaatctgctgattatgcctggtaatggtaaagtgggtaatgaactgaccgtgcaggttctgccggataataatgatagcgaaatcagcttcgattttcagtataaattcaaagattga

SEQ ID NO: 69 - protein, 408 aa, Cylindrospermopsis raciborskii T3
MKRLTLLIIAGILSVSTFLCITPVALANITDYYLKNEKLSGQFSVPVNLSVGVRFAHRSSYATAINFPTGLDADSVAVGDFNSDSKLDLAVTNWFDNNVSVLLGNGNGSFGAATNFPVGTNPVFVVTGDVNGDSKLDLAVANFSSNNVSVLLGNGNGSFGAATNFSVGTNPYSVAIGDVNNDSELDLAFTNWFDNKVLVLLGNGNGSFGAASSFPVDTYSISVAIADFNSDSKLDLAITNWVSNNVSVLLGNGNGSFGAATNFPVGTNPIFVATGDVNGDSKLDLAVANTSSNNVSVLLGNGNGSFGAATNFPAGTNPYSVAIRDVNGDSKLDLAVTNYSSNNVSVLPGNGNGSFGIATNFPVGTNPESIAIADFNGDSKLDLAVTNSGNNNVSILLNNFQGLPKNKI

SEQ ID NO: 70 - DNA, 1227 bp, Cylindrospermopsis raciborskii T3
gtgaaaaggctcactttactaattatagcggggatattatctgttagtacatttttatgtataactcctgttgcattagcaaatataactgactattatctgaagaatgaaaagctttctgggcaatttagtgttccggttaatttgtccgtaggagtgagatttgcccacaggagtagttatgctactgctattaacttcccaactggtcttgatgctgactctgtagcagttggggatttcaatagcgatagtaagctcgacctggctgttacaaattggttcgacaataacgtctcggtcttactgggaaatggtaatgggtcttttggcgcagccactaactttccagtcggtactaatcccgtctttgtagtgactggggatgtaaatggcgacagcaagcttgacctggctgttgcaaattttagtagcaataacgtctcggtcttactaggaaatggtaatgggtcttttggcgcagccactaacttttcagttggtactaacccttattctgtagccattggagatgtgaataacgatagtgagcttgaccttgcttttacaaattggttcgacaataaggtcttggttttactgggaaatggtaatgggtcttttggcgcagccagcagcttccctgtcgatacttattcgatttccgtagcgattgcggattttaatagcgacagtaagctcgaccttgctattacaaattgggtcagcaataacgtctcggtcttactgggaaatggtaatgggtcttttggcgcagccactaactttccagtcggtactaatcccatatttgtagcaactggggatgtaaatggcgacagcaagcttgacctggctgttgcaaatactagcagcaataacgtctcggtcttactgggaaatggtaatgggtcttttggcgcagccactaactttccagccggtactaatccctactctgtagcgattagagatgtgaatggcgacagtaaacttgacctggctgttacaaattatagtagcaataacgtctcggtcttaccaggaaatggtaatgggtcttttggcatagctactaactttccagtcggtactaatcctgaatctatagcaattgcggatttcaacggcgacagcaagcttgacctggctgtcacaaattctggcaacaacaacgtctcgatcttgttgaataattttcagggacttccaaaaaataagatatag

SEQ ID NO: 71 - DNA, 1227 bp, Cylindrospermopsis raciborskii T3
atgaaacgtctgacgctgctgatcattgcaggtattctgtcagttagcacctttctgtgtattacaccggttgcactggccaatattaccgattattatctgaaaaacgagaaactgagcggtcagtttagcgttccggtgaatctgtctgttggtgttcgttttgcacatcgtagcagctatgcaaccgcaattaactttccgaccggtctggatgcagatagcgttgcagttggtgattttaacagcgatagcaaactggatctggccgttaccaattggtttgataacaatgttagcgtgctgctgggtaatggcaatggcagctttggtgcagcaaccaattttccggttggcaccaatccggtttttgttgttaccggtgatgttaatggtgacagtaaactggatttagccgtggcaaattttagcagcaataatgtttcagttctgctgggaaacggtaatggttcttttggcgcagccacaaactttagcgttggtacaaatccgtatagcgtggccattggtgatgtgaataatgatagtgaactggacctggcatttacgaactggttcgataataaagttctggtgctgttaggcaatggtaatggctcgtttggtgccgcaagctcatttccggtggatacctatagcattagcgttgcgattgcagatttcaactcagattctaaattagacctggcgatcaccaattgggtgtcaaataatgtgagtgtgttactggggaatggtaacggtagttttggagctgcgacaaattttcctgtgggtacaaacccgatttttgtggcaaccggtgacgtgaatggcgattctaagctggacttagcagttgcaaataccagctctaataacgttagcgttctgttaggtaacgggaacggctcattcggtgctgccacgaattttccagcaggcaccaacccgtatagtgttgcaattcgcgacgttaacggtgatagcaaattagatttagcggtgaccaactatagcagcaacaacgtgagtgttctgccaggcaacggtaacggatcatttggtattgcgaccaactttccagtaggtacgaatccggaaagcattgcaattgccgattttaatggggattccaagttagatctggcagtgacaaatagcggtaacaataatgtaagcatactgctgaataactttcagggtctgccgaaaaacaagatttga

SEQ ID NO: 72 - protein, 200 aa, Cylindrospermopsis raciborskii T3
MKSTNIHYTKHLISPYDRYLKNGHKSGILWFTGLSGAGKTTLALKLEQTLFEKGWSTFVLDGDSVRHGLCSDLGFSASDRSENIRRLGEVAKLFAESGCLVITAFISPYRNDREQVRRLAGDLFHEVYIATPLELCEQRDPKGLYLKARSGEIDGFTGISAPYEPPNSPDLWVETSELTVEESLEQLLKYVENKFTIFKQ

SEQ ID NO: 73 - DNA, 603 bp, Cylindrospermopsis raciborskii T3
atgaaatcaactaatattcactatacaaaacatcttatatctccatatgatcgttatctaaagaatggtcataaaagcgggattctatggtttactggactgtccggggctggtaaaacaacattggctttaaaattagagcagactttgttcgagaaaggatggtctacctttgttttagatggtgatagtgttcgtcatggactgtgttccgatttaggattttctgctagtgatcgctcagaaaatatccgtcgtttgggtgaggttgccaaactctttgcggagtcaggatgcctagtgatcactgccttcatctcaccctacaggaatgaccgagaacaggtgcgtagactagctggagatctatttcatgaagtatacattgcaactccactggaactttgtgagcagcgtgatccgaaaggtctttatctaaaagcacgcagtggggaaatagatggatttacgggaatcagcgccccttatgaaccacccaatagcccagatttatgggtggaaacatccgaactcaccgtcgaggaaagcctagaacaactactcaaatacgtggaaaacaaattcacaattttcaaacaatag

SEQ ID NO: 74 - protein, 221 aa, Cylindrospermopsis raciborskii T3
MKAVVKYTIFEKPQPIRAIKRLERDVLRMGALVEQSFRLSHQALFNRDLTAAEQIRRLDKKIDRFYRQIEVDCATIMSSQAPTDQESRCLSSFMQLVRDLERIGDYAKDLAEIAMKIFPYPPHPTLGEVAIMSDHAQSMLATSLVALADLDEISGRRIKLLDDTVDDAYKKLYRNLAQQKDVPGVVEPILLLTLAIQCLERMADHATNIGQRVAYIVTGQR

SEQ ID NO: 75 - DNA, 666 bp, Cylindrospermopsis raciborskii T3
atgaaagctgttgtgaaatatacaatttttgaaaaacctcaacctatacgtgccattaaaagactggaacgagatgttttgcgtatgggtgctttagtagagcagtcattccgtctgagtcaccaagctctattcaatcgggatttaacagcagctgagcaaatacggagattagacaaaaaaattgatcgcttctacagacaaatagaagtcgattgtgccacaattatgagcagtcaagctcccacagaccaagaatctcggtgtttaagctcattcatgcaattagttagagacttggaacgtattggggactatgccaaagatttggcagaaatagcaatgaaaatatttccctatcccccccatcctactttgggggaggttgccattatgtccgatcatgcccaatctatgttggctaccagcctagtagctttagcggatttagacgagattagtggtagaaggattaaattattagatgatacagtagatgatgcttacaaaaagttatatcgtaatttggcgcagcagaaagatgttcccggggtagtggagcccattttactattaacattagcaattcagtgtttagagagaatggcagatcatgctactaatattggtcaaagggtagcatacattgttacagggcaaagatag

SEQ ID NO: 76 - protein, 450 aa, Cylindrospermopsis raciborskii T3
MFLLGFLLGLAVGFGFWLWQQFQLNSHLEQLTQPLNPHAEKILLPLLAGLHRKISTVRDEQQNLRLSLKAYEQLLDAAPLGYLQVDEENQLLWCNQCAREMLYLQRWQPGQVRLLLELVRSYELDQLIEQTRDWQKPQMQEWIFHPSRDHGQGILGLKPLSLAANSFPLPGGQVGVFLESHQQFVDIHQQRDRSFSDLAHELRTPLTSIRLVAETLQTRLDPPLNRWVIRLMQEVDRLINLVQNWLDLTQMEITSSIQLNLEMLEVRSLIFSVWENLEPLAANQHLSISYSGPEKVYICADKSRIYQVFLNLLDNCIKYSNLNGTIFIEMNPVCGEKSINGVDPEADTILNQVSNQILEINIIDSGVGFAPMDLPHVFQRFYRGDKARHRESRSENETVEITGSGLGLSIVRQIIIAHGGKIRAMNHPDTGGAWIQIHLPQVVQHDGGYF

SEQ ID NO: 77 - DNA, 1353 bp, Cylindrospermopsis raciborskii T3
atgttcttattgggatttcttctgggtttggcagtcggttttggtttttggctttggcaacaatttcaacttaacagtcatttggagcagttaacccaacccttaaaccctcacgctgaaaagatattattacccctattagctggattacatcgtaaaatatctaccgttagagatgagcaacaaaacttacgcttgtcactcaaagcttatgaacagttgctggatgctgcgcctttgggatatttacaagtagatgaagaaaaccaactactatggtgtaatcagtgcgcgcgggaaatgctgtatttacaaagatggcaaccgggtcaagtgcgcctgctactggaattagtgagatcctatgagctggatcagttaattgagcaaacccgggattggcaaaaaccgcaaatgcaagagtggatttttcacccttcccgagatcatggtcagggtattttaggattaaagccattgtctttagcagctaacagttttcccctaccggggggacaagtgggtgtgtttctagaaagtcaccaacaatttgtagacattcatcagcaacgtgaccgctctttttcagacctggcccatgaactgagaacacctctgacttccattcgtctggtcgcagaaaccctgcaaactcgcttagatccccctctaaaccgttgggtcatccgcttgatgcaggaggttgacagactaattaatttagtccaaaattggttagacctgacccagatggaaataacctcctccatacaactgaatttggaaatgctagaagtccgctccctaattttttcagtctgggagaatttagagcccctagccgctaatcagcatcttagtatttcttactccggcccggaaaaggtctatatatgtgctgataagtccagaatttatcaagtgtttcttaatctgttagataactgtattaaatacagcaacctgaacggtactattttcattgaaatgaatccagtttgtggggagaagtctattaatggggttgatccagaagcagatacaatattaaaccaagtatcaaatcagattttagaaattaacattattgattccggggttggatttgctcccatggatctaccccatgtctttcaaagattttatcggggggacaaagctagacaccgcgagtcccgctctgagaatgaaacagtagaaattactggtagtggtttagggttatccattgtccgccaaataattatagctcatggtggcaaaatcagggccatgaaccatcctgataccggtggtgcttggatacaaattcatcttccccaggtggttcaacatgatggcggatatttctga

SEQ ID NO: 78 - protein, 240 aa, Cylindrospermopsis raciborskii T3
VNQSIVWQRAPENFQLCAQEVHIWKINLKVSPSEVELCRRILSGDEIARAERFSFPEHQERFIVGRAFLRKILSRYLNVEAQAIEFEYEERGKPLLGFKFKYSGICFNLSHSQELALCGVTHQRSIGVDLEGVRHTSDIENLANRFFSVKEYGVIKSVPPEQQQQVFFRYWTCKEAYLKAIGKGLSELSQIEIELTPNKSARLRVLGDWQLKELVPADNFAAAVVIASHNHLDRFEFWEP

SEQ ID NO: 79 - DNA, 723 bp, Cylindrospermopsis raciborskii T3
gtgaatcagtctattgtttggcaacgggcacctgaaaatttccagttgtgcgctcaggaagtacatatctggaagattaacctgaaagtatcaccatcagaggtggaactttgtcgcaggattttatctggtgatgaaatagctcgtgcggaaagattttcttttccggaacatcaagagcgttttattgttggtcgtgcctttcttagaaaaatactatcaagatatttaaacgtagaagcacaagcaatagagtttgagtatgaagagagaggaaaaccactgttagggttcaagtttaagtactctggaatatgttttaatttatcccattctcaggaattagctttatgcggtgtgactcatcaaagatccattggagtagatctagaaggtgttcgtcacacatcagatatagaaaacctagccaaccgctttttttcagttaaagaatatggggtaattaaatcagtacccccggaacaacaacagcaggtatttttccgttattggacttgtaaagaggcctatttaaaagctattggaaaaggtttgtctgagttatctcaaatagaaatagaattaacgccaaataaatctgctaggttgcgtgtattgggagattggcagttaaaagaactagtaccagcagataattttgcagcagcagttgttatagctagccataatcatttagacaggtttgagttttgggaaccttaa

SEQ ID NO: 80 - DNA, 723 bp, Cylindrospermopsis raciborskii T3
atgaatcaatcaatcgtgtggcagcgtgcgccggaaaacttccaactgtgtgctcaagaagtgcatatctggaaaatcaacctgaaagtgagcccgtctgaagtggaactgtgccgtcgcattctgagtggcgatgaaatcgcgcgtgccgaacgcttttccttcccggaacatcaggaacgttttattgtgggtcgtgcattcctgcgcaaaatcctgagccgctatctgaacgttgaagcacaggctattgaatttgaatacgaagaacgtggcaaaccgctgctgggtttcaaattcaaatactctggcatctgcttcaatctgagtcattcccaggaactggcgctgtgtggtgttacccaccaacgttcaattggcgtcgatctggaaggtgtgcgccacacgtcggacatcgaaaacctggccaatcgtttctttagcgtcaaagaatacggcgtgattaaaagcgtgccgccggaacagcaacagcaagtgtttttccgctattggacctgtaaagaagcgtacctgaaagccatcggcaaaggtctgtcagaactgtcgcagattgaaatcgaactgacgccgaacaaatcagcgcgtctgcgcgttctgggtgattggcaactgaaagaactggtcccggcagacaattttgctgcagcagttgtcattgcgagtcataatcatctggaccgttttgaattttgggaaccgtga

SEQ ID NO: 81 - DNA, 27 bp, Artificial Sequence
  Primer
gggctttcatatgttacaaaagattaa

SEQ ID NO: 82 - DNA, 27 bp, Artificial Sequence
  Primer
aaagtatgcggccgcatgcttgagtat

SEQ ID NO: 83 - DNA, 26 bp, Artificial Sequence
  Primer
ggcatccatgggcaagatttacggaa

SEQ ID NO: 84 - DNA, 27 bp, Artificial Sequence
  Primer
ggcatctcgagttataaaagcgcttcg

SEQ ID NO: 85 - DNA, 27 bp, Artificial Sequence
  Primer
ggttaagatctgaaattaatacgactc

SEQ ID NO: 86 - DNA, 27 bp, Artificial Sequence
  Primer
ttttaagatcttttcagcaaaaaaccc

SEQ ID NO: 87 - DNA, 30 bp, Artificial Sequence
  Primer
atatccatgggacctggtgatcgcaaagga

SEQ ID NO: 88 - DNA, 29 bp, Artificial Sequence
  Primer
tatctcgagagtgttgatttcgttggctg

SEQ ID NO: 89 - DNA, 675 bp, Bacillus subtilis
atgaagatttacggaatttatatggaccgcccgctttcacaggaagaaaatgaacggttcatgactttcatatcacctgaaaaacgggagaaatgccggagattttatcataaagaagatgctcaccgcaccctgctgggagatgtgctcgttcgctcagtcataagcaggcagtatcagttggacaaatccgatatccgctttagcacgcaggaatacgggaagccgtgcatccctgatcttcccgacgctcatttcaacatttctcactccggccgctgggtcattggtgcgtttgattcacagccgatcggcatagatatcgaaaaaacgaaaccgatcagccttgagatcgccaagcgcttcttttcaaaaacagagtacagcgaccttttagcaaaagacaaggacgagcagacagactatttttatcatctatggtcaatgaaagaaagctttatcaaacaggaaggcaaaggcttatcgcttccgcttgattccttttcagtgcgcctgcatcaggacggacaagtatccattgagcttccggacagccattccccatgctatatcaaaacgtatgaggtcgatcccggctacaaaatggctgtatgcgccgcacaccctgatttccccgaggatatcacaatggtctcgtacgaagagcttttataa

SEQ ID NO: 90 - protein, 224 aa, Bacillus subtilis
MKIYGIYMDRPLSQEENERFMTFISPEKREKCRRFYHKEDAHRTLLGDVLVRSVISRQYQLDKSDIRFSTQEYGKPCIPDLPDAHFNISHSGRWVIGAFDSQPIGIDIEKTKPISLEIAKRFFSKTEYSDLLAKDKDEQTDYFYHLWSMKESFIKQEGKGLSLPLDSFSVRLHQDGQVSIELPDSHSPCYIKTYEVDPGYKMAVCAAHPDFPEDITMVSYEELL

SEQ ID NO: 91 - DNA, 7035 bp, Artificial Sequence
  Sequence of sxt1 fragment after integration into E. coli lactose operon
gtttcatctgtggtgcaacgggcgctgggtcggttacggccaggacagtcagtggagatgcccaagggcacttcgggtcgaggaacccgacctgcattgggacgcggccacggagagcgcgggcaaacgccggcactatagccagtggagtttgtaaaacgctatttcagagcttggagagtgtctaagaaagccgggcgatgccaacccatcccttcttcggctacgttcgtaatcaagccacttcctttttgcattgacgcagggtgtcggaaggcaactcgccgaacgcgctcctatagttttcagcgaagcgtcccaaatgtaagaagccgtagtctagggctatctcagttatactacgcacattggcactgggatcgttcaagcaggcgcggatgctttcgagcttgcggttgcggatgtagttcttcggcgtggtgccggcatgcttctcgaacaaattgtagagcgagcgtggactcatcatcgccagctccgctaaccgctcaaggctgatattccgtttgagattctcctcaatgaattgaacgactcgctcgaaagacgggttacctttgctgaaaatttcacggctgacattgctgcccagcatttcgagcagcttggaagcgatgatccccgcatagtgctcttggacccgaggcatcgactttgtatgttccgcttcgtcacaaactaacccgagtagattgataaagccatcgagttgctggagattgtgtcgcgcggcgaaacggataccctccctcggcttgtgccaattgttgtcactgcatgcccgatcaaggaccactgagggcaatttaacgataaatttctcgcaatcttctgaataggtcaggtcggcttggtcatccggattgagcagcaatagttcgcccggcgcaaaatagtgctcctggccatggccacgccacaggcaatggcctttgagtattatttgcagatgataacaggtctctaatccaggcgagattaccctcacgctaccgccgtagctgattcgacacaggtcgaggcatccgaagattctgtggtgcagcctgcctgccgggggcccgcccttgggcaggcgaatagagtgcgtaccgacatactggttaacataatcggagactgcatagggctcggcgtggacgaagatctgacttttctcgttcaataagcaaaaatccatagttcacggttctcttattttaatgtgggctgcttggtgtgatgtagaaaggcgccaagtcgatgaaaatgcaggaattaattcgcagatcctggcggatgagagaagattttcagcctgatacagattaaatcagaacgcagaagcggtctgataaaacagaatttgcctggcggcagtagcgcggtggtcccacctgaccccatgccgaactcagaagtgaaacgccgtagcgccgatggtagtgtggggtctccccatgcgagagtagggaactgccaggcatcaaataaaacgaaaggctcagtcgaaagactgggcctttcgttttatctgttgtttgtcggtgaacgctctcctgagtaggacaaatccgccgggagcggatttgaacgttgcgaagcaacggcccggagggtggcgggcaggacgcccgccataaactgccaggcatcaaattaagcagaaggccatcctgacggatggcctttttgcgtagatcccagccttgcaagaagcggatacaggagtgcaaaaaatggctatctctagaaaggcctaccccttaggctttatgcaacagaaacaataataatggagtcatgaacatgctgcagaaaatcaatcgttatacccatggttttgttgccgttccggttattctggcatgtcgtgaaaaaggtgtttttgaactgctggcagatgaaagtccgctgagcctgaatcagatggttgaacatctgggtgccaatagcggtcattttcaggttgcactgcgtatgctggaaagtctgcattggctgagccgtaataaagaactgaaatatagcctgaccgcagaagcagcaattcataacaaaattagcgaagatatcctgcagctgtataatctgccgattcagagctatctggaaggtaaacagggcaatctgctgggtcgttggattgaacgtagctgtcagctgtggaatctggataatccgctgatggcagattttctggatggtctgctggttattccgctgctgctggcactgcataaacataacctgctggccgattctgaagataaaccgctgctgagcagcctgagcagtaccgttcaagaagaactgggtaaactgtttctgcatctgggttgggcagatctgacagcaggtcgtctgaccattaccgaactgggtcgctttatgggtgaacgtgcactgaataccgcaattgttgcaagctataccccgatgctgagtcgtattcatgatgttctgtttggtaattgcctgagcgtttttcagcgtgatgcaagcggtcatgaacgtcatattgatcgtaccctgaatgttattggtagcggttttcagcaccagaaatactttgcagatctggaagaaagcattctgagcgtgtttaatcagctgccgctggaagaacagccgaaatacattaccgatatgggttgtggtgatggcaccctgctgaaacgtgtttgggaaaccattcagtttaaaagcgcacgtggtaaagcactggaacagtatccgctgcgtctgattggtgttgattataatgaagcaagcctgaaagcaaccacccgtaccctggcaagcctgccgcatctggttctgcagggtgatattggtaatccggaacaaatggttcgtagcctggaagcacatggcattcatgatccggaaaatattctgcatattcgcagctttctggatcacgatcgtctgtttattccgcctcagaaacgtaatgaactgaaagaacgtgcccatctgccgtatcagagtgtttgtgttgatgatcagggtgaactgattcctccgcatgttatggttcagagcctggtggaacacctggaacgttggagccaggttgttaataaacatggtctgatgattctggaagtgcattgtctggaaccgcgtgttgtttatcagtttctggataaaagcgaaaacctgcactttgatgcatttcagggttttagccagcagtatctggttgaagccgaagtttttctgatgagcgcagcacaggttggtctgtttccgaaactggaactgagcaaacgttatccgaaaacctttccgtttacccgtattaccctgaactatttcgaaaaacgtccgtacaaaatcagccatgcatatctgagcgatctgcctgcactggttgacctggaagttaaatgttggcctgagaatctgcgtgcaagcacccatgaaattcgtcgtcgtctggaactgaatccgcagggtaacctggttctgattattgaagatcagattatcggtgccatttacagccagaccattacaagcaccgaagccctggaaaatgttaaatatgcacaggttccgaccctgcatacaccgcagggttcagtgattcagctgctggccctgaacattctgccggaatttcaggcacgtggtctgggcaatgaactgcgtgattttatgctgtattattgcaccctgaaaggtggtattgaaagcgttgttggtgttacccgttgtcgcaattatgtgaattatagccagatgccgatgatggaatatctgaaactgcataatgaacagcgtcaactgctggatccgattgttggttttcatgttagcggtggtgcagaaattcgtggcattattgcaaattatcgtccggaagatacagataatctgggtatgggtattctgatcgaatataacctgcgtgatagcgcactgcattcaccgggtgatcgtaaaggtccgtatatcaatagcgcaattggtagcctggttccgaaagcgaccagcgcaaccaaagaaaacaaaaccgttgcggatctggtgaaagaatgtattctgaaagtgatgggtagccagcgtcaggcagcatatgcaccgcagcagaaactgctggacatgggtctggatagcctggatctgctggaactgcagaccctgctggaagaacgtctgggtattaatctgagcggcaccttttttctgcaaaaaaacaccccgaccgccatcattacctattttcagaatcaggtcgtgcaagagaaacagagtgatctggcaccgcctgttgatagcgccaatgaaatcaatacactggaaaacgttgtgaatcagcagaaaattccgcaggttacacgtgttgttaccgaacagcagggacgtaaagttctgattgatggtcattgggttattgattttgccagctgtaattatctgggcctggacctgcatccgaaagttaaagaagcaattcctccggcactggataaatggggcacccatccgagctggacccgtctggttgcaagtccggcaatttatgaggaactggaagaggaactgtcaaaactgctgggtgtgccggatgttctggtttttccggcagttacactgctgcagattggtattctgcctctgctgaccggtaataatggtgtgatttttggcgatattgcagcccatcgttgtatttatgaagcatgttgtctggcccagcataaaggtgcacagtttattcagtatcgtcataacgacctgaatgatctggccgaaaaactggccaaatatccgcctgaacaggttaaaatcattgtgatcgatggtgtgtatagcatgagtgccgatttcccggacctgcctgcatatgttcatctggcaaaagaatataacgccctgatctatatggatgatgcacatggctttggcattctgggtgaaaatccgagcagcgatatgccgtatggttataaaggtaatggcatggtgaactactttgatctgcgttttgccgaagataacatcatttatgttgcaggtctgagcaaagcctatagcagctatgcagcatttctgacctgtggtgatcgtcgtattaaaaccaattttcgtaatgcatggaccgcgatttttagcggtccgagtccggttgcaagcctggccagcgcactggcaggtctgcaggttaatcgtcaagaaggtgaacagctgcgcaaacaaatctatcatctgacacataaactggttacccaggctcgtgccattggttttgaagttgataattatggttatgtgccgattgtgggtgttctggtgggtgatgcacagcatatgattgatgtgtgccaactgctgtgggaatatggtatcctgattacccctgcaatttttccgattgtgccgctgaataaatcagcactgcgttttagcattaccgcagcaaataccgaagaagaaattgatcaggccatcaaaagtctgaaagcagtttgggacctgctgcaaaaacgtaaagccctgccgtgtaaacaagaagaaaatatcctgaaacattgagaaggagatatacatatgacccatgttgccctggaacaggcaattgcaaaagttccgcgtagcattcagagcgaactgcgtaccattctggcacagcatgcagttattgatagcagcgttgtggcaagctggattgatcgtctgggcaccaatattagtaccctgatgatccagctgctgccggttgcagcaacctatgcacgtgttccgattagccagttttatgttggtgccattgcactgggcaaaccgcagagtaaaaatcagctgggtagcggcaccctgtattttggtgcagatatggaatttgttggtcaggcactgagctttagcgttcatgcagaacagagcgccaccattaatgcctggctgcatggcgaaaccggactgcaggcactggcaatccatgaagcaccgtgtggttattgtcgccagtttctgtatgaaatggcaaccgtgaatcagaattttgtgctgctggtgaaaagcaatgaaagccagccggaacagacctataccagcaacaaactgccgcattttctgcctgaaccgtttggtccagccgatctgggtctgaccggtggcctgatgcagaccgtgtttcacgatctggaaacctatagcaccgatgatgttgttctggcagcactgagtgcagcaaatcagagttatgcaccgtataccaaaaactttgccggtgttgcactgaaagatagtcatggtaacatttttacaggtcgctatgccgaaaacgcagcatttaatagcagcatgagcccgatggaaagcgcactgacctttatgaatatgaatcgttattcacagagcctgttcgatatttgtgatgcagttctggtagaagtggaaaccggtattagtcagcgtccggttaccgaagcctttctgagtagcattgcaccgaaagtgaaactgcgctatgcaccggcaaccccgagcagtaacaaactgtgagaaggagatatacatatgtttcagaccaaaagctattatagcgtcgttggcctggaaaccgaactgattaaaggtaaattcttcatgagcaacgaactgaccaatgaacaggtgtttaaactggtgtgcatggaagtgattgaaaaaatgggttttgcacactttccgcctattatcctggtttatgaaatgaccaattccggctttgttgattggtgcgagcagatggtttttgtggatgataaaggcaaactggatgagggcgaaaaatttctgctggattggatgcgtcgtaatgtgggtaattttgatctgattcgcgaactgatgccggtggcagaacgcctggaaatgaaaatgcgtagctaactcggtaccaaattccagaaaagaggcctcccgaaaggggggccttttttcgttttggtcccgaagttcctattctctagaaagtataggaacttcgaccgcctgtctatttctcttacggttccaacatccatataggccgcaatt

SEQ ID NO: 92 - DNA, 12758 bp, Artificial Sequence
  Sequence of sxt3 fragment version 1 integrated into the E. coli xylose operon
ttgcatttccttgagccttatccgacttgtcagtcggataaggctttttactttgtctcaggcagttgagctacgagcctgaagcgttgttggtgcgttttatcatgcctggcgggtaggtcggataaggcgttcacgccgcatccgacaaccacgcagcgttacctgatgtgacgccgacaattctcatcatcgctacaacatgacctcgctatttacatcgcgatactcttttggcgtcgtgtcatatgcttttttaaaaacagagtagaaatattgcagcgatggataaccgcacatttgcgatatctcattgatcgacaaggtggttgaaatcagcagactgcgcgctttctccagcttctcggcatgaatcatggcatggatggtttcacccacctcttctttaaaacgcttctcaagattggagcgcgagatcccgaccgcatccagtacctgatccactttaatccctttacaggcgtgattacgaatgtaatgcatggcctgaataacggcgggatcggtcagcgagcgataatctgttgagcgccgttcaatgacgcgaactggtgggaccaaaattcgctgtagcggcatttcttctttatctaataatcgatgcaacagttttgccgcctgatagcccatttgccgcgcgccctgagcgaccgaagaaagggcgacacgcgacagatagcgggtcagttcttcgttatcgatgccaatcacgcataatttttccggtacgggaatatgtagatgttcacatacttgcagaatatgccgcgctcgggcgtcagtaacggcaataatcccggtttgcggtggtagcgtttgtagccagtctgccagccgattttgcgcgtgttgccagttctctggcgcggtttctaacccctgataaaccactccgcgatacttttcttcggcgacaagctgacgaaatgcatattcgcgctcagtggcccaacgtttgccgcttgattccggaagaccataaaaagcaaagcggttaacgcctttctcttttaaatgcaaaaatgcgctttcaaccagcgcatagttatcggtggcaatgtaatgaacgggtgggtaactttctgcaaggtgatacgagccgccaaccccaacaatggggacgtcgacatcagccagcgcttgctcgatctgtttgtcgtcgaagtcggcaatgacgccatctcctaaccagtccttgattttatcaatgcgggcgcggaaatcttcttcaatgaaaatatcccattccgattgtgacgcctgtaaatattcccctacgccttctactacctgccggtcataggctttattggcattgaacagtaatgtgatgcggtgacgtttagtaaacatggttcttttcctgctgaatcatgcaaaaactcaaaaccggtaatacgtaaccggctttgagaaaatttttatcaaaatcaagaacggcgtttggttgcggagtccatccatactgccagcaacagaatcgcacctttaacgatatactgccagaaggtcggtacatccatcatactcatgccgttatccagtgaagccatgataaatgcccccattactgctccggcaacgcttcccacaccgccagccaggctggtgccgccaatcacgcatgctgcaattgcgtccagttcggcgatatttcccgcagaaggtgaaccagcgccaagtcgagaactaaggattaatccggcgatggctaccattaatccgttaatcgcgaacacggcaagtttggtgcgttcaacgttaatcccggagagacgtgctgcttccagattgccgccgatggcataaatgcgtcgtccaaatgccgtccgcgtttccataaacattccgccgagtaacagcaacgtcagcagcagaacaggagtgggaacgccacggtaatcattcaacagccagattgcgcctaatacgatgatagcggttaaagcctggcgaccgactactgcggtagaggccggagactgcaaacccaaagcctgacggcgcattcttccgcgccattgccaaccaacaaaagccattaagccaagcgcgccaatgatgaagccagtgctggcaggtagatagctttgcccaatttgtgacatcgcggcgctggtgggggaaacagtcgtgccgttggtgatgccaatgagtatgccgcgaaatgccaacatgcccgcgagggtgacaataaatgaagggactttgcggtacgcgacccaccatccgttccaggcaccgagaagcagtcccagaaccaacgtcacaatgatggtaagtggcaaaggccagcctaaccagacgtcacaaatcgccgcgacgccacctaatagccccatcattgagccgacggaaaggtcgatttcagcagaaattatgacgaacaccattcctaccgcgaggatgccggtaatcgcggtctggcgtaacaggttggagacgttacgggcgcttaagtaggcaccatcggtggtccaggtaaagaacagcatgattgcgatgatagctgcaatcatcacgaagacctgcaaattcagtgatttcagcccggagaagctaccggatgtcggtacggccaatttcacttcagacggattgcttttcgacatgatgttcgctcctcaatgcggcttccatcacctgctcctgagtcaggttatgatttatcaggttggcttttagtttcccttcatgcatcaccagtacacgatcgctaaggccgagcacttcaggtaattcggaagagatgacaataacggcaataccctgctggacgagttggttaattaatttgtagatctcgtatttcgcgccaatatcgatacccctggtgggttcatcaagaatgagaatgcgcgggttaagtaacagacagcgagcgaggatcgctttttgctgattgccgccgctcaaacgtccaatagcaaggtcgggggacgacgttttaactttgagttgctggattgattccagaatacatttttgctctgccgcgtcatcaagctggctaatgccaccggtaaatttattgagtcggcgagggtaatatttttaccaaccgccattaccggaacgatgccgtcgcgctttctgtcttcgggtaccatcgcaatcccctgggcgatggcttgctgacagttacgaatatctacctgtttgccatcaatataaatttttccttcccattgtccgggccacacgccaaacaggcactgaatggtctcggtacgtccggcaccaacgagtccggcaatacccagtatttcgccacgtttcagggaaaacgagacatcattaactcgtttaatatgacgattgaccggatgccatgccgtcagatgttcaatacgtaatatttcatctccggtggtatgtggttcattagggtaaagcgcggttaactctcgcccgaccatcatggtgataatatcgtcttcactcattccggcagcatcacgcgtaccaatgtgctgtccgtcgcgaataacgcaaatcgtatcggaaatcgctttgacttcgttgagtttgtgcgaaatataaatacaggcgataccgtgctgttgtagatcgcgaataatatccagtaaaaccgacgtttcctgctcagttaatgaggctgtcggttcatcgagaattaacaagcgcacctgtttattaagtgccttggcaatttcaaccagttgttgttgcccaagccctaaatcgccaacgcgggtatcaggtgaaatggataaactgacctgtgcgagcagcttctgacagcgtagcgtcatcaggtcataatccataatgccattgtgggttatttcgttacccaggaagatattttccagcacggtcaattctttcaccagggccaattcctgatgaatgatggcgatacctttgcgttcggtatcgcggatgtgactcgcctgaatctcttctcccgcaaaaataatttcgccttcgtaggagccatggggataaataccacacagcactttcatcagcgttgatttaccagacccattttccccacaaagtgagacgatttcgccagcattcaaccgcaagcagacgttatcaatcgccttcacactgccgaaggttttggtaatgttcttcatttcaagtagataaggcataacgactccacctaagccaattcattcacgcggcatggagagaaatcacgcccccgctccgcgccgggcgtaacgcttacagctcgctctctttgtggaatccgtctttaattaccgtatctttgatgttgtttttattcacatcgatcggtgtcaggaggcgggaggggacatctttcaggccattattcagtgaggtccagccttgcaagaagcggatacaggagtgcaaaaaatggctatctctagaaaggcctaccccttaggctttatgcaacagaaacaataataatggagtcatgaacatatggtgattaaaaacctgtgtccggatggtgttaccccgatttggaataaaagccagatggaaagcagcctgctggaagaatgtctgcctgcatgggttcgtaccagctatagcacctttgttgaaaccattagcgatagcgcatttccgtgtttttggggcaccattggtgaacagaaaggtatgattcgttatctgattgttagcagcctgaccgatccgattctggttgaacataccctggaaggtatctacaaatatatcgatgaagtgaacgaaaacgaactgctgcagcatgaaaatgcagatctgctgaccctggttatcttttttccgcctgaaccgaccgttctgaccgttgaagaatatgcaggtcaggcatttgattttctgaatgcactgcatagcctggatgcagttagctgtccgtgtcattggagcgcagatccgcagagcgcaaattggagctatagcctgggtggttgtgcactgtttgttagcgttagcacaccggcaaatcagaaacgtcgtagccgtcatctgggtagcggtatgacctttgttattacaccggttgaagtgctgctgaataaacatggtggtgaaaacagcagcatttttcgtcgtgttcgtgaatatgatggtattccgcctcatccgaatctgctgattatgcctggtaatggtaaagtgggtaatgaactgaccgtgcaggttctgccggataataatgatagcgaaatcagcttcgattttcagtataaattcaaagattgagaaggagatatacatatgaccatccagattgtgcagcataacctggaatatagctttgtgaccccgaaagaaaccagcgattttgttgaacgtaccatgagcgtttttgatcaggcatatccgaaatttctgatccatgatgtttgggcagatccggcaagcctggccctgtttgaaatttatccggaatttcagtttggtctggtggaagcaaccacccagctgatgattgcacagggtaattgtattccgctgacctatgaaagccgttttgatgaactgccggatgaaggttgtgattgggcactggcaaaatggctggaagatcgcgaacagaatcgtctgccgaatgccctgtgtgttgtgagcattagcatcctgccggaatatcagggtaaaaatctgagccagtatctgatcggctatatgaaagaactggcacagtatcatggtctgaatagcctgattatggcagcacgtccgagcctgaaatatctgtatccgctgattccgattgaacgctatattacctggcgtgataaaaacggcctgatttttgatccgtggctgcgtgttaatgttaaacatggcgcaaaaattgccggtatctgctttaaaagcaccaccattaatgataccattgatggttgggaggatcgtgttggtatgcgttttccggaaaccggtgattatatcattccgaaaggtctggttccggtgaaaattgattatccgaataacatgggcatctacatcgaaccgaatatctggctgtattatgatctggactgagaaggagatatacatatgatcaacatcgaacagtttcgccaagaaatcgaagattggattattaacgttgtcagcattccgaacccgctgaccggtaattttcctccgtgtccgtatgcaaaagcagcatggctgaataatcgtgttagcgtgcgttggtttcatggtccggaactgcctgaactgctgatggaacaaattcgtacatggaacaacgatttcgagatggtgatttttggttgcgatcctcagaatctggatgcacagcgtctggaacgttatatcaccaaagcaaattatgtgctgcccgaatatgacctggttgcactgggtagccatccggataaacagtatgttggtgatgatgccgaaaatgtgaacaacgtgattattacccatccgaaatatgttctggcaagcgttcagagctttagccagctgcaagaggcaagtgatgagctgctgcgtctgggttatttccagtattggtcagcagaaaaactggccgaaatgaaaagcgaacgtgcaagccataatctgagcagcattcagcgtaaaaatagctatcgtattatcccgaccaaccattgagaaggagatatacatatgctgaccgcagaacagaaacaggcatataccaatgatggctattttaccgtggaagaagcagttccgaaagcactgattgaagaaattcgccatgaagtggaactgatcaccgagcagaaacgtggtggtgtgctggcaggcgattatgaatggtggtcagaacacaccattccggatccggttcgttatcagaaaattatccagcgtctgctggaactgccgaccgttatgggtccggttcaggccctgattggtagcgatatttttctgttaattaccgacctggcaattattcgtgcaggcaccggttatattgcatggcatcaggatcatggctatgttgttgaagttctgaacgccctggcaagcatgagcaaaaatgagctgaatgatgatgcactgcgcctgctggtgccggttgcaaatcaggcaatggtgtttattaccatctatctgcaggataccgataacaccatgggcaccatgcgtgtgattccgagcagccatcagtgggaacatagtctggatagcagcagcgccaattcactgaatgcagaaatttgtctgagcctgcctggtggtgcagcaatgttttataccccgaccgtttggcataccgcagcagcaaataccagcattaccgattatcgtatgctgacgctgatcttcaccaaaaacaacattaaaccgctgctggttgatgccctgaaacgtattatttgagaaggagatatacatatgacaaccaccgatccgatcctgattaataactggcatgttgtggcaaatgtcgaggattgtaaaccgggtagcattacccgtagccgtttactgggtgttaaactggttctgtggcgtagctatgaacagaatagcccgattcaggtttggctggattattgtccgcatcgtggtgttccgctgagcatgggtgaaattaccaataataccctggtttgtccgtatcatggctggcgttataatgaagcaggtaaatgtattcagattccggcacatccgggtatggttccgcctgcaagcgcagaagcacgtacctatcatagccaagaacgttatggtctggtttgggtttgtctgggtgatccggttaatgatattccgtcatttccggaatgggatgatccgaattatcacaaaacctacaccaaaagctatctgattaaagcaagcgcctttcgcgttatggataattcactggatgttagccattttccgtttattcatgatggctggctgggcgatcgtaactataccaaagtggaagaatttgaagtgaaactggataaagatggtctgacgatgggcaaatatcagtttcagaccagccgtattgtgagccatattgaagatgatagctgggtgaattggtttcgtctgagccatccgctgtgtcagtattgtgttagcgaaagtccggaaatgcgtattgttgatctgatgaccattacgccgattgatgaagaaaatagcgttctgcgcatgctgatcatgtggaatggttatgaaaccctggaaagcaaaatgctgacagagtatgatgaaacgatcgaacaggatattcgtattctgcatgcccagcagccggtgcgtctgccgctgctgacaccgaagcagattaatacccagctgtttagccatgaaattcatgttccgagcgatcgttgtaccctggcatatcgtcgttggctgaaacaactgggtgtgacctatggtgtttgttgagaaggagatatacatatggcaggtaaactggatggtaaggttgcaattattaccggtgcaagcagcggtattggtgaagccaccgcatttgcactggcagcagaaggtgcaaaagttgcaattgcagcccgtcgtgcagaactgttacatgcactggccaaacgtattgaagcaagcggtggtcaggcactgccgattgttaccgatatcaccgatgaaagccaggttaatcatctggttcagaaaaccaaagttgaactgggtcatgttgatatcctggtgaataatgcaggtattggcgtttttggtgcaatcgataccggtaatccggcagattggcgtcgtgcatttgatgttaatgtgctgggtgttctgtatgcaattcatgcagttctgcctttactgaaagcacagaaaagcggtcatattgtgaatattagcagcgtggatggtcgtattgcacagagcggtgcagttgtttatagcgcagcaaaaagcggtgttaatgccctgagcgaagcactgcgtcaagaagtgagcctggataatattcgtgtgaccattattgaaccgggtctggtagataccccgtttaatgatctgattagtgatccgattaccaaacagctgagcaaagaacagctgtcaaccattactccgctgcagagcgaagatattgcacgtgccattatctatgcagttacccagccggatcatgttaacgttaatgaaattctgattcgtccgaccgcagaggataattgagaaggagatatacatatgaacctgaccctgaacaaagaagaaaaacagctgctgacggcatatagcggcaccgaactgcagctgacagcagatgttctggttattggtggtggtccggcagccgcatgggcagcttgggcagcaggcgcacagggtgtgaaagttattattgtggataaaggttttctgggcaccagcggtgccgcagccgcaagcggtaatagcgttatggcaccgtcaccggaaaattgggaaaaagatgtgagcgaatgttacagcaaaggtaataatctggcaaatctgcgttggattgaacgtgttattgaaaaagcctggctgtcactgccgctggttgaagattggggttatcgttttcctaaagaaaatggtgaaagcgtgcgtcagagctattatggtcctgaatatatgcgtgttctgcggaaaaatctgctgcgcgttggtgttcagatctttgatcagtcaccggcactggaattactgctggcacaggatggtagcgttgccggtgcacgtggtgtgcagcgtcagaatcatcgtacatataccgttcgtgccggtgccgttgttctggccaatggtggttgcgcatttctgagtaaagcactgggttgtaataccaataccggtgatggtctgttaatggcagttgaagccggtggtgaactgagcagtatggaagccagcagccattataccattagcaccgcctttaatgcaaccgttacccgtgcagctccgttttattgggcaagctataccgatgaagctggcaatgatctgggtggctatattaacggtcgtcgtgatccgagctttctgccgaacgcactgctgaaaggtccggtttatgcacgtctggatcgtgcaacaccggaaattcaggcgctggtagaaaaaagccattttattgcatttctgccgtacaagaaagccggtattgatccgtataccgaacgtgttccggttaccctggtgctggaaggcaccgtgcgtggcaccggtggtattcgcattgttaatgattcatgtggcaccaaagttccgggactgtatgcagcgggtgatgcagcaagccgtgaatttctggcaggcattgccagcggtggtgatggaccgaatgcagcatgggcaatttcaaccggtcagtgggcaggcgaaggtgcagcagcctttgcaaaaagtctgggtgcacatgttcatgaacgcgttgttcgtccggcaggccaggcaggtctgcgtagtcagtatccgggtagcgaaacctttgatagtgaagcagttgttcgtggcgttcaggcagaaatgtttccgctggaaaaaaactatctgcgctgtgaacagggactgctggatagcctggcaaaactggaaatgctgtggcagcaggttcagggtaatccgaaacaggatacagttcgtgatctggaattttcacgtcgtgcggcagcactggttagcgtggcacgttgggcatattttagcgcactgcatcgtaaagaaacccgtagcgaacatatccgtattgattacccggaaacggatccgaatcaactgtattatcaggcaaccggtggcctggaacgtctgtgggtgcgtcgtgattgggttaaagatgcaagcgccacccctccggtgctgaccacctgagaaggagatatacatatgattgaactggtgagccataagctgtgcattaattgtaatgtttgtgttcaggtgtgcccgaccaatgtttttgatgcagtgccgaatcagcctccggcaattgcacgccaagaagattgtcagacctgttttatttgtgaagcatattgtcctgcagatgcgctgtatgttgcaccgcagagccataccaatgttgcagttaacgaagatgatttaatcgacagcggcattatgggtgaatatcgtcgcattctgggttggggctatggtcgtaaaaacaatagcgaactggataccgaccataaactgcgtctgtttgaatgagaaggagatatacatatgtcatttcagaaatttgtgcaagaagcagcctataaagtcgcaccgtttaaaccgaatcgttttgccaaaattagcgagcgtgaagataaatgtgcaattccggttccggcatggcgtgcactgctggccaatcgtgacctgtttacctggaaaggtattccgtttctgaaaggttgtaccgaaattgcactgtatagcatgctgctgtatgaactgcgtccgaaaacgattattgaaattggtgcgctgagcggtggtagcgcaatttggctggcagatcatctggaactgtttcagattgaaggttgcgtgtattgcattgatattgatctgtctctgctggacgaaaaagcaaaaaccgatagccgtgttcattttctggaaggtgattgcaataatatgggtgcaattatgtcaagcgagctgctgagtggtctggcacatccttggctgattgttgaagatgcacatgcaaatgccgttggtgtggttgaatattttcacgaaaacggtctgaaaagtggcgattacctgatcgtggaagataccaataaaacaatgtgggaactggatcgcgaagaactggaccgtgatgacctggatgaacaagaactgatcgaaaaaggtgagcagaaattagcagaactgaaaagctggctgatgctgcatgagaatgaatatctgatagatacctactatcaggatatgtatggctataatggtagccgtaattggaacagcattctgaaacgtgtggaaaagaacttttaatctaactaaaaacaccctaacgggtgttttttcttttctggtctccccgaagttcctattctctagaaagtataggaacttcgctggattgggccgcgaaattaaccggcctgagcaatgtcccagctttaatcgctgcagctcaacaggctgatgaaagtgccgagccagtttggtttctgccttatctttccggcgagcgtacgccacacaataatccccaggcgaagggggttttctttggtttgactcatcaacatggccccaatgaactggcgcgagcagtgctggaaggcgtgggttatgcgctggcagatggcatggatgtcgtgcatgcctgcggtattaaaccgcaaagtgttacgttgattgggggcggggcgcgtagtgagtactggcgtcagatgctggcggatatcagcggtcagcagctcgattaccgtacgggaggggatgtggggccagcactgggcgcagcaaggctggcgcagatcgcggcgaatccagagaaatcgctcattgaattgttgccgcaactaccgttagaacagtcgcatctaccagatgcgcagcgttatgccgcttatcagccacgacgagaaacgttccgtcgcctctatcagcaacttctgccattaatggcgtaaacgttatcccctgcctgaccgggtgggggataattcacatctatatatctcagtaattaattaatatttagtatgaatttattctgaaaatcatttgttaatggcatttttcagttttgtctttcgttggttactcgtaatgtatcgctggtagatatggagatcgtt

SEQ ID NO: 93 - DNA, 7185 bp, Artificial Sequence
  Sequence of sxt3 fragment version 2 integrated into the E. coli xylose operon
ggtgtcaggaggcgggaggggacatctttcaggccattattcagtgaggtccagccttgcaagaagcggatacaggagtgcaaaaaatggctatctctagaaaggcctaccccttaggctttatgcaacagaaacaataataatggagtcatgaacatatggtgattaaaaacctgtgtccggatggtgttaccccgatttggaataaaagccagatggaaagcagcctgctggaagaatgtctgcctgcatgggttcgtaccagctatagcacctttgttgaaaccattagcgatagcgcatttccgtgtttttggggcaccattggtgaacagaaaggtatgattcgttatctgattgttagcagcctgaccgatccgattctggttgaacataccctggaaggtatctacaaatatatcgatgaagtgaacgaaaacgaactgctgcagcatgaaaatgcagatctgctgaccctggttatcttttttccgcctgaaccgaccgttctgaccgttgaagaatatgcaggtcaggcatttgattttctgaatgcactgcatagcctggatgcagttagctgtccgtgtcattggagcgcagatccgcagagcgcaaattggagctatagcctgggtggttgtgcactgtttgttagcgttagcacaccggcaaatcagaaacgtcgtagccgtcatctgggtagcggtatgacctttgttattacaccggttgaagtgctgctgaataaacatggtggtgaaaacagcagcatttttcgtcgtgttcgtgaatatgatggtattccgcctcatccgaatctgctgattatgcctggtaatggtaaagtgggtaatgaactgaccgtgcaggttctgccggataataatgatagcgaaatcagcttcgattttcagtataaattcaaagattgagaaggagatatacatatgaccatccagattgtgcagcataacctggaatatagctttgtgaccccgaaagaaaccagcgattttgttgaacgtaccatgagcgtttttgatcaggcatatccgaaatttctgatccatgatgtttgggcagatccggcaagcctggccctgtttgaaatttatccggaatttcagtttggtctggtggaagcaaccacccagctgatgattgcacagggtaattgtattccgctgacctatgaaagccgttttgatgaactgccggatgaaggttgtgattgggcactggcaaaatggctggaagatcgcgaacagaatcgtctgccgaatgccctgtgtgttgtgagcattagcatcctgccggaatatcagggtaaaaatctgagccagtatctgatcggctatatgaaagaactggcacagtatcatggtctgaatagcctgattatggcagcacgtccgagcctgaaatatctgtatccgctgattccgattgaacgctatattacctggcgtgataaaaacggcctgatttttgatccgtggctgcgtgttaatgttaaacatggcgcaaaaattgccggtatctgctttaaaagcaccaccattaatgataccattgatggttgggaggatcgtgttggtatgcgttttccggaaaccggtgattatatcattccgaaaggtctggttccggtgaaaattgattatccgaataacatgggcatctacatcgaaccgaatatctggctgtattatgatctggactgagaaggagatatacatatgctgaccgcagaacagaaacaggcatataccaatgatggctattttaccgtggaagaagcagttccgaaagcactgattgaagaaattcgccatgaagtggaactgatcaccgagcagaaacgtggtggtgtgctggcaggcgattatgaatggtggtcagaacacaccattccggatccggttcgttatcagaaaattatccagcgtctgctggaactgccgaccgttatgggtccggttcaggccctgattggtagcgatatttttctgttaattaccgacctggcaattattcgtgcaggcaccggttatattgcatggcatcaggatcatggctatgttgttgaagttctgaacgccctggcaagcatgagcaaaaatgagctgaatgatgatgcactgcgcctgctggtgccggttgcaaatcaggcaatggtgtttattaccatctatctgcaggataccgataacaccatgggcaccatgcgtgtgattccgagcagccatcagtgggaacatagtctggatagcagcagcgccaattcactgaatgcagaaatttgtctgagcctgcctggtggtgcagcaatgttttataccccgaccgtttggcataccgcagcagcaaataccagcattaccgattatcgtatgctgacgctgatcttcaccaaaaacaacattaaaccgctgctggttgatgccctgaaacgtattatttgagaaggagatatacatatgacaaccaccgatccgatcctgattaataactggcatgttgtggcaaatgtcgaggattgtaaaccgggtagcattacccgtagccgtttactgggtgttaaactggttctgtggcgtagctatgaacagaatagcccgattcaggtttggctggattattgtccgcatcgtggtgttccgctgagcatgggtgaaattaccaataataccctggtttgtccgtatcatggctggcgttataatgaagcaggtaaatgtattcagattccggcacatccgggtatggttccgcctgcaagcgcagaagcacgtacctatcatagccaagaacgttatggtctggtttgggtttgtctgggtgatccggttaatgatattccgtcatttccggaatgggatgatccgaattatcacaaaacctacaccaaaagctatctgattaaagcaagcgcctttcgcgttatggataattcactggatgttagccattttccgtttattcatgatggctggctgggcgatcgtaactataccaaagtggaagaatttgaagtgaaactggataaagatggtctgacgatgggcaaatatcagtttcagaccagccgtattgtgagccatattgaagatgatagctgggtgaattggtttcgtctgagccatccgctgtgtcagtattgtgttagcgaaagtccggaaatgcgtattgttgatctgatgaccattacgccgattgatgaagaaaatagcgttctgcgcatgctgatcatgtggaatggttatgaaaccctggaaagcaaaatgctgacagagtatgatgaaacgatcgaacaggatattcgtattctgcatgcccagcagccggtgcgtctgccgctgctgacaccgaagcagattaatacccagctgtttagccatgaaattcatgttccgagcgatcgttgtaccctggcatatcgtcgttggctgaaacaactgggtgtgacctatggtgtttgttgagaaggagatatacatatggcaggtaaactggatggtaaggttgcaattattaccggtgcaagcagcggtattggtgaagccaccgcatttgcactggcagcagaaggtgcaaaagttgcaattgcagcccgtcgtgcagaactgttacatgcactggccaaacgtattgaagcaagcggtggtcaggcactgccgattgttaccgatatcaccgatgaaagccaggttaatcatctggttcagaaaaccaaagttgaactgggtcatgttgatatcctggtgaataatgcaggtattggcgtttttggtgcaatcgataccggtaatccggcagattggcgtcgtgcatttgatgttaatgtgctgggtgttctgtatgcaattcatgcagttctgcctttactgaaagcacagaaaagcggtcatattgtgaatattagcagcgtggatggtcgtattgcacagagcggtgcagttgtttatagcgcagcaaaaagcggtgttaatgccctgagcgaagcactgcgtcaagaagtgagcctggataatattcgtgtgaccattattgaaccgggtctggtagataccccgtttaatgatctgattagtgatccgattaccaaacagctgagcaaagaacagctgtcaaccattactccgctgcagagcgaagatattgcacgtgccattatctatgcagttacccagccggatcatgttaacgttaatgaaattctgattcgtccgaccgcagaggataattgagaaggagatatacatatgaacctgaccctgaacaaagaagaaaaacagctgctgacggcatatagcggcaccgaactgcagctgacagcagatgttctggttattggtggtggtccggcagccgcatgggcagcttgggcagcaggcgcacagggtgtgaaagttattattgtggataaaggttttctgggcaccagcggtgccgcagccgcaagcggtaatagcgttatggcaccgtcaccggaaaattgggaaaaagatgtgagcgaatgttacagcaaaggtaataatctggcaaatctgcgttggattgaacgtgttattgaaaaagcctggctgtcactgccgctggttgaagattggggttatcgttttcctaaagaaaatggtgaaagcgtgcgtcagagctattatggtcctgaatatatgcgtgttctgcggaaaaatctgctgcgcgttggtgttcagatctttgatcagtcaccggcactggaattactgctggcacaggatggtagcgttgccggtgcacgtggtgtgcagcgtcagaatcatcgtacatataccgttcgtgccggtgccgttgttctggccaatggtggttgcgcatttctgagtaaagcactgggttgtaataccaataccggtgatggtctgttaatggcagttgaagccggtggtgaactgagcagtatggaagccagcagccattataccattagcaccgcctttaatgcaaccgttacccgtgcagctccgttttattgggcaagctataccgatgaagctggcaatgatctgggtggctatattaacggtcgtcgtgatccgagctttctgccgaacgcactgctgaaaggtccggtttatgcacgtctggatcgtgcaacaccggaaattcaggcgctggtagaaaaaagccattttattgcatttctgccgtacaagaaagccggtattgatccgtataccgaacgtgttccggttaccctggtgctggaaggcaccgtgcgtggcaccggtggtattcgcattgttaatgattcatgtggcaccaaagttccgggactgtatgcagcgggtgatgcagcaagccgtgaatttctggcaggcattgccagcggtggtgatggaccgaatgcagcatgggcaatttcaaccggtcagtgggcaggcgaaggtgcagcagcctttgcaaaaagtctgggtgcacatgttcatgaacgcgttgttcgtccggcaggccaggcaggtctgcgtagtcagtatccgggtagcgaaacctttgatagtgaagcagttgttcgtggcgttcaggcagaaatgtttccgctggaaaaaaactatctgcgctgtgaacagggactgctggatagcctggcaaaactggaaatgctgtggcagcaggttcagggtaatccgaaacaggatacagttcgtgatctggaattttcacgtcgtgcggcagcactggttagcgtggcacgttgggcatattttagcgcactgcatcgtaaagaaacccgtagcgaacatatccgtattgattacccggaaacggatccgaatcaactgtattatcaggcaaccggtggcctggaacgtctgtgggtgcgtcgtgattgggttaaagatgcaagcgccacccctccggtgctgaccacctgagaaggagatatacatatgattgaactggtgagccataagctgtgcattaattgtaatgtttgtgttcaggtgtgcccgaccaatgtttttgatgcagtgccgaatcagcctccggcaattgcacgccaagaagattgtcagacctgttttatttgtgaagcatattgtcctgcagatgcgctgtatgttgcaccgcagagccataccaatgttgcagttaacgaagatgatttaatcgacagcggcattatgggtgaatatcgtcgcattctgggttggggctatggtcgtaaaaacaatagcgaactggataccgaccataaactgcgtctgtttgaatgagaaggagatatacatatgtcatttcagaaatttgtgcaagaagcagcctataaagtcgcaccgtttaaaccgaatcgttttgccaaaattagcgagcgtgaagataaatgtgcaattccggttccggcatggcgtgcactgctggccaatcgtgacctgtttacctggaaaggtattccgtttctgaaaggttgtaccgaaattgcactgtatagcatgctgctgtatgaactgcgtccgaaaacgattattgaaattggtgcgctgagcggtggtagcgcaatttggctggcagatcatctggaactgtttcagattgaaggttgcgtgtattgcattgatattgatctgtctctgctggacgaaaaagcaaaaaccgatagccgtgttcattttctggaaggtgattgcaataatatgggtgcaattatgtcaagcgagctgctgagtggtctggcacatccttggctgattgttgaagatgcacatgcaaatgccgttggtgtggttgaatattttcacgaaaacggtctgaaaagtggcgattacctgatcgtggaagataccaataaaacaatgtgggaactggatcgcgaagaactggaccgtgatgacctggatgaacaagaactgatcgaaaaaggtgagcagaaattagcagaactgaaaagctggctgatgctgcatgagaatgaatatctgatagatacctactatcaggatatgtatggctataatggtagccgtaattggaacagcattctgaaacgtgtggaaaagaacttttaatctaactaaaaacaccctaacgggtgttttttcttttctggtctccccgaagttcctattctctagaaagtataggaacttcgctggattgggccgcgaaattaaccggcctgagcaatgtcccagctttaat

SEQ ID NO: 94 - DNA, 5599 bp, Artificial Sequence
  Sequence of sxt3 fragment version 3 integrated into the E. coli xylose operon
ggtgtcaggaggcgggaggggacatctttcaggccattattcagtgaggtccagccttgcaagaagcggatacaggagtgcaaaaaatggctatctctagaaaggcctaccccttaggctttatgcaacagaaacaataataatggagtcatgaacatgctgaccgcagaacagaaacaggcatataccaatgatggctattttaccgtggaagaagcagttccgaaagcactgattgaagaaattcgccatgaagtggaactgatcaccgagcagaaacgtggtggtgtgctggcaggcgattatgaatggtggtcagaacacaccattccggatccggttcgttatcagaaaattatccagcgtctgctggaactgccgaccgttatgggtccggttcaggccctgattggtagcgatatttttctgttaattaccgacctggcaattattcgtgcaggcaccggttatattgcatggcatcaggatcatggctatgttgttgaagttctgaacgccctggcaagcatgagcaaaaatgagctgaatgatgatgcactgcgcctgctggtgccggttgcaaatcaggcaatggtgtttattaccatctatctgcaggataccgataacaccatgggcaccatgcgtgtgattccgagcagccatcagtgggaacatagtctggatagcagcagcgccaattcactgaatgcagaaatttgtctgagcctgcctggtggtgcagcaatgttttataccccgaccgtttggcataccgcagcagcaaataccagcattaccgattatcgtatgctgacgctgatcttcaccaaaaacaacattaaaccgctgctggttgatgccctgaaacgtattatttgagaaggagatatacatatgacaaccaccgatccgatcctgattaataactggcatgttgtggcaaatgtcgaggattgtaaaccgggtagcattacccgtagccgtttactgggtgttaaactggttctgtggcgtagctatgaacagaatagcccgattcaggtttggctggattattgtccgcatcgtggtgttccgctgagcatgggtgaaattaccaataataccctggtttgtccgtatcatggctggcgttataatgaagcaggtaaatgtattcagattccggcacatccgggtatggttccgcctgcaagcgcagaagcacgtacctatcatagccaagaacgttatggtctggtttgggtttgtctgggtgatccggttaatgatattccgtcatttccggaatgggatgatccgaattatcacaaaacctacaccaaaagctatctgattaaagcaagcgcctttcgcgttatggataattcactggatgttagccattttccgtttattcatgatggctggctgggcgatcgtaactataccaaagtggaagaatttgaagtgaaactggataaagatggtctgacgatgggcaaatatcagtttcagaccagccgtattgtgagccatattgaagatgatagctgggtgaattggtttcgtctgagccatccgctgtgtcagtattgtgttagcgaaagtccggaaatgcgtattgttgatctgatgaccattacgccgattgatgaagaaaatagcgttctgcgcatgctgatcatgtggaatggttatgaaaccctggaaagcaaaatgctgacagagtatgatgaaacgatcgaacaggatattcgtattctgcatgcccagcagccggtgcgtctgccgctgctgacaccgaagcagattaatacccagctgtttagccatgaaattcatgttccgagcgatcgttgtaccctggcatatcgtcgttggctgaaacaactgggtgtgacctatggtgtttgttgagaaggagatatacatatggcaggtaaactggatggtaaggttgcaattattaccggtgcaagcagcggtattggtgaagccaccgcatttgcactggcagcagaaggtgcaaaagttgcaattgcagcccgtcgtgcagaactgttacatgcactggccaaacgtattgaagcaagcggtggtcaggcactgccgattgttaccgatatcaccgatgaaagccaggttaatcatctggttcagaaaaccaaagttgaactgggtcatgttgatatcctggtgaataatgcaggtattggcgtttttggtgcaatcgataccggtaatccggcagattggcgtcgtgcatttgatgttaatgtgctgggtgttctgtatgcaattcatgcagttctgcctttactgaaagcacagaaaagcggtcatattgtgaatattagcagcgtggatggtcgtattgcacagagcggtgcagttgtttatagcgcagcaaaaagcggtgttaatgccctgagcgaagcactgcgtcaagaagtgagcctggataatattcgtgtgaccattattgaaccgggtctggtagataccccgtttaatgatctgattagtgatccgattaccaaacagctgagcaaagaacagctgtcaaccattactccgctgcagagcgaagatattgcacgtgccattatctatgcagttacccagccggatcatgttaacgttaatgaaattctgattcgtccgaccgcagaggataattgagaaggagatatacatatgaacctgaccctgaacaaagaagaaaaacagctgctgacggcatatagcggcaccgaactgcagctgacagcagatgttctggttattggtggtggtccggcagccgcatgggcagcttgggcagcaggcgcacagggtgtgaaagttattattgtggataaaggttttctgggcaccagcggtgccgcagccgcaagcggtaatagcgttatggcaccgtcaccggaaaattgggaaaaagatgtgagcgaatgttacagcaaaggtaataatctggcaaatctgcgttggattgaacgtgttattgaaaaagcctggctgtcactgccgctggttgaagattggggttatcgttttcctaaagaaaatggtgaaagcgtgcgtcagagctattatggtcctgaatatatgcgtgttctgcggaaaaatctgctgcgcgttggtgttcagatctttgatcagtcaccggcactggaattactgctggcacaggatggtagcgttgccggtgcacgtggtgtgcagcgtcagaatcatcgtacatataccgttcgtgccggtgccgttgttctggccaatggtggttgcgcatttctgagtaaagcactgggttgtaataccaataccggtgatggtctgttaatggcagttgaagccggtggtgaactgagcagtatggaagccagcagccattataccattagcaccgcctttaatgcaaccgttacccgtgcagctccgttttattgggcaagctataccgatgaagctggcaatgatctgggtggctatattaacggtcgtcgtgatccgagctttctgccgaacgcactgctgaaaggtccggtttatgcacgtctggatcgtgcaacaccggaaattcaggcgctggtagaaaaaagccattttattgcatttctgccgtacaagaaagccggtattgatccgtataccgaacgtgttccggttaccctggtgctggaaggcaccgtgcgtggcaccggtggtattcgcattgttaatgattcatgtggcaccaaagttccgggactgtatgcagcgggtgatgcagcaagccgtgaatttctggcaggcattgccagcggtggtgatggaccgaatgcagcatgggcaatttcaaccggtcagtgggcaggcgaaggtgcagcagcctttgcaaaaagtctgggtgcacatgttcatgaacgcgttgttcgtccggcaggccaggcaggtctgcgtagtcagtatccgggtagcgaaacctttgatagtgaagcagttgttcgtggcgttcaggcagaaatgtttccgctggaaaaaaactatctgcgctgtgaacagggactgctggatagcctggcaaaactggaaatgctgtggcagcaggttcagggtaatccgaaacaggatacagttcgtgatctggaattttcacgtcgtgcggcagcactggttagcgtggcacgttgggcatattttagcgcactgcatcgtaaagaaacccgtagcgaacatatccgtattgattacccggaaacggatccgaatcaactgtattatcaggcaaccggtggcctggaacgtctgtgggtgcgtcgtgattgggttaaagatgcaagcgccacccctccggtgctgaccacctgagaaggagatatacatatgattgaactggtgagccataagctgtgcattaattgtaatgtttgtgttcaggtgtgcccgaccaatgtttttgatgcagtgccgaatcagcctccggcaattgcacgccaagaagattgtcagacctgttttatttgtgaagcatattgtcctgcagatgcgctgtatgttgcaccgcagagccataccaatgttgcagttaacgaagatgatttaatcgacagcggcattatgggtgaatatcgtcgcattctgggttggggctatggtcgtaaaaacaatagcgaactggataccgaccataaactgcgtctgtttgaatgagaaggagatatacatatgtcatttcagaaatttgtgcaagaagcagcctataaagtcgcaccgtttaaaccgaatcgttttgccaaaattagcgagcgtgaagataaatgtgcaattccggttccggcatggcgtgcactgctggccaatcgtgacctgtttacctggaaaggtattccgtttctgaaaggttgtaccgaaattgcactgtatagcatgctgctgtatgaactgcgtccgaaaacgattattgaaattggtgcgctgagcggtggtagcgcaatttggctggcagatcatctggaactgtttcagattgaaggttgcgtgtattgcattgatattgatctgtctctgctggacgaaaaagcaaaaaccgatagccgtgttcattttctggaaggtgattgcaataatatgggtgcaattatgtcaagcgagctgctgagtggtctggcacatccttggctgattgttgaagatgcacatgcaaatgccgttggtgtggttgaatattttcacgaaaacggtctgaaaagtggcgattacctgatcgtggaagataccaataaaacaatgtgggaactggatcgcgaagaactggaccgtgatgacctggatgaacaagaactgatcgaaaaaggtgagcagaaattagcagaactgaaaagctggctgatgctgcatgagaatgaatatctgatagatacctactatcaggatatgtatggctataatggtagccgtaattggaacagcattctgaaacgtgtggaaaagaacttttaatctaactaaaaacaccctaacgggtgttttttcttttctggtctccccgaagttcctattctctagaaagtataggaacttcgctggattgggccgcgaaattaaccggcctgagcaatgtcccagctttaat

SEQ ID NO: 95 - DNA, 7064 bp, Artificial Sequence
  Sequence of sxt1 fragment, integrated into the E. coli lactose operon
atgaccatgattacggattcactggccgtcgttttacaacgtcgtgactgggaaaaccctggcgttacccaacttaatcgccttgcagcacatccccctttcgccagctggcgtaatagcgaagaggcccgcaccgatcgcccttcccaacagttgcgcagcctgaatggcgaatggcgctttgcctggtttccggcaccagaagcggtgccggaaagctggctggagtgcgatcttcctgaggccgatactgtcgtcgtcccctcaaactggcagatgcacggttacgatgcgcccatctacaccaacgtgacctatcccattacggtcaatccgccgtttgttcccacggagaatccgacgggttgttactcgctcacatttaatgttgatgaaagctggctacaggaaggccagacgcgaattatttttgatggcgttaactcggcgtttcatctgtggtgcaacgggcgctgggtcggttacggccaggacagtcagtggagatgcccaagggcacttcgggtcgaggaacccgacctgcattgggacgcggccacggagagcgcgggcaaacgccggcactatagccagtggagtttgtaaaacgctatttcagagcttggagagtgtctaagaaagccgggcgatgccaacccatcccttcttcggctacgttcgtaatcaagccacttcctttttgcattgacgcagggtgtcggaaggcaactcgccgaacgcgctcctatagttttcagcgaagcgtcccaaatgtaagaagccgtagtctagggctatctcagttatactacgcacattggcactgggatcgttcaagcaggcgcggatgctttcgagcttgcggttgcggatgtagttcttcggcgtggtgccggcatgcttctcgaacaaattgtagagcgagcgtggactcatcatcgccagctccgctaaccgctcaaggctgatattccgtttgagattctcctcaatgaattgaacgactcgctcgaaagacgggttacctttgctgaaaatttcacggctgacattgctgcccagcatttcgagcagcttggaagcgatgatccccgcatagtgctcttggacccgaggcatcgactttgtatgttccgcttcgtcacaaactaacccgagtagattgataaagccatcgagttgctggagattgtgtcgcgcggcgaaacggataccctccctcggcttgtgccaattgttgtcactgcatgcccgatcaaggaccactgagggcaatttaacgataaatttctcgcaatcttctgaataggtcaggtcggcttggtcatccggattgagcagcaatagttcgcccggcgcaaaatagtgctcctggccatggccacgccacaggcaatggcctttgagtattatttgcagatgataacaggtctctaatccaggcgagattaccctcacgctaccgccgtagctgattcgacacaggtcgaggcatccgaagattctgtggtgcagcctgcctgccgggggcccgcccttgggcaggcgaatagagtgcgtaccgacatactggttaacataatcggagactgcatagggctcggcgtggacgaagatctgacttttctcgttcaataagcaaaaatccatagttcacggttctcttattttaatgtgggctgcttggtgtgatgtagaaaggcgccaagtcgatgaaaatgcaggaattaattcgcagatcctggcggatgagagaagattttcagcctgatacagattaaatcagaacgcagaagcggtctgataaaacagaatttgcctggcggcagtagcgcggtggtcccacctgaccccatgccgaactcagaagtgaaacgccgtagcgccgatggtagtgtggggtctccccatgcgagagtagggaactgccaggcatcaaataaaacgaaaggctcagtcgaaagactgggcctttcgttttatctgttgtttgtcggtgaacgctctcctgagtaggacaaatccgccgggagcggatttgaacgttgcgaagcaacggcccggagggtggcgggcaggacgcccgccataaactgccaggcatcaaattaagcagaaggccatcctgacggatggcctttttgcgtagatcccagccttgcaagaagcggatacaggagtgcaaaaaatggctatctctagaaaggcctaccccttaggctttatgcaacagaaacaataataatggagtcatgaacatgctgcagaaaatcaatcgttatacccatggttttgttgccgttccggttattctggcatgtcgtgaaaaaggtgtttttgaactgctggcagatgaaagtccgctgagcctgaatcagatggttgaacatctgggtgccaatagcggtcattttcaggttgcactgcgtatgctggaaagtctgcattggctgagccgtaataaagaactgaaatatagcctgaccgcagaagcagcaattcataacaaaattagcgaagatatcctgcagctgtataatctgccgattcagagctatctggaaggtaaacagggcaatctgctgggtcgttggattgaacgtagctgtcagctgtggaatctggataatccgctgatggcagattttctggatggtctgctggttattccgctgctgctggcactgcataaacataacctgctggccgattctgaagataaaccgctgctgagcagcctgagcagtaccgttcaagaagaactgggtaaactgtttctgcatctgggttgggcagatctgacagcaggtcgtctgaccattaccgaactgggtcgctttatgggtgaacgtgcactgaataccgcaattgttgcaagctataccccgatgctgagtcgtattcatgatgttctgtttggtaattgcctgagcgtttttcagcgtgatgcaagcggtcatgaacgtcatattgatcgtaccctgaatgttattggtagcggttttcagcaccagaaatactttgcagatctggaagaaagcattctgagcgtgtttaatcagctgccgctggaagaacagccgaaatacattaccgatatgggttgtggtgatggcaccctgctgaaacgtgtttgggaaaccattcagtttaaaagcgcacgtggtaaagcactggaacagtatccgctgcgtctgattggtgttgattataatgaagcaagcctgaaagcaaccacccgtaccctggcaagcctgccgcatctggttctgcagggtgatattggtaatccggaacaaatggttcgtagcctggaagcacatggcattcatgatccggaaaatattctgcatattcgcagctttctggatcacgatcgtctgtttattccgcctcagaaacgtaatgaactgaaagaacgtgcccatctgccgtatcagagtgtttgtgttgatgatcagggtgaactgattcctccgcatgttatggttcagagcctggtggaacacctggaacgttggagccaggttgttaataaacatggtctgatgattctggaagtgcattgtctggaaccgcgtgttgtttatcagtttctggataaaagcgaaaacctgcactttgatgcatttcagggttttagccagcagtatctggttgaagccgaagtttttctgatgagcgcagcacaggttggtctgtttccgaaactggaactgagcaaacgttatccgaaaacctttccgtttacccgtattaccctgaactatttcgaaaaacgtccgtacaaaatcagccatgcatatctgagcgatctgcctgcactggttgacctggaagttaaatgttggcctgagaatctgcgtgcaagcacccatgaaattcgtcgtcgtctggaactgaatccgcagggtaacctggttctgattattgaagatcagattatcggtgccatttacagccagaccattacaagcaccgaagccctggaaaatgttaaatatgcacaggttccgaccctgcatacaccgcagggttcagtgattcagctgctggccctgaacattctgccggaatttcaggcacgtggtctgggcaatgaactgcgtgattttatgctgtattattgcaccctgaaaggtggtattgaaagcgttgttggtgttacccgttgtcgcaattatgtgaattatagccagatgccgatgatggaatatctgaaactgcataatgaacagcgtcaactgctggatccgattgttggttttcatgttagcggtggtgcagaaattcgtggcattattgcaaattatcgtccggaagatacagataatctgggtatgggtattctgatcgaatataacctgcgtgatagcgcactgcattcaccgggtgatcgtaaaggtccgtatatcaatagcgcaattggtagcctggttccgaaagcgaccagcgcaaccaaagaaaacaaaaccgttgcggatctggtgaaagaatgtattctgaaagtgatgggtagccagcgtcaggcagcatatgcaccgcagcagaaactgctggacatgggtctggatagcctggatctgctggaactgcagaccctgctggaagaacgtctgggtattaatctgagcggcaccttttttctgcaaaaaaacaccccgaccgccatcattacctattttcagaatcaggtcgtgcaagagaaacagagtgatctggcaccgcctgttgatagcgccaatgaaatcaatacactggaaaacgttgtgaatcagcagaaaattccgcaggttacacgtgttgttaccgaacagcagggacgtaaagttctgattgatggtcattgggttattgattttgccagctgtaattatctgggcctggacctgcatccgaaagttaaagaagcaattcctccggcactggataaatggggcacccatccgagctggacccgtctggttgcaagtccggcaatttatgaggaactggaagaggaactgtcaaaactgctgggtgtgccggatgttctggtttttccggcagttacactgctgcagattggtattctgcctctgctgaccggtaataatggtgtgatttttggcgatattgcagcccatcgttgtatttatgaagcatgttgtctggcccagcataaaggtgcacagtttattcagtatcgtcataacgacctgaatgatctggccgaaaaactggccaaatatccgcctgaacaggttaaaatcattgtgatcgatggtgtgtatagcatgagtgccgatttcccggacctgcctgcatatgttcatctggcaaaagaatataacgccctgatctatatggatgatgcacatggctttggcattctgggtgaaaatccgagcagcgatatgccgtatggttataaaggtaatggcatggtgaactactttgatctgcgttttgccgaagataacatcatttatgttgcaggtctgagcaaagcctatagcagctatgcagcatttctgacctgtggtgatcgtcgtattaaaaccaattttcgtaatgcatggaccgcgatttttagcggtccgagtccggttgcaagcctggccagcgcactggcaggtctgcaggttaatcgtcaagaaggtgaacagctgcgcaaacaaatctatcatctgacacataaactggttacccaggctcgtgccattggttttgaagttgataattatggttatgtgccgattgtgggtgttctggtgggtgatgcacagcatatgattgatgtgtgccaactgctgtgggaatatggtatcctgattacccctgcaatttttccgattgtgccgctgaataaatcagcactgcgttttagcattaccgcagcaaataccgaagaagaaattgatcaggccatcaaaagtctgaaagcagtttgggacctgctgcaaaaacgtaaagccctgccgtgtaaacaagaagaaaatatcctgaaacattgagaaggagatatacatatgacccatgttgccctggaacaggcaattgcaaaagttccgcgtagcattcagagcgaactgcgtaccattctggcacagcatgcagttattgatagcagcgttgtggcaagctggattgatcgtctgggcaccaatattagtaccctgatgatccagctgctgccggttgcagcaacctatgcacgtgttccgattagccagttttatgttggtgccattgcactgggcaaaccgcagagtaaaaatcagctgggtagcggcaccctgtattttggtgcagatatggaatttgttggtcaggcactgagctttagcgttcatgcagaacagagcgccaccattaatgcctggctgcatggcgaaaccggactgcaggcactggcaatccatgaagcaccgtgtggttattgtcgccagtttctgtatgaaatggcaaccgtgaatcagaattttgtgctgctggtgaaaagcaatgaaagccagccggaacagacctataccagcaacaaactgccgcattttctgcctgaaccgtttggtccagccgatctgggtctgaccggtggcctgatgcagaccgtgtttcacgatctggaaacctatagcaccgatgatgttgttctggcagcactgagtgcagcaaatcagagttatgcaccgtataccaaaaactttgccggtgttgcactgaaagatagtcatggtaacatttttacaggtcgctatgccgaaaacgcagcatttaatagcagcatgagcccgatggaaagcgcactgacctttatgaatatgaatcgttattcacagagcctgttcgatatttgtgatgcagttctggtagaagtggaaaccggtattagtcagcgtccggttaccgaagcctttctgagtagcattgcaccgaaagtgaaactgcgctatgcaccggcaaccccgagcagtaacaaactgtgactcggtaccaaattccagaaaagaggcctcccgaaaggggggccttttttcgttttggtcccgaagttcctattctctagaaagtataggaacttc

SEQ ID NO: 96 - DNA, 4413 bp, Artificial Sequence
  Sequence of sxt4 fragment integrated into the E. coli melobiose operon
aagcctgccgtcagggcaatatcgagaatacttttatcggtatcgctcagccagccttgcaagaagcggatacaggagtgcaaaaaatggctatctctagaaaggcctaccccttaggctttatgcaacagaaacaataataatggagtcatgaacatatggaaaccacgagcaaaaaattcaaaagcgatctgattctggaagcacgtgcaagcctgaaactgggtattccgctggttattagccagatgtgtgaaaccggtatttataccgcaaatgcagttatgatgggtctgctgggcacccaggttctggcagccggtgctctgggtgcactggcatttctgaccctgctgtttgcatgtcatggtattctgagcgttggtggtagcctggcagcggaagcatttggtgcaaacaaaattgatgaagttagccgtattgcaagcggtcagatttggctggcagttaccctgagcctgcctgcaatgctgctgctgtggcatggtgataccattctgctgttatttggtcaagaagaaagcaacgttctgctgaccaaaacctatctgcatagcattctgtggggttttccggcagcactgagtattctgacactgcgtggtattgccagcgcactgaatgttccgcgtctgattaccattaccatgctgacccagctgattctgaataccgcagcagattatgttctgatctttggtaaatttggtctgccgcagctgggtctggcaggtattggttgggcaaccgcactgggtttttgggttagctttaccctgggtctgatcctgctgatttttagcctgaaagtgcgtgattataaactgtttcgttatctgcaccagttcgacaagcagatctttgtgaaaatctttcagaccggttggccgatgggttttcagtggggtgcagaaacagcactgtttaatgttaccgcatgggttgcaggttatctgggcaccgttaccctggcagcacatgatattggttttcagacagcagaactggcaatggttatcccgctgggtgttggtaatgttgcaatgacccgtgttggtcagagcattggtgaaaaaaatccactgggtgcccgtcgtgttgcaagcattggtattaccattgttggtatttatgccagcattgttgccctggttttttggctgtttccgtatcagattgcaggcatttatctgaacattaataacccggaaaacattgaagccatcaaaaaagccaccacctttattccactggcaggtctgtttcagatgttttatagcattcagatcattatcgttggtgcgctggttggtctgcgtgatacctttgttccggttagcatgaatctgattgtttggggtctgggtttagcaggtagctattttatggcaattattctgggttggggtggtattggtatctggctggccatggttctgagtccgctgctgagcgcagttattctgaccgttcgtttttatcgcgtgattgataatctgctggccaacagtgatgatatgctgcagaatgcaagcgttaccaccctgggatgagaaggagatatacatatgaaacgtctgacgctgctgatcattgcaggtattctgtcagttagcacctttctgtgtattacaccggttgcactggccaatattaccgattattatctgaaaaacgagaaactgagcggtcagtttagcgttccggtgaatctgtctgttggtgttcgttttgcacatcgtagcagctatgcaaccgcaattaactttccgaccggtctggatgcagatagcgttgcagttggtgattttaacagcgatagcaaactggatctggccgttaccaattggtttgataacaatgttagcgtgctgctgggtaatggcaatggcagctttggtgcagcaaccaattttccggttggcaccaatccggtttttgttgttaccggtgatgttaatggtgacagtaaactggatttagccgtggcaaattttagcagcaataatgtttcagttctgctgggaaacggtaatggttcttttggcgcagccacaaactttagcgttggtacaaatccgtatagcgtggccattggtgatgtgaataatgatagtgaactggacctggcatttacgaactggttcgataataaagttctggtgctgttaggcaatggtaatggctcgtttggtgccgcaagctcatttccggtggatacctatagcattagcgttgcgattgcagatttcaactcagattctaaattagacctggcgatcaccaattgggtgtcaaataatgtgagtgtgttactggggaatggtaacggtagttttggagctgcgacaaattttcctgtgggtacaaacccgatttttgtggcaaccggtgacgtgaatggcgattctaagctggacttagcagttgcaaataccagctctaataacgttagcgttctgttaggtaacgggaacggctcattcggtgctgccacgaattttccagcaggcaccaacccgtatagtgttgcaattcgcgacgttaacggtgatagcaaattagatttagcggtgaccaactatagcagcaacaacgtgagtgttctgccaggcaacggtaacggatcatttggtattgcgaccaactttccagtaggtacgaatccggaaagcattgcaattgccgattttaatggggattccaagttagatctggcagtgacaaatagcggtaacaataatgtaagcatactgctgaataactttcagggtctgccgaaaaacaagatttgagaaggagatatacatatgaccaataccgaacgtggtctggccgaaattaccagcaccggttataaaagcgaactgcgtagcgaagcccgtgttagcctgcagctggcaattcctctggttctggttgaaatttgtggcaccagcattaatgttgttgatgttgtgatgatgggtttactgggtacacaagtgttagcagcgggtgccctgggagcaattgccttcctgagcgttagcaatacctgctataatatgctgctgagtggtgttgcaaaagcaagcgaagcctttggagccaataaaatcgatcaggtttcacgtattgcctcaggccagatttggttagccctgaccctgtcattaccagccatgctgttactgtggtatatggataccatcctggttctgtttggtcaggttgaaagcaataccctgattgcgaaaacatacctgcattcaattgtgtggggctttcctgccgcagttggtatcctgattctgcgtggcatagcaagtgcagttaacgttcctcagctggttaccgtgaccatgctggttggcctggtgctgaatgcaccggctaattatgtgctgatgttcggcaaattcggtttaccggaattaggcctggctggcattggctgggccagcacactggtgttttggattagttttctggttggtgttgtgctgctgatattttcaccgaaagttcgcgactacaaactgttccgctatttacatcagtttgatcgtcagaccgtggttgagatttttcagacgggctggcctatgggcttcctgctgggtgtggaaagcgttgttctgagcctgaccgcatggctgaccggctatctgggtacagtgaccttagcagcccatgaaattgcaatccagactgccgaactggcgattgtgattccgttaggtattggcaatgttgccgttacccgtgtgggccagacaatcggcgaaaaaaacccgctgggagcacgccgtgcagccctgattggcattatgattggtggcatttatgcgagcctggttgcagtgattttttggttattcccttatcaaatcgcaggcctgtacctgaaaattaacgatccggaatcaatggaagcagttaaaaccgcaacaaactttctgtttttagctggcctgttccagttttttcatagcgtgcagattattgttgtgggtgttctgattggcctgcaggatacctttatccctctgctgatgaatctggtgggctggggactgggcctggcggtttcctattatatgggtattatcctgtgctggggtggcatgggcatctggttaggtctggtactgtcaccgctgctgtcaggcctgatcctgatggtgcgcttttatcaagaaattgccaatcgcattgcgaatagcgacgatggccaagaaagcattagcattgataatgttgaagaactgagctaatagaccaaccccttgcggcctcaatcgggggggatggggttttttgtcgaagttcctattctctagaaagtataggaacttcgcaaccgtctgctgaaggaagccatctgacacttaaagccatcgttgcgct

SEQ ID NO: 97 - DNA, 7377 bp, Artificial Sequence
  Sequence of sxt2 fragment integrated into the E. coli maltose operon
ctgtgaactaaaccgaggtcatgtaaggaatttcgtgatgttgcttgcaaccagccttgcaagaagcggatacaggagtgcaaaaaatggctatctctagaaaggcctaccccttaggctttatgcaacagaaacaataataatggagtcatgaacatgattgataccattagcgttctgctgcgtgaatggaccgttatttttctgaccggtctggcattttggctgtgggaaattcgtagtccgctgcatcagattgaatacaaagccaaatttttcaaagaactgggttgggcaggtatcagctttgtttttcgtattgtttatgcctatgttagcgtggccattatcaaactgctgagcagcctgtttatgggtgaaagcgcaaattttgccggtgttatgtatgttccgctgtggctgcgtattattaccgcatatattctgcaggatctgaccgattatctgctgcatcgtaccatgcatagcaatcagtttctgtggctgacccataaatggcatcatagcaccaaacagagttggtggctgagcggtaataaagatagctttaccggtggtctgctgtataccgttaccgcactgtggtttccgctgctggatattccgagcgaagttatgagcgttgttgcagttcatcaggtgattcataacaactggattcacctgaatgtgaaatggaatagctggctgggtattatcgaatggatttatgttacaccgcgtatccataccctgcatcatctggataccggtggtcgtaatctgagcagtatgtttacctttattgatcgtctgtttggcacctatgtgtttccggaaaactttgatatcgaaaaaagcaaaaaccgcctggatgatcagagcgttaccgttaaaaccattctgggtttctgagaaggagatatacatatgctgaaagattttaaccagttcctgattcgtaccctggcatttgtttttgcctttggcatttttctgacaaccggtgttggtattgcaaaagcagattatctggtgaaaggtggcaaaattaccaatgttcagaataccagcagcaacggtgataattatgcagttagcattagcggtggttttggtccgtgtgcagatcgtgttattattctgccgaccagcggtgttattaatcgtgatattcacatgcgtggttatgaagcagcactgaccgcactgagcaatggttttctggttgatatctatgattataccggtagcagctgtagcaatggtggccagctgaccattaccaatcagctgggtaaactgattagcaattgagaaggagatatacatatgaccaatcagaacaaccaagagctggaaaatgatctgccgattgcaaaacagccgtgtccggttaatagctataatgaatgggataccctggaagaagttattgttggtagcgttgaaggtgcaatgctgcctgcactggaaccgattaacaaatggacctttccgtttgaagaactggaaagcgcacagaaaattctgagcgaacgtggtggtgttccgtatccgcctgaaatgattaccctggcacataaagaactgaacgagtttattcatatcctggaagccgaaggtgttaaagttcgtcgtgttaaaccggttgattttagcgttccgtttagcacaccggcatggcaggttggtagcggtttttgtgcagcaaatccgcgtgatgtttttctggttattggcaacgaaattatcgaagcaccgatggcagatcgtaatcgttattttgaaacctgggcatatcgcgaaatgctgaaagaatattttcaggcaggcgcaaaatggaccgcagcaccgaaaccgcagctgtttgatgcacagtatgatttcaattttcagtttccgcagctgggtgaaccgcctcgttttgttgttaccgaatttgaaccgacctttgatgcagccgattttgttcgttgtggtcgtgatatttttggccagaaaagccatgttaccaatggtctgggtattgaatggctgcagcgtcatctggaagatgaatatcgcattcatatcatcgaaagccattgtccggaagcactgcatattgataccaccctgatgccgctggcaccgggtaaaattctggttaatccggaatttgtggacgtgaataaactgccgaaaattctgaaaagctgggatattctggttgcaccgtatccgaatcatattccgcagaatcagctgcgtctggttagcgaatgggcaggtctgaatgttctgatgctggatgaagaacgtgtgatcgtggaaaaaaatcaagagcagatgatcaaagccctgaaagattggggttttaaaccgattgtttgccacttcgaaagctattatccgtttctgggtagctttcattgtgcaaccctggatgttcgtcgtcgtggcaccctgcagagctatttttgagaaggagatatacatatgacgaccgcagatctgattctgatcaataattggtatgttgtggccaaggtggaagattgtaaaccgggtagcattaccaccgcactgctgctgggtgttaaactggttctgtggcgtagccgtgaacagaatagcccgattcagatttggcaggattattgtccgcatcgtggtgttgcactgagcatgggtgaaattgtgaataataccctggtttgtccgtatcatggttggcgttataatcaggcaggtaaatgtgttcatattccggcacatccggatatgacccctccggcaagcgcacaggcaaaaatctatcattgtcaagaacgttatggtctggtttgggtttgtctgggtgatccggttaatgatattccgagtctgccggaatgggatgatccgaattatcataatacctgcaccaagagctactttatccaggcaagcgcatttcgtgtgatggataactttattgatgtgagccattttccgtttgtgcatgatggtggtctgggcgatcgtaatcatgcacagattgaagaatttgaggtgaaagtggataaagacggtattagcattggcaatctgaaactgcagatgcctcgttttaatagcagcaatgaagatgatagctggaccctgtatcagcgtattagccatccgctgtgtcagtattatatcaccgaaagcagcgaaattcgtacagcagatctgatgctggttaccccgattgatgaagataattcactggttcgtatgctggtgacctggaatcgtagcgaaattctggaaagcaccgttctggaagaatttgatgaaaccattgaacaggatatcccgattattcatagccagcagcctgcacgtctgccgctgctgccgagcaagcagattaatatgcagtggctgagccaagaaattcatgttccgagcgatcgttgtaccgttgcatatcgtcgttggctgaaagaactgggcgttacctatggtgtttgttgagaaggagatatacatatgcagattctgggtatcagcgcctattatcatgatagcgcagcagcaatggttattgatggtgaaattgttgcagcagcacaagaagaacgttttagccgtcgtaaacatgatgcaggttttccgaccggtgcaattacctattgtctgaaacaggttggcaccaaactgcagtatattgatcagatcgtgttctatgataaaccgctggtgaaatttgaacgtctgctggaaacctatctggcctatgcaccgaaaggttttggtagttttattaccgcaatgccggtgtggctgaaagagaaactgtatctgaaaaccctgctgaaaaaagaactggcactgctgggtgaatgtaaagcaagccagctgcctccgctgctgtttaccagccatcatcaggcacatgcagcagcagcattttttccgagcccgtttcagcgtgcagcagttctgtgtctggatggtgttggtgaatgggcaaccaccagtgtttggctgggtgaaggtaataaactgacaccgcagtgggaaattgattttccgcatagcctgggcctgctgtatagcgcatttacctattataccggctttaaagtgaacagcggtgagtataaactgatgggtctggcaccgtatggtgaaccgaaatatgttgatcagattctgaaacatctgctggatctgaaagaagatggcacctttcgtctgaacatggattatttcaattataccgttggtctgaccatgaccaaccataaatttcatagcatgtttggtggtccgcctcgtcaggcagaaggtaaaattagccagcgtgatatggatctggcaagcagcattcagaaagttaccgaagaagtgattctgcgtctggcacgtaccattaagaaagaattaggtgttgaatacctgtgtctggcaggcggtgttggtctgaattgtgttgcaaatggtcgtattctgcgtgagagcgattttaaagatatttggattcagcctgcagccggtgatgcaggtagcgcagttggtgcagcactggcaatttggcatgaatatcataaaaaaccgcgtaccagcaccgcaggcgatcgtatgaaaggtagctatctgggtccgagctttagcgaagcagaaattctgcagtttctgaacagcgtgaatattccgtatcatcgttgtgtggataatgaactgatggcacgtctggcggaaattctggatcagggtaatgttgttggttggtttagcggtcgtatggaatttggtccgcgtgcactgggtggtcgtagcattattggtgatagccgtagcccgaaaatgcagagcgttatgaatctgaaaatcaaatatcgcgaaagcttccgtccgtttgcaccgagcgttctggcagaacgtgttagcgattattttgatctggatcgtccgagcccgtatatgctgctggttgcacaggttaaagaaaatctgcatattccgatgacccaagaacagcatgaactgtttggtatcgaaaaactgaatgttccgcgtagccagattccggcagttacccatgttgattatagcgcacgtattcagaccgttcataaagaaaccaatccgcgttattatgaactgatccgtcattttgaagcacgtaccggttgtgcagttctggttaataccagctttaatgttcgtggtgaaccgattgtgtgtacaccggaagatgcatatcgttgttttatgcgtaccgagatggattacctggtgatggaaaattttctgctggtgaaaagcgaacagcctcgtggtaatagtgatgaaagctggcagaaagaatttgagctggattgagaaggagatatacatatggaacaaattaaagaactggataagaaaggcctgcgtgaatttggtctgattggtggtagcattgttgccgttctgtttggttttctgctgccggttattcgtcatcatagcctgagcgttattccgtgggttgttgcaggttttctgtggatttgggcaattattgcaccgaccaccctgagctttatctatcagatttggatgcgtattggtctggtgctgggttggattcagacccgtattattctgggtgttctgttctatattatgattaccccgatcggttttattcgtcgtctgctgaatcaggatccgatgacccgtatttttgaaccggaactgccgacctatcgtcagctgagcaaaagccgtaccacccagagcatggaaaaaccgttctgagaaggagatatacatatgttaaaagacacctgggattttatcaaggatatcgcaggctttatcaaagaacagaaaaactatctgctgattccgctgattattaccctggttagcctgggtgcactgattgtttttgcacagagcagcgcaattgcaccgtttatctataccctgttttgagaaggagatatacatatgagcaacttcaaaggcagcgttaaaattgcactgatgggcattctgattttttgcggtctgatttttggtgtggcctttgttgaaattggtctgcgtattgcaggcattgaacatattgcctttcatagcattgatgaacatcgtggttgggttggtcgtccgcatgttagcggttggtatcgtaccgaaggtgaagcacatattcagatgaatagtgatggttttcgtgatcgcgaacacattaaagtgaaaccggaaaatacctttcgtattgccctgctgggtgatagctttgttgaaagcatgcaggttccgctggaacagaatctggcagcagttattgaaggcgaaattagcagctgtattgcactggcaggtcgtaaagccgaagttattaactttggtgttaccggttatggcaccgatcaagaactgattaccctgcgtgaaaaagtgtgggattatagtccggatattgttgtgctggatttctataccggtaacgatattgttgataatagccgtgcactgtcccagaaattctatccgaatgaactgggtagcctgaaaccgttttttatcctgcgtgatggtaatctggttgttgatgcaagctttatcaacaccgataactatcgtagcaaactgacctggtggggtaaaacctatatgaaaatcaaagatcatagccgcattctgcaggtcctgaatatggttcgtgatgcactgaataatagcagccgtggttttagcagccaggcaattgaagaaccgctgtttagtgatggtaaacaggataccaaactgagcggcttcttcgatatctataaaccgcctaccgatccggaatggcagcaggcctggcaggttaccgaaaaactgattagtagcatgcagcatgaagtgaccgccaaaaaagccgattttctggttgttacctttggcggtccgtttcagcgcgaaccgctggttcgtcagaaagaaatgcaagaactgggtctgaccgattggttttatccggaaaaacgtattacccgtctgggtgaagatgaaggttttagcgtgctgaatctgagcccgaatctgcaggtttatagcgaacagaataatgcctgtctgtatggttttgatgatacccagggttgtgttggtcattggaatgcactgggtcatcaggttgcaggtaaaatgattgcaagcaaaatttgtcagcagcagatgcgtgaaagcattctgccgcataaacatgatccgagcagccagagcagcccgattacccagagcgttattcagtaatactctaaccccatcggccgtcttaggggttttttgtcgaagttcctattctctagaaagtataggaacttcgacctgtggggtgactttgccgccgctgccgtgatgtctgcattaccgatc

SEQ ID NO: 98 - DNA, 6062 bp, Artificial Sequence
  Sequence of sxt2 fragment integrated into the maltose operon after deletetion of sxtL
ctgtgaactaaaccgaggtcatgtaaggaatttcgtgatgttgcttgcaaccagccttgcaagaagcggatacaggagtgcaaaaaatggctatctctagaaaggcctaccccttaggctttatgcaacagaaacaataataatggagtcatgaacatgattgataccattagcgttctgctgcgtgaatggaccgttatttttctgaccggtctggcattttggctgtgggaaattcgtagtccgctgcatcagattgaatacaaagccaaatttttcaaagaactgggttgggcaggtatcagctttgtttttcgtattgtttatgcctatgttagcgtggccattatcaaactgctgagcagcctgtttatgggtgaaagcgcaaattttgccggtgttatgtatgttccgctgtggctgcgtattattaccgcatatattctgcaggatctgaccgattatctgctgcatcgtaccatgcatagcaatcagtttctgtggctgacccataaatggcatcatagcaccaaacagagttggtggctgagcggtaataaagatagctttaccggtggtctgctgtataccgttaccgcactgtggtttccgctgctggatattccgagcgaagttatgagcgttgttgcagttcatcaggtgattcataacaactggattcacctgaatgtgaaatggaatagctggctgggtattatcgaatggatttatgttacaccgcgtatccataccctgcatcatctggataccggtggtcgtaatctgagcagtatgtttacctttattgatcgtctgtttggcacctatgtgtttccggaaaactttgatatcgaaaaaagcaaaaaccgcctggatgatcagagcgttaccgttaaaaccattctgggtttctgagaaggagatatacatatgctgaaagattttaaccagttcctgattcgtaccctggcatttgtttttgcctttggcatttttctgacaaccggtgttggtattgcaaaagcagattatctggtgaaaggtggcaaaattaccaatgttcagaataccagcagcaacggtgataattatgcagttagcattagcggtggttttggtccgtgtgcagatcgtgttattattctgccgaccagcggtgttattaatcgtgatattcacatgcgtggttatgaagcagcactgaccgcactgagcaatggttttctggttgatatctatgattataccggtagcagctgtagcaatggtggccagctgaccattaccaatcagctgggtaaactgattagcaattgagaaggagatatacatatgaccaatcagaacaaccaagagctggaaaatgatctgccgattgcaaaacagccgtgtccggttaatagctataatgaatgggataccctggaagaagttattgttggtagcgttgaaggtgcaatgctgcctgcactggaaccgattaacaaatggacctttccgtttgaagaactggaaagcgcacagaaaattctgagcgaacgtggtggtgttccgtatccgcctgaaatgattaccctggcacataaagaactgaacgagtttattcatatcctggaagccgaaggtgttaaagttcgtcgtgttaaaccggttgattttagcgttccgtttagcacaccggcatggcaggttggtagcggtttttgtgcagcaaatccgcgtgatgtttttctggttattggcaacgaaattatcgaagcaccgatggcagatcgtaatcgttattttgaaacctgggcatatcgcgaaatgctgaaagaatattttcaggcaggcgcaaaatggaccgcagcaccgaaaccgcagctgtttgatgcacagtatgatttcaattttcagtttccgcagctgggtgaaccgcctcgttttgttgttaccgaatttgaaccgacctttgatgcagccgattttgttcgttgtggtcgtgatatttttggccagaaaagccatgttaccaatggtctgggtattgaatggctgcagcgtcatctggaagatgaatatcgcattcatatcatcgaaagccattgtccggaagcactgcatattgataccaccctgatgccgctggcaccgggtaaaattctggttaatccggaatttgtggacgtgaataaactgccgaaaattctgaaaagctgggatattctggttgcaccgtatccgaatcatattccgcagaatcagctgcgtctggttagcgaatgggcaggtctgaatgttctgatgctggatgaagaacgtgtgatcgtggaaaaaaatcaagagcagatgatcaaagccctgaaagattggggttttaaaccgattgtttgccacttcgaaagctattatccgtttctgggtagctttcattgtgcaaccctggatgttcgtcgtcgtggcaccctgcagagctatttttgagaaggagatatacatatgacgaccgcagatctgattctgatcaataattggtatgttgtggccaaggtggaagattgtaaaccgggtagcattaccaccgcactgctgctgggtgttaaactggttctgtggcgtagccgtgaacagaatagcccgattcagatttggcaggattattgtccgcatcgtggtgttgcactgagcatgggtgaaattgtgaataataccctggtttgtccgtatcatggttggcgttataatcaggcaggtaaatgtgttcatattccggcacatccggatatgacccctccggcaagcgcacaggcaaaaatctatcattgtcaagaacgttatggtctggtttgggtttgtctgggtgatccggttaatgatattccgagtctgccggaatgggatgatccgaattatcataatacctgcaccaagagctactttatccaggcaagcgcatttcgtgtgatggataactttattgatgtgagccattttccgtttgtgcatgatggtggtctgggcgatcgtaatcatgcacagattgaagaatttgaggtgaaagtggataaagacggtattagcattggcaatctgaaactgcagatgcctcgttttaatagcagcaatgaagatgatagctggaccctgtatcagcgtattagccatccgctgtgtcagtattatatcaccgaaagcagcgaaattcgtacagcagatctgatgctggttaccccgattgatgaagataattcactggttcgtatgctggtgacctggaatcgtagcgaaattctggaaagcaccgttctggaagaatttgatgaaaccattgaacaggatatcccgattattcatagccagcagcctgcacgtctgccgctgctgccgagcaagcagattaatatgcagtggctgagccaagaaattcatgttccgagcgatcgttgtaccgttgcatatcgtcgttggctgaaagaactgggcgttacctatggtgtttgttgagaaggagatatacatatgcagattctgggtatcagcgcctattatcatgatagcgcagcagcaatggttattgatggtgaaattgttgcagcagcacaagaagaacgttttagccgtcgtaaacatgatgcaggttttccgaccggtgcaattacctattgtctgaaacaggttggcaccaaactgcagtatattgatcagatcgtgttctatgataaaccgctggtgaaatttgaacgtctgctggaaacctatctggcctatgcaccgaaaggttttggtagttttattaccgcaatgccggtgtggctgaaagagaaactgtatctgaaaaccctgctgaaaaaagaactggcactgctgggtgaatgtaaagcaagccagctgcctccgctgctgtttaccagccatcatcaggcacatgcagcagcagcattttttccgagcccgtttcagcgtgcagcagttctgtgtctggatggtgttggtgaatgggcaaccaccagtgtttggctgggtgaaggtaataaactgacaccgcagtgggaaattgattttccgcatagcctgggcctgctgtatagcgcatttacctattataccggctttaaagtgaacagcggtgagtataaactgatgggtctggcaccgtatggtgaaccgaaatatgttgatcagattctgaaacatctgctggatctgaaagaagatggcacctttcgtctgaacatggattatttcaattataccgttggtctgaccatgaccaaccataaatttcatagcatgtttggtggtccgcctcgtcaggcagaaggtaaaattagccagcgtgatatggatctggcaagcagcattcagaaagttaccgaagaagtgattctgcgtctggcacgtaccattaagaaagaattaggtgttgaatacctgtgtctggcaggcggtgttggtctgaattgtgttgcaaatggtcgtattctgcgtgagagcgattttaaagatatttggattcagcctgcagccggtgatgcaggtagcgcagttggtgcagcactggcaatttggcatgaatatcataaaaaaccgcgtaccagcaccgcaggcgatcgtatgaaaggtagctatctgggtccgagctttagcgaagcagaaattctgcagtttctgaacagcgtgaatattccgtatcatcgttgtgtggataatgaactgatggcacgtctggcggaaattctggatcagggtaatgttgttggttggtttagcggtcgtatggaatttggtccgcgtgcactgggtggtcgtagcattattggtgatagccgtagcccgaaaatgcagagcgttatgaatctgaaaatcaaatatcgcgaaagcttccgtccgtttgcaccgagcgttctggcagaacgtgttagcgattattttgatctggatcgtccgagcccgtatatgctgctggttgcacaggttaaagaaaatctgcatattccgatgacccaagaacagcatgaactgtttggtatcgaaaaactgaatgttccgcgtagccagattccggcagttacccatgttgattatagcgcacgtattcagaccgttcataaagaaaccaatccgcgttattatgaactgatccgtcattttgaagcacgtaccggttgtgcagttctggttaataccagctttaatgttcgtggtgaaccgattgtgtgtacaccggaagatgcatatcgttgttttatgcgtaccgagatggattacctggtgatggaaaattttctgctggtgaaaagcgaacagcctcgtggtaatagtgatgaaagctggcagaaagaatttgagctggattgagaaggagatatacatatggaacaaattaaagaactggataagaaaggcctgcgtgaatttggtctgattggtggtagcattgttgccgttctgtttggttttctgctgccggttattcgtcatcatagcctgagcgttattccgtgggttgttgcaggttttctgtggatttgggcaattattgcaccgaccaccctgagctttatctatcagatttggatgcgtattggtctggtgctgggttggattcagacccgtattattctgggtgttctgttctatattatgattaccccgatcggttttattcgtcgtctgctgaatcaggatccgatgacccgtatttttgaaccggaactgccgacctatcgtcagctgagcaaaagccgtaccacccagagcatggaaaaaccgttctgagaaggagatatacatatgttaaaagacacctgggattttatcaaggatatcgcaggctttatcaaagaacagaaaaactatctgctgattccgctgattattaccctggttagcctgggtgcactgattgtttttgcacagagcagcgcaattgcaccgtttatctataccctgttttgatactctaaccccatcggccgtcttaggggttttttgtcgaagttcctattctctagaaagtataggaacttcacctgtggggtgactttgccgccgctgccgtgatgtctgcattaccgatc

SEQ ID NO: 99 - DNA, 5462 bp, Artificial Sequence
  Sequence of sxt2 fragment integrated into the maltose operon
ctgtgaactaaaccgaggtcatgtaaggaatttcgtgatgttgcttgcaaccagccttgcaagaagcggatacaggagtgcaaaaaatggctatctctagaaaggcctaccccttaggctttatgcaacagaaacaataataatggagtcatgaacatgattgataccattagcgttctgctgcgtgaatggaccgttatttttctgaccggtctggcattttggctgtgggaaattcgtagtccgctgcatcagattgaatacaaagccaaatttttcaaagaactgggttgggcaggtatcagctttgtttttcgtattgtttatgcctatgttagcgtggccattatcaaactgctgagcagcctgtttatgggtgaaagcgcaaattttgccggtgttatgtatgttccgctgtggctgcgtattattaccgcatatattctgcaggatctgaccgattatctgctgcatcgtaccatgcatagcaatcagtttctgtggctgacccataaatggcatcatagcaccaaacagagttggtggctgagcggtaataaagatagctttaccggtggtctgctgtataccgttaccgcactgtggtttccgctgctggatattccgagcgaagttatgagcgttgttgcagttcatcaggtgattcataacaactggattcacctgaatgtgaaatggaatagctggctgggtattatcgaatggatttatgttacaccgcgtatccataccctgcatcatctggataccggtggtcgtaatctgagcagtatgtttacctttattgatcgtctgtttggcacctatgtgtttccggaaaactttgatatcgaaaaaagcaaaaaccgcctggatgatcagagcgttaccgttaaaaccattctgggtttctgagaaggagatatacatatgctgaaagattttaaccagttcctgattcgtaccctggcatttgtttttgcctttggcatttttctgacaaccggtgttggtattgcaaaagcagattatctggtgaaaggtggcaaaattaccaatgttcagaataccagcagcaacggtgataattatgcagttagcattagcggtggttttggtccgtgtgcagatcgtgttattattctgccgaccagcggtgttattaatcgtgatattcacatgcgtggttatgaagcagcactgaccgcactgagcaatggttttctggttgatatctatgattataccggtagcagctgtagcaatggtggccagctgaccattaccaatcagctgggtaaactgattagcaattgagaaggagatatacatatgaccaatcagaacaaccaagagctggaaaatgatctgccgattgcaaaacagccgtgtccggttaatagctataatgaatgggataccctggaagaagttattgttggtagcgttgaaggtgcaatgctgcctgcactggaaccgattaacaaatggacctttccgtttgaagaactggaaagcgcacagaaaattctgagcgaacgtggtggtgttccgtatccgcctgaaatgattaccctggcacataaagaactgaacgagtttattcatatcctggaagccgaaggtgttaaagttcgtcgtgttaaaccggttgattttagcgttccgtttagcacaccggcatggcaggttggtagcggtttttgtgcagcaaatccgcgtgatgtttttctggttattggcaacgaaattatcgaagcaccgatggcagatcgtaatcgttattttgaaacctgggcatatcgcgaaatgctgaaagaatattttcaggcaggcgcaaaatggaccgcagcaccgaaaccgcagctgtttgatgcacagtatgatttcaattttcagtttccgcagctgggtgaaccgcctcgttttgttgttaccgaatttgaaccgacctttgatgcagccgattttgttcgttgtggtcgtgatatttttggccagaaaagccatgttaccaatggtctgggtattgaatggctgcagcgtcatctggaagatgaatatcgcattcatatcatcgaaagccattgtccggaagcactgcatattgataccaccctgatgccgctggcaccgggtaaaattctggttaatccggaatttgtggacgtgaataaactgccgaaaattctgaaaagctgggatattctggttgcaccgtatccgaatcatattccgcagaatcagctgcgtctggttagcgaatgggcaggtctgaatgttctgatgctggatgaagaacgtgtgatcgtggaaaaaaatcaagagcagatgatcaaagccctgaaagattggggttttaaaccgattgtttgccacttcgaaagctattatccgtttctgggtagctttcattgtgcaaccctggatgttcgtcgtcgtggcaccctgcagagctatttttgagaaggagatatacatatgacgaccgcagatctgattctgatcaataattggtatgttgtggccaaggtggaagattgtaaaccgggtagcattaccaccgcactgctgctgggtgttaaactggttctgtggcgtagccgtgaacagaatagcccgattcagatttggcaggattattgtccgcatcgtggtgttgcactgagcatgggtgaaattgtgaataataccctggtttgtccgtatcatggttggcgttataatcaggcaggtaaatgtgttcatattccggcacatccggatatgacccctccggcaagcgcacaggcaaaaatctatcattgtcaagaacgttatggtctggtttgggtttgtctgggtgatccggttaatgatattccgagtctgccggaatgggatgatccgaattatcataatacctgcaccaagagctactttatccaggcaagcgcatttcgtgtgatggataactttattgatgtgagccattttccgtttgtgcatgatggtggtctgggcgatcgtaatcatgcacagattgaagaatttgaggtgaaagtggataaagacggtattagcattggcaatctgaaactgcagatgcctcgttttaatagcagcaatgaagatgatagctggaccctgtatcagcgtattagccatccgctgtgtcagtattatatcaccgaaagcagcgaaattcgtacagcagatctgatgctggttaccccgattgatgaagataattcactggttcgtatgctggtgacctggaatcgtagcgaaattctggaaagcaccgttctggaagaatttgatgaaaccattgaacaggatatcccgattattcatagccagcagcctgcacgtctgccgctgctgccgagcaagcagattaatatgcagtggctgagccaagaaattcatgttccgagcgatcgttgtaccgttgcatatcgtcgttggctgaaagaactgggcgttacctatggtgtttgttgagaaggagatatacatatgcagattctgggtatcagcgcctattatcatgatagcgcagcagcaatggttattgatggtgaaattgttgcagcagcacaagaagaacgttttagccgtcgtaaacatgatgcaggttttccgaccggtgcaattacctattgtctgaaacaggttggcaccaaactgcagtatattgatcagatcgtgttctatgataaaccgctggtgaaatttgaacgtctgctggaaacctatctggcctatgcaccgaaaggttttggtagttttattaccgcaatgccggtgtggctgaaagagaaactgtatctgaaaaccctgctgaaaaaagaactggcactgctgggtgaatgtaaagcaagccagctgcctccgctgctgtttaccagccatcatcaggcacatgcagcagcagcattttttccgagcccgtttcagcgtgcagcagttctgtgtctggatggtgttggtgaatgggcaaccaccagtgtttggctgggtgaaggtaataaactgacaccgcagtgggaaattgattttccgcatagcctgggcctgctgtatagcgcatttacctattataccggctttaaagtgaacagcggtgagtataaactgatgggtctggcaccgtatggtgaaccgaaatatgttgatcagattctgaaacatctgctggatctgaaagaagatggcacctttcgtctgaacatggattatttcaattataccgttggtctgaccatgaccaaccataaatttcatagcatgtttggtggtccgcctcgtcaggcagaaggtaaaattagccagcgtgatatggatctggcaagcagcattcagaaagttaccgaagaagtgattctgcgtctggcacgtaccattaagaaagaattaggtgttgaatacctgtgtctggcaggcggtgttggtctgaattgtgttgcaaatggtcgtattctgcgtgagagcgattttaaagatatttggattcagcctgcagccggtgatgcaggtagcgcagttggtgcagcactggcaatttggcatgaatatcataaaaaaccgcgtaccagcaccgcaggcgatcgtatgaaaggtagctatctgggtccgagctttagcgaagcagaaattctgcagtttctgaacagcgtgaatattccgtatcatcgttgtgtggataatgaactgatggcacgtctggcggaaattctggatcagggtaatgttgttggttggtttagcggtcgtatggaatttggtccgcgtgcactgggtggtcgtagcattattggtgatagccgtagcccgaaaatgcagagcgttatgaatctgaaaatcaaatatcgcgaaagcttccgtccgtttgcaccgagcgttctggcagaacgtgttagcgattattttgatctggatcgtccgagcccgtatatgctgctggttgcacaggttaaagaaaatctgcatattccgatgacccaagaacagcatgaactgtttggtatcgaaaaactgaatgttccgcgtagccagattccggcagttacccatgttgattatagcgcacgtattcagaccgttcataaagaaaccaatccgcgttattatgaactgatccgtcattttgaagcacgtaccggttgtgcagttctggttaataccagctttaatgttcgtggtgaaccgattgtgtgtacaccggaagatgcatatcgttgttttatgcgtaccgagatggattacctggtgatggaaaattttctgctggtgaaaagcgaacagcctcgtggtaatagtgatgaaagctggcagaaagaatttgagctggattgatactctaaccccatcggccgtcttaggggttttttgtcgaagttcctattctctagaaagtataggaacttcacctgtggggtgactttgccgccgctgccgtgatgtctgcattaccgatc

SEQ ID NO: 100 - DNA, 112 bp, Cylindrospermopsis raciborskii T3
agtccagccttgcaagaagcggatacaggagtgcaaaaaatggctatctctagaaaggcctaccccttaggctttatgcaacagaaacaataataatggagtcatgaacatg

SEQ ID NO: 101 - DNA, 114 bp, Cylindrospermopsis raciborskii T3
agtccagccttgcaagaagcggatacaggagtgcaaaaaatggctatctctagaaaggcctaccccttaggctttatgcaacagaaacaataataatggagtcatgaacatatg